European Patent Specification EP 3 895 529 B1, published April 29, 2026. Title: RODENTS HAVING A HUMANIZED TMPRSS GENE. Applicant: REGENERON PHARMACEUTICALS, INC. The sequence listing filed with the application follows.

SEQUENCE LISTING (72 sequences)

SEQ ID NO: 1 - DNA, 3175 bp, Mus musculus
gcctttcctggccgttccctccttctggccgaggtgcctgcgtttaggggtgtcaccctggctcccgggacgccgcctccggagatttaagcgagaactggagtaggtcgtgtacttggagcggacgaggaagccaagagctcggacagaggcggagaggggcgggaagcgcaacaggtcacctggaggaagccccatactgacctcctcatgctgctgacacaggcaggatggcattgaactcagggtcacctccaggaatcggaccttgctatgagaaccacgggtatcagtctgagcacatctgtcctccgagaccaccagtggctcccaatggctacaacttgtatccagcccagtactacccatctccagtgcctcagtatgctccgaggattacaacgcaagcctcaacatctgtcatccacacacatcccaagtcctcaggagcactgtgcacctcaaagtctaagaaatcgctgtgtttagccctcgccctgggcactgtcctcacgggagctgctgtggctgctgtcttgctttggaggttctgggacagcaactgttctacgtctgagatggagtgtgggtcttcaggcacatgcatcagctcttctctctggtgtgacggggtagcacattgtcccaacggagaagatgagaaccgttgtgttcgtctctacggacaaagcttcatcctccaggtttactcatctcagaggaaagcctggtatcccgtgtgccaggatgattggagtgagagctacgggagagcagcatgtaaagacatgggatacaagaacaatttttattctagccaagggataccagaccagagcggggcaacgagctttatgaagctgaatgtgagctcaggcaacgttgacctctataaaaaactctaccacagtgactcatgttcatcccgcatggtggtttctttgcgctgtatagaatgcggggttcgctcagtgaaacgccagagcaggattgtgggtggattgaatgcctcaccaggagactggccctggcaggtcagcctgcacgtccaaggcgtccacgtctgcggaggctccatcatcacccccgagtggattgtgacggccgcccactgtgtggaagaacccctcagcagcccgaggtactggacggcatttgcgggaattctgagacagtctctcatgttctatggaagtagacaccaggtagaaaaagtaatttcccatccaaattacgactctaagaccaagaataacgacattgctctcatgaagctgcagacacctttggcttttaatgatctagtgaagccagtgtgtctgccgaacccaggcatgatgctagacctagaccaggaatgctggatttcggggtggggggccacctatgagaaagggaagacctcggacgtgttgaatgctgccatggtacccttgatcgagccctccaaatgtaatagtaaatacatatacaacaacctaatcacaccagccatgatctgtgccggcttcctccaggggtctgtcgactcttgccagggagacagtggagggccgctggttactttgaagaatgggatctggtggctgattggggacacgagctggggctcgggctgtgccaaggcactcagacctggagtatacgggaacgtgacggtatttacagattggatctaccagcaaatgagggcgaacagctaatccacgtggctttgtcccagacttcctttgtcttcaacaaccttctgcaagaaaaccaagggcctgaattttaacttcctgtgcacaatgtaccttttgagatgattcgaagggcctttcacttttattaaacagtgacttgtttgactgtgctccctggtcctgtgagggcttcagtgccccacccctgggccacttctgcagctcccaccagaatggatgaccagattctgttgggtttgggcacatagggccaaaggcagaggagggtggcactctcatgttggaacttcttttgggctcatgctcaggccttttttggatcactaaggactatgacctctgagtaacctgatgacctgagaaagagtaaggaggccaggcagggccttgggcccaggaacaggtaccttgagagtgagagctacccattgcctgtggcctaaatctgctgtgcaggttgggctggtcatactgtcatgatttcattaacagcctgggtgaacatggctgggagtaaagggcttgctctcctgcatgttgacatgacggccctttccaagggtgatggaggctttcccaagctaagggcctaggcagatctctcagagcaagaagctaatgccggcatgtcccttgggtgagctctacatggtgttattcagtctggttcttggctccccactactgtttctctcagcctctcagagcctgaaacttacctcttagctttggctacaggcatggcctagtacctgatggagcctgtatagctcagctaatcaaatggaggctcaggtccatcagaatcagggacttgtgatttcagtcaccttgcttctgggttgtgtttcttctcttactacctcactgcacctggacactagagtggatgaatgtctggagttcacctgcatttggactgtgtgattgtgcctcagacactagacctcttccagatggttaggttgttctgtagactggcaatgagattagaagttcctagcttcagataaagatgaaagagaggagatcattgtcttctgtcttcttctggccctgggtttataccaggaaagccatgccagaattaccaaatatgaagtatgaatgtcttacccacggtgaggctctgcctccttctctctgcctggttcttcagaaggcagtgaatgggtcataactgggactccatctttgctggggaaagtctcccacctagggaatggttaccactccatgtaaagaaaactccctcatgcgtcctctgggaccttcttagatgctgtaaggtacctacatacagactaaatgtgcaagcaccttgaagtgtgagaacctgtcccctccttagctctccttgtctttgctgttggttggttatttcctgctttgtgtctgttctgagctgtgagattccactgtgaaatatatgaataaagtatataattcttttaaaaaaaaaaaaaaaa

SEQ ID NO: 2 - protein, 490 aa, Mus musculus
MALNSGSPPGIGPCYENHGYQSEHICPPRPPVAPNGYNLYPAQYYPSPVPQYAPRITTQASTSVIHTHPKSSGALCTSKSKKSLCLALALGTVLTGAAVAAVLLWRFWDSNCSTSEMECGSSGTCISSSLWCDGVAHCPNGEDENRCVRLYGQSFILQVYSSQRKAWYPVCQDDWSESYGRAACKDMGYKNNFYSSQGIPDQSGATSFMKLNVSSGNVDLYKKLYHSDSCSSRMVVSLRCIECGVRSVKRQSRIVGGLNASPGDWPWQVSLHVQGVHVCGGSIITPEWIVTAAHCVEEPLSSPRYWTAFAGILRQSLMFYGSRHQVEKVISHPNYDSKTKNNDIALMKLQTPLAFNDLVKPVCLPNPGMMLDLDQECWISGWGATYEKGKTSDVLNAAMVPLIEPSKCNSKYIYNNLITPAMICAGFLQGSVDSCQGDSGGPLVTLKNGIWWLIGDTSWGSGCAKALRPGVYGNVTVFTDWIYQQMRANS

SEQ ID NO: 3 - DNA, 3212 bp, Homo sapiens
gagtaggcgcgagctaagcaggaggcggaggcggaggcggagggcgaggggcggggagcgccgcctggagcgcggcaggtcatattgaacattccagatacctatcattactcgatgctgttgataacagcaagatggctttgaactcagggtcaccaccagctattggaccttactatgaaaaccatggataccaaccggaaaacccctatcccgcacagcccactgtggtccccactgtctacgaggtgcatccggctcagtactacccgtcccccgtgccccagtacgccccgagggtcctgacgcaggcttccaaccccgtcgtctgcacgcagcccaaatccccatccgggacagtgtgcacctcaaagactaagaaagcactgtgcatcaccttgaccctggggaccttcctcgtgggagctgcgctggccgctggcctactctggaagttcatgggcagcaagtgctccaactctgggatagagtgcgactcctcaggtacctgcatcaacccctctaactggtgtgatggcgtgtcacactgccccggcggggaggacgagaatcggtgtgttcgcctctacggaccaaacttcatccttcaggtgtactcatctcagaggaagtcctggcaccctgtgtgccaagacgactggaacgagaactacgggcgggcggcctgcagggacatgggctataagaataatttttactctagccaaggaatagtggatgacagcggatccaccagctttatgaaactgaacacaagtgccggcaatgtcgatatctataaaaaactgtaccacagtgatgcctgttcttcaaaagcagtggtttctttacgctgtatagcctgcggggtcaacttgaactcaagccgccagagcaggattgtgggcggcgagagcgcgctcccgggggcctggccctggcaggtcagcctgcacgtccagaacgtccacgtgtgcggaggctccatcatcacccccgagtggatcgtgacagccgcccactgcgtggaaaaacctcttaacaatccatggcattggacggcatttgcggggattttgagacaatctttcatgttctatggagccggataccaagtagaaaaagtgatttctcatccaaattatgactccaagaccaagaacaatgacattgcgctgatgaagctgcagaagcctctgactttcaacgacctagtgaaaccagtgtgtctgcccaacccaggcatgatgctgcagccagaacagctctgctggatttccgggtggggggccaccgaggagaaagggaagacctcagaagtgctgaacgctgccaaggtgcttctcattgagacacagagatgcaacagcagatatgtctatgacaacctgatcacaccagccatgatctgtgccggcttcctgcaggggaacgtcgattcttgccagggtgacagtggagggcctctggtcacttcgaagaacaatatctggtggctgataggggatacaagctggggttctggctgtgccaaagcttacagaccaggagtgtacgggaatgtgatggtattcacggactggatttatcgacaaatgagggcagacggctaatccacatggtcttcgtccttgacgtcgttttacaagaaaacaatggggctggttttgcttccccgtgcatgatttactcttagagatgattcagaggtcacttcatttttattaaacagtgaacttgtctggctttggcactctctgccattctgtgcaggctgcagtggctcccctgcccagcctgctctccctaaccccttgtccgcaaggggtgatggccggctggttgtgggcactggcggtcaagtgtggaggagaggggtggaggctgccccattgagatcttcctgctgagtcctttccaggggccaattttggatgagcatggagctgtcacctctcagctgctggatgacttgagatgaaaaaggagagacatggaaagggagacagccaggtggcacctgcagcggctgccctctggggccacttggtagtgtccccagcctacctctccacaaggggattttgctgatgggttcttagagccttagcagccctggatggtggccagaaataaagggaccagcccttcatgggtggtgacgtggtagtcacttgtaaggggaacagaaacatttttgttcttatggggtgagaatatagacagtgcccttggtgcgagggaagcaattgaaaaggaacttgccctgagcactcctggtgcaggtctccacctgcacattgggtggggctcctgggagggagactcagccttcctcctcatcctccctgaccctgctcctagcaccctggagagtgcacatgccccttggtcctggcagggcgccaagtctggcaccatgttggcctcttcaggcctgctagtcactggaaattgaggtccatgggggaaatcaaggatgctcagtttaaggtacactgtttccatgttatgtttctacacattgctacctcagtgctcctggaaacttagcttttgatgtctccaagtagtccaccttcatttaactctttgaaactgtatcatctttgccaagtaagagtggtggcctatttcagctgctttgacaaaatgactggctcctgacttaacgttctataaatgaatgtgctgaagcaaagtgcccatggtggcggcgaagaagagaaagatgtgttttgttttggactctctgtggtcccttccaatgctgtgggtttccaaccaggggaagggtcccttttgcattgccaagtgccataaccatgagcactactctaccatggttctgcctcctggccaagcaggctggtttgcaagaatgaaatgaatgattctacagctaggacttaaccttgaaatggaaagtcatgcaatcccatttgcaggatctgtctgtgcacatgcctctgtagagagcagcattcccagggaccttggaaacagttggcactgtaaggtgcttgctccccaagacacatcctaaaaggtgttgtaatggtgaaaacgtcttccttctttattgccccttcttatttatgtgaacaactgtttgtctttttttgtatcttttttaaactgtaaagttcaattgtgaaaatgaatatcatgcaaataaattatgcaatttttttttcaaagtaaaaaaaaaa

SEQ ID NO: 4 - protein, 492 aa, Homo sapiens
MALNSGSPPAIGPYYENHGYQPENPYPAQPTVVPTVYEVHPAQYYPSPVPQYAPRVLTQASNPVVCTQPKSPSGTVCTSKTKKALCITLTLGTFLVGAALAAGLLWKFMGSKCSNSGIECDSSGTCINPSNWCDGVSHCPGGEDENRCVRLYGPNFILQVYSSQRKSWHPVCQDDWNENYGRAACRDMGYKNNFYSSQGIVDDSGSTSFMKLNTSAGNVDIYKKLYHSDACSSKAVVSLRCIACGVNLNSSRQSRIVGGESALPGAWPWQVSLHVQNVHVCGGSIITPEWIVTAAHCVEKPLNNPWHWTAFAGILRQSFMFYGAGYQVEKVISHPNYDSKTKNNDIALMKLQKPLTFNDLVKPVCLPNPGMMLQPEQLCWISGWGATEEKGKTSEVLNAAKVLLIETQRCNSRYVYDNLITPAMICAGFLQGNVDSCQGDSGGPLVTSKNNIWWLIGDTSWGSGCAKAYRPGVYGNVMVFTDWIYRQMRADG

SEQ ID NO: 5 - DNA, 27947 bp, Artificial Sequence
  Recombinant polynucleotide
gcagagtctaagaaatcgctgtgtttagccctcgccctgggcactgtcctcacgggagctgctgtggctgctgtcttgctttggaagttcagtaagtgcagggagcctcgatcccaccatgtgctcctgcagtccccagtgctctgagccagaccctgctctctgggctattgagacctctggaggccctccgtgaggttcctctcttacataacgaggctgtctctcttcccttctcttgtttagctatgagattgacacatcatggggaaagcatttagaatgtacccagtgctttggggtgcttggtgccacccagcactgtgagcacaggttcttctaccttggggccacacccagttacctgtatctcactgcacagcagtggctgttggggaccaggcccacccctccatgtcccacctcctgcaactgcagcctgagccttcccatcagcctggggtggtgcagacccatgtgccattgtggatccttcaagttacctgtgtggcagagaggacgtgtgagtgccgtccaaacccaaacactgagagggtccttcccattgcccccacggaagtaaggtgccccagtgctaattccacttatacttgctggtggcaaggacacttctcctccttattaaagtgggggattggctgggtgaggtggctcacgcctgttatcccagcactttaagaggccaaggcaggtggaccacctgaggtcaggagtttgagaccacaagcctggccaacatgttgaaactccatctctactaaaaatacaaaaattagtcaggcgtggtggcgtgcacctgtaatcccagctacttaggaggctggggcaggaggatcacttgaacccaggagttggaggttgcagtgagccaagattgtgcccctgcactccagcctgggtgacagaatgagacttcatctcaaaaacaaaacaaaacaaaacacagtggggccaggagttggaggctgcagcgagctacagtaatgccacggtgttcctcactccatgaggctcattgcgtttctcagcctgaagggcacctctcttctgttttctctgcaagtgggcagcaagtgctccaactctgggatagagtgcgactcctcaggtacctgcatcaacccctctaactggtgtgatggcgtgtcacactgccccggcggggaggacgagaatcggtgtggtgagtcagccttgaccttgggaagggactcctctgctcaccttggagacagcagccgggtccaggggcctttgggtgactgggcctggcgtgcgtccagtacgctgacacatgatgtcattgaatccctgctccaggctgagccctggggctcagagaggttgtgtttccggcccaacctcacccagcaggtgggagatgacagggccaccgaggactgtgtcattggaaccacacgtgctctgaactgccacaggaagtcagttaagatgagcaaactgtttataaagttggagatgcaggctaggaacggtggctcatgcctgtaatcccagcactttgggaggccgaggcagatggatcacctgaggtcaggagtttgagaccagcctgaccaatatggtgaaaccttatctccactaaaaatacaaaaattagccaagcgcggtggcgggtgcctgtaattccagctattcaggaggctgaggcaggagaatcacttgaacctgggaggcggaggttgcagtgagctgagatcacgccactgcattccagcctgggagacagagctggctcaaaaaataaattaattaattaaaaacaaaattggagatgcactatgttattttcaaaacaagctgcctttaaagatctatctgttgtcacagggtgggctcatctgtttcattttattttctgtggtttatctatttattcattttaatgaactaggaagcattgctcctatttatggcataccacatgatgtttggatacgtgtatgcctgtggcatggctaagtcaagctagaacatgggccttacctcatatacgtgtcttattaagaacacataaaacctactcttgtagtgattttcaaatatgcaacatatagtttattaactgcagtcactatgatgtacaatagattgctcgaacttattcctcctgtctaactaagattttgtgacctctgaccaacatctccccagtgttgtcaccccccgcccccagcctctgatagctgcctttctactctctgcttctgtgagtttgatgtttatacattccacatgtaagtggcctcatgcagtgtttctgtctctgtgtctggcttgttcacttagcgtaatgtcctccagcttcatctatgttgttggaaatgacaggatttccttctttcttgtggctgaatagtattgccttgtgcatatacaccacattttctttatcccttcattcactgatggactcttaggttgatgtcatgtcttggctgttgtgaaaaatgccgcagtgagcgtgggcgtgcaggtccctcttcaacacacggatttcctttcctttggatataaacccagcagtgagattgctggatcacatggcagttctgtttctcaccttttgaggaaactccatactgttttccataatggctgtagcaacttccactcccacccccacggtgcaaagtctccatttctcttctacaacctcaccaactcctgttattttccatctttctgatagtagccatttgaagaggtatgagatgatacctcattgtggttttcatttgcatttttatttgtatttttcatgaatttttgagggtgatttcaagggtagttagtgactcgaacagggaaacgatcctgagtatgagggttgtgctaatcatccccctcctgccagctgcgtacggaatggggctctgcagatggcagggagctggctcgtttctctttaagagctgccttttacttttcttcctcttcctttaaaacttatttcctggccggacgcagtggctcatgcctgtaatcccagcactttgggaggccgaggtgggcggatcacgaggtcaggaattccagaccagcctggccaacatggtgaaaccccgtctctactaaaaatacaaaaattagccagacgtggtggtgcgggcctatagtcccagctactcgggaggctgaggcaggagaatcacttgaacctgggaggagggggttgcagtgagccgagattgcgccactgcactccagcctgggcgacagagccagactccatctcaaaaaacaaaaaaaagttatttcccaagcacagccatgtattccaggcttgtggatcagcgttggtggtggtgtgtgctctcatatcttagttccagctaagcacactctgacatgtttacactagaaccatttgttttttctagaaatagaaatttcagaattgtagagtcagaggacttaccagaaatctcttaggtagttctcctcccctccctcaagtgcagtcctaacctcctggagttttctgtagaaaccacaagcctcagagctggccgagaattctagccaaagatttttccatgccaaagtaatcccccctctcctaagggccatccttggtggggactggtttcctgttaagccctcgctgtcagtcctggctgtggaatttcctggtgaggagcactggcccgtggagctcggccctcgtgccggccttgagcaggcccaagtgttccgtgttcttgatacctttcctccagcacagtcttgcttcccagaaaaaggtttgcacttgaaaatgatgcatttgctgattaaacatagttcttttgctttatttggtttctaaaataaagtgggagtttttgagattgagtaacgtgaggttaagatagcacgtggaatggctttttcttttctttctattttttttttttttttcctggagacagggtttcactctgttgcccaggctggagtgcagaggcatgaccatggctcactgcaacttcgatgtcctggggttaagcgatcccccagcctcagccccccaagtggctgggactacaggtgctcgccaccacacctggctaatttttgtattttttgtagaaaatgggtttcatcaatgttgtccagactggtctcgaactcctgacctcaagcaattctcctgcctcagcctcccagactgctgggattacaggcgtgaactaccacgcctggcctggaatggcttttgatgttctcctatgtgcacatgtgggtgaataaacaccaacaaagtccttatgttacctgaagagttgctctcttcttaatatttaagtcgtatttatttaaatactttaatagttgtacactattaaagtattattaggtcaaaatcaaggaagtacaaaagggtatgctgtgaaaaatctcttcttccttgctctgcttacttacctaccccgcatccccccatacaccccagacacacacacacacacacacacacacacacacacacgcatcactcccatacatgcccacctgtttaccagccaatcacatttcttggggcaactcatctgagttgcttctctttccagagagtttttgcataaagaagcacaggtatttctgcgttaccatgaccctatttcccagtggttcctagccagttgactctcctgcactggataccatcctggacagcattccttagggaaatgagccccctgttttttcccaccatggcacagttggtcctttgcatggacgcaccattattgcccctgtctcttcttggtggaccttaaggttttctccatccttttgctgtaacacacactgctccaagtgtgtgagcatatcagtaggaaacgcttccaggagtagaactgctaggtcagagggcgtgtggatctgtaacctgacagacctagaccggcttcagtttggttttatccagtttccatattgattattcatataaaaggaaacagacaaacataacgctgtgcatgtattctctcttagaccagaacaggcatagggtgcacttttaatttgtccatttcgtagagtagaaattgtttttgctgaaatgaacaccttaggatgctgaagaatatgacccgtcccatggaaaacattcaaaaatgtgtgtagcgctttcttcccaagggtgtgtgtgcgcatattttaacactaattcactttctacttccgttgctatcctttctgtgagtctttctcagaatctcagaaaagaaactaaattgttcactctagttatcaatgctgtactctatacctggaatttgctaaaagggcagattttaagtattctcaccacagaaaagagaaaagaaaatggtaattatgtgacgtggtggacatgttaactagctttattatggtgagcatttcacagcggatatccagtcatcacgctgtacacattaaacatgtacaattgggtttttttgagacaaggtctccttctgtcacccagtctggagtgcagtggctcagtcatggctcattgcagcctcgacctcctgggctcaatccatccttccccctcagcctcctgaaaagctggggccacaggcatgtaccatcatgccaggctaatgcatatatatttatattttttggtggagatggggttggtctcgaactctgggctcaagtgatcctcccgccttgcccttccaaagtgctgagattacaggcatgaaccacagcaccaggcctacatgtaaaatttttatttgtcaactatactttgacaaagctgagaaaaaaaatcctaatatttaaaaaaaaaaaaaaaaggactagcttgagaccttttccagctctctggcttatcagctgccgtctcttccgggtgcagatagctggaagggaaagaaaatccctaaaattacccacaagccaagaatgaagtgtctccctttgagccacagtggcagttttgtttttaatcatagaagtgtattttgagccgggtgtgctggctcacgcctgtaatccccgcactttgggaggccgaggtggggggcggagggggtggggatcgcctgaggtcaggagttcgagaccagcctgaccaacatggagaaaccccgtctctactaaaaatacaaaattagccggcgtggtggtgcatgcctgtaatcccagctactcatgaggctgagtcaggagaatctcttgaacccaggaggtggaggttgcggtgagctgagatcatgccattgcactccagcctgggaacaagaaaaaaaaagaagaagaagaagaagtgtattcatttcagttacttttaaaaaagtgaacagactttatattttagagcggttttaggtttacagaaaatgaaacagacagggcagcgagctccttgtactcctccccagcacacagttgccctgttatgaacatcccacatcagtgctgtgcgttcattaacaccgatgaacctgatgcatacattatgatgaactgaagtcctggacttcaccctttctcttgtacagttctgtgggatttgacaaatgcataatgctgtacagccacaatgatagtatcgtccagagtagttctcctgccttaaaacctcttttgctgcacctgtttctctctccccactcaccccagctatctgatcttcttagtgcctccgaagttttggtcttttcaggatgttgtagcgttggaatcatggagtatgtagccttcaccacatacaccttccttcactttgttggcttcctttacttagtaatatgcattcaagtttcctccatgccttttcatggcttgatagctcatttctttttagcaccaaataatattccgttgtccagatgtagcacaatgtttatccattcatgtaacctgtgaccgactcacagataggatgtggaatcactcaccacagaggcattagacaataatcagacccaagtcatttcatgggggaacaagcccacaggtaccagactgtccagtgagtcagggccactcgtaggaagtaagaagagaggctagagcatagccaggtcctcactttatactttaagcccatgtgtatttctcccaaaccacacagcattgtttccatgctttcagctttgcatgaataacgtgatacttgaacgcatcatttatcacttgctctctttcccacagcgctgttttcaagcttcttcctgttcatgatgctctgcttaacccttaagctgcatgggattctgttctgtgaatacgcccaccccatgtattatcctgcccagcaaaaagtccccaaaactctggatggtggttacctctagggagggagagaagagattgggaatagggagcgacttcaacggtgtttgtaatgttttgtttctttaaataaaagagctgagatcatttcagcagaatgttgatttagagtctcctggacaatttgttgctcaaagtgctctcttaaagagcactttaaaaaaaaaaaccttttatcttattatttatttatttatttattgagacggagttttgctctgtcacccaggctggagtggagtggtgtgatctcagctcactgcaacctttacctcctgggttcaagcaattcccctgcctcagcctcccaagtaggtgggattacagatgcgtgccaccacacttggctaatttttgcattttagtagagatcggtttctccatgttggccaggctgatctcaaacgcctgacctcaggtgatctgcccgccttggcctcccaaagtgctggtattacaggcgtgagctaccatgcctggcttatcttatatatttttaaaaacagcttattgagatctaatttatgtaccataaaattcaagtatataattcagtgcttttatatataaaacatatatatgaaatagcttattgagatataattttttatataaaacagcttattgatatgtaatgtatgtaccataaaatttaaatatataattcactggcttttatatattcacgaatatgtgcaactatcaccacagtcaattttagcatattttcatcagctcataaagaaaccccaagcccttgaactatcaccccatatccctcctcccagcccgtccctcctactcataagcaaccactaatctacttagtgtctatagatttcctactctaggcattccatgtgagcgggatcatgcaatacgtgggctcacacaatataagtggcattccatgtgagtcggctcatgcagtatgtccggctcctttcactgagcataaggtcttcagcactcatccaggttgcagcctgtgtctgaatttcattccctcttctggctgaatcgtattccattgtgtatcttggacatatcctattctgctcacccagccgttggtgggcgtttggagtgttttcgcctttcagctgttttaagagggttgcagtgaacatttgtacaagttttggacccaatgcctgttttcaattctcttgtgtagagagcactttttagcagaaaaagaatagatttgtggcctccctttgtgtgcggtcagtgccttgagaagagtgaactgtgctgccacctccggagccgtggagagcgcggggcttgggtagcagctaggacgatacaagttgggacaaggccaggtgcaatggctcacgcctgtaattccaacactttgggagaccgaggcagggggatcacctgaggtcaggagttcaagaccagcctggccaacatggtgaaaccccatctctaataaaacagaaaaattaactggacggggtggtggacgcctgtaatcccagctactcgggaggctgaggcaggagaatcacttgaacctgggaggcggaggctgcagtgagtggagatcagaccactgcacttcagcctaggtgacagagcgagactccgtctcaaaaaaaagaaaaaaaaagaaagaaactcatggataatcctccctctcgtgcagttcgcctctacggaccaaacttcatccttcaggtgtactcatctcagaggaagtcctggcaccctgtgtgccaagacgactggaacgagaactacgggcgggcggcctgcagggacatgggctataagtgagtatggggcagcacccgccgagtgacagtaacagacagcagaaacacgagaagaccctctctctgcctccctgtgaaagcaccggcacatgagtgctggggacaattgtcaccttccaaaagctgagccctataaccagcaggtggaatttgtcctgctagggctgtgcccagcacacagaccttggctcactgccaccttgccctgcctcctccttggcctctatagactcctggttgctcgggagtgcccagtgctgtggtcatctggtcagaggggtaggctgagggcgttaggtgcctctttttccaaggtgcctctcagccagggtccattcacctccctgggtagaggttggaccagaacagctggcgaggagggttgggctggggagagcagcagagacaaatcctgtgccagtttcacttcattcgggagccatggaagccttttgagctggggagagaatcaatcaatcagactgatacttaaaaaatgtcattcctgctcgtagctctgagggaaggtgggaaggcttaacagggtgtgtgtcgcctgacagtgattcctaacgggggtggggcggtggttaccatttaccagcactgcctggggagatgcggcagccctcaggcatcgggggagagggtggtaggatgctactgccactttgttttccatgggagggtccccaggtgatttctatgcaactttagggtattcaatatgccagttttcagaatgaattaccactcggtgagaaagttggcatcttagctagtcactgtgacatccctaaacagcaggggtgaattacacagcaaagcccccccatcacagtccaggaacctggtggaattgataactggggccatgttaacatctgtaccttttattagattaaatgtgtgtatgattatacaatcctatgtccttctcatagtttcttgatcctaacctggataagaaacacgaccaatgaaggaattttgtctgacactttagggttattgaatcgaaaaatcgttacaatattctagcacttggttagaacgtgtgattttttttcctaaatgctaaggtttttccctcttattctgaatgtcgtatgagcggtattatgacatagtataggatttgtgtttgcttatgccttaaccattatcacaaataaggttttcttttttaggaataatttttactctagccaaggaatagtggatgacagcggatccaccagctttatgaaactgaacacaagtgccggcaatgtcgatatctataaaaaactgtaccacaggtatgcagcaatttcttcttgaaaaattttggaatgaaatcaactaggagacaccatggggaatcgttgtcctgagtctgatttctctgagctgcaatactcggtctggatgggttttgcattgggaggagattagagtctgaccaggcctggttactctaagcagcccttggtttattcataggaagtggctgaggtttctctgctatttcattttcagcctctaccgtctgcccttgttggtagcggctcacacttgcaacatcgacattcaactctatttagttttctttcctcttcagacatttagaggtgtacctattttgtcagggcgtggttctaggaatccaagataatgtctcagtgtcccagccagggtgaccggctcattccagtttgccagggacttcactggcttgagcaagggaagtcctgctccattccaggcagctgggctggctggtcccgttagccccaaccccgggacagcagtgccagagggtgctctgtgagggatgggcagcattctggcggcctgggaatgagttgtggtgtttccagggggtagaagtgggtacaagccacaggtcacatgatgagtggctgacctggctgggagggcagaagaggggatggacttaggctcttccttttgctttgcacatatttaggatgtttgcagacttgctatgattgttgctgttatgtgttttctgatgtgaaagatacacagtgtcctttgcccatgagctctccttgcctcccaggtccccagggcttatgcctggtgtctaggcatcacctccctgcctgccaggtgccaggtgctgcatttcgggggaggatgaactaatcaccccgcgccacctttcctctgagtgggagcctggggcaggtttgcattcctggaggccgctggtggaggggtctgggggcctgacttccactgcagcctgctgtcctggggaatgtggcagggcaagcccagtggggagggctgtgcacggccaggtgcacccatcaaaacagcagggctgcggtttgtccctgtggagaagctaaacacagctgcctgggcactttgtaaatgctgagtggttctttgtctttctgggttacacacggaatcagggagccaagtccagccgggcagggacggggggaggggaggaggtgctgccgtcccttggcaagagccttgggaactcacaaggaggctggagggcttggaagaaagaagagaaggccattgtctggtaggctctattctatctcggtggtggtggtggggggaggcgcacttcttttcctctttctgtgcagcagttgccctttgatgcctgagttcttggcttgttttctgtcgggcttctgtgaataaccacatgtgccctggcgctgtgaccacacagggctatccctaccgaccttaggattcttaggaaatgtcttctcttaaaggggacatgtcttcacttggccgtgtcagtgccccagagccagagtccacctggaatgcacctgtagtcactgagaacccggggggtgtgccttagtaagaaggtgtcaggaaggacctattattgtagggcctgggctcctgcaaggtggtttgggggtggttggaggaagcagagatttgctctggattggatgctgtcaggaagcaggggtaattctgtgaggctgctttattattttttttctaggaggaggttggaatgaggctaggctaaagctgtgattggtaaagaaacgtccgtcgctcaagttagccaggacaggaggagacatcagatcgtgattttgtggttgtgagcacaaggttcctgttctgtctgttcagacatcatttcggaggaggctccttgtgtcttgccccatctcaggcatggaggggcctagtccgatattgacgctcagtgaaataattcaggttccgcagagcacacggcccagctatcagggcgggccagctctgcatgccaggggccgcgtcttcccttctcagcatagcctgggaaattcactgcaggacaaaatgcatcagttacttcctcttcatccataacctgggatgtttgactcccaaatgagtaactcttacgtttcttctaatcctagggaaactattggttatattgctttcaacactacaaatttaaagcagttataggagcccagaggtttccaaatggcttccttaaaaattagaagatgattttaaattccaagaggaaaaacaaaactagcattattgtatacttaccctcacaaccgtcctaggagctggtacaattttaagagaggttaagtaacttgcccaaggtcacactgtggggatgtgagccgcgtaccttggctcagtgtctggtctttgccactgtccctatatggatttacttaccttattggagttgtaactagcagacccttctatgtctcagaagacaggagagggaacatcggaagaaatgactgatttctaagcatgtgagaggcaggtgactccgcactatcgtgaccagaatttcccctgttctttttgcagtgatgcctgttcttcaaaagcagtggtttctttacgctgtataggtaagttcatctggagtcccccttttgatacttctaactaggaaaagctctctactttcagaacagtactccctgtgtctctgggggcgtgggagggaagaaggtggggtcacgggttggaatgtgcccagcggcgtctcgctctttccaaggagctcctggtttagatttccatggcctgtagacaccttcagccttgggtccaagggacaccccctgagatcaggcacgctcaagaagctgacaaagccctacactttatgccacccatgagctggaggcccggcaggtctctttctccagaaagcaaaggggggtggcgttagtgagccctggcagccacctaacgtggacttggagcatctgcggggctgtggtccagcaccaccgtgtggccaccaggtgctcatcagccagtgggacccgggaggagggacaagaccagagaacaacagtgctcttgcctcttctctcctgaattttggacggtggcttagacttgggtgtccccatctctgtgtttagagtgcttacagtttccaaactgtttgcaaatgtggaagccaccgtccctctcctctgggatggcccagtgctgtcgtggggccgtggtcctgagctcagcttttcatttgaagaggtggaaggagctgacaccgtcccatcccggcagggctggctcaggtcttctttaggtcctgagtgggggtccagcacagccccaagggtgcgtggcacccgccctgccctctgcccatgcactcatctcctggtggagaagacactcacacacaggaagcagggaaggcagcagacctcactcacccctcaccccctcactcaccccctactcaccccctcaacctctcattcaccacccaccccctcgccccctcactcaccccctcactccctcaaccctcactcacctcctcactccctcaaccctcactcacctcctcacctcctcactctccccctcatccctccctcaccccaccccgtcacctcctcactcacctcctcaccccctcactcacccttcaccccctcactcaccacctcacctcctcactcaccccctactcaacccctcattcacccctcaccccctcactcacccctgcaccccctcactcaccccttcatccactcacccacctgctcacctcctcactcaacccctcaccccctcactaatccctcactccctcaccccctcacgccctcactcacaccttcacctcctcactcaccccctcaccccctcaaccccttacttaccccctcactcatcccttcacccctcactcaccccctctctcacccattcaccccctcactcatgccttcaccccctcactcacctcctcactcacaccttcacccctcagtcaccccctcactcaccccttcaccccctcaatcatgccttcactccctcactcaccccttcaccctctgaattactccctcatcccctcactcaccccctcactcaccccttcaccccctcacccaccacctcacccacccctcacccaccccctcacctccttacccctcacccccctcactcacccctcaccccctcactcaccacctcacccacccctcacccaccccctcactcactccctcatcccctcactcaccccctcaccccctcactcaccccctcacccacccctcacccaccccctcaccccctcactcaccccttcaccccctcactcaccccctcactcaccccttcaccccctcactcaccacctcacccacccctcacccaccccctcactcactccctcaccccctcactcaccccctcaccccctcactcaccccctcatctcctcactcaccccctcacctcctcactcacccgctcacctcctcactcaccccctcgccccctcactcacccctcaccccctcaccccctcactcacccctcaccccctcgccccctcactcaccccctcgccccctcactcacccctcaccccctcaccccctcactcatcccctcacctcctcactcaccccctcacctcctcactcaccccctcacctcctcactcaccccctcacctcctcacccaccccctcactcactccctcaccccctcaccccctcactcaccccctcacctcctcactcaccccctcacctcctcacccaccccctcactcactccctcaccccctcaccccctcactcaccccctcacctcctcactcaccccctcacctcctcactcaccccctcacctcctcactcatgccctcaccccctcactcaccctttcacctccttgctcatcccctcacttaccccctcacttcgtcaatcacccccccacctcgtcaatcaccccctcaccttttcactcaccccctcactcacccccttacttcctcacttacctcctcaccccccactcaccccctcaccccccactcaccccctcaccccacactcaccccctcaccccccactcaccccctcacccctctcacctcctcactcaccccctcacctcctcacttatcccctcaccccctcaattaccccctcaccccctcaattactccctcatcctttcaattacccactcaccccctcacctcctcactcctcactcactccctcactcaccccttcaccttctcactcacctcctcgtctcctcaccccctcactcacttccagccctgcccctcccatcttccttttctttgtgtgagaatctggggtccctgagtggtgtcagtccctccaagactcaaggagtccccagggccttgttatccagaacacccccacctgggtcccgggagaccccatgggatcacaggagtgttcagggaagtggtgcttcctgggtctgggtgggctggaggggcatcctcccttccccaagaggagacccccaggagccccctaagtccatccccagcagtggtgcccctgccctgtccttgcagcctgggagacccttgggaggggcgggcgctgggtggctgggcggcttctgctggtctcaccccactggcctcctgtttgtcatcctcagcctgcggggtcaacttgaactcaagccgccagagcaggattgtgggcggcgagagcgcgctcccgggggcctggccctggcaggtcagcctgcacgtccagaacgtccacgtgtgcggaggctccatcatcacccccgagtggatcgtgacagccgcccactgcgtggaaaagtatgccaggggcggcgcgggccgggtgggggctcagggctggcctacagccaccctgtgaccttgagcaggtctcaacccttgcagccccggcatccttgtgtttaaatggggagagtattgcacctgcttcctagggctgtgagacatcaagtgcgctcatgccaggcagtgcatggctgtatgcactgagtgtcccctgcacgcagggcacagggtgcaggtggaacattctccacgatgtcgccgtgaccagcgttccttccagccactgtcctctgagctctgtcctgcccttgagcaaagcccctgccccctgaggtatcctgtctccgggacgctagtcccaggagagggcacactcagacaggcttcaggctgccctgctggaaggtccctggggttaagcgttcttggccacagcattgctcatgcagagggttaggtaggggtgaggctagccgtgacagtattagcatttatggacgctaccaccccctccccttttccttaaacacatagtgcttttggtcacatgctgctttggaggaggcctcacttggcggatgtatttttctgccttagagagaggctgaactgggtttgactgttggcccagccctctcttgctgcgtgcccttagacgattcactcaacgtctctgatccatggcatgtacaactataagatgggcatgcccttctcctctcgggctgttatgaaggtcaaggaagcaagggctgttacccaagggtgctcccttctctccccctcttcacacccccaggtgctctgggccctctaggaactgggtttctctcaagggctgttacccaagggtgctcccttctctccccctcttcacaccactgggtgctctgggcccactaggagctgggattctcttaagagggaaactcttggataaaggaaatggtttgattgatatcggacaagtctgttcattagtatccatttattaagcacctaccatgtgccaggaaatgctttggcgtacaaaggaaaataagggccagtcctgctagaaatggccttgaaaccccagggagggatgtcggcccattgtgggtgctgcagattccttgaaggtgatgcaagagccagaaagaaggatgatgtggggggctgaggcagggagtcggggttgggggagtgtgggggagaaggggagaccgagcacctcttccactatctccctgtgtggtttttggtgaaccatcctgcctctgggtgtcttgcctccagcttctgacgttggaagttcatccactgagagctctgtgtttatggctctgagatactgagtccttcttctctcccagacctcttaacaatccatggcattggacggcatttgcggggattttgagacaatctttcatgttctatggagccggataccaagtagaaaaagtgatttctcatccaaattatgactccaagaccaagaacaatgacattgcgctgatgaagctgcagaagcctctgactttcaacggtacgtgtggctcaggcttggcaagcaggttggcagaatcttaaagagatgttgattggaaatgacacttgtgctatgccaaatggaagggaggcatttgcgttgagcgagggtagcgtgcagcgggtggccaatgggagaggctcacagaggctaagagcacctgccgcattttgggggaggcagcagccaccacatctgttctgtactgtactgagtggtggtgattcaagccaggcatggaaaaggctagaacagggctttcccactgcagcacccttgacatctgggtggttctctgttgtagggctctcttgtgccttgtaggatgtttaacagcgtccccagcctctacccactggaggccagtagctaccaagctgtgacaaccagtgttgcctgctgacattgccaaacatccgctttgaggcaaagtcacttccagttgagaactactggcctaaaatgtgtaaagatccttgatttttaaagatacattctaaaaccaagttgcttaattcaggacaaacatgctttctcttagcctcttattcggtcccactctggtccatccaagggtctggaatgttctagccccatgtggatacagaagaagcaaaacctcagccctccctacagcatgtctgtattcacattgggaaatggttcacatatagaagagcgaatgcctgagcaatggcgtggtgcctctggggcgaaagctgactccattgactccatcggctttttggctgttgcctcctgtgtgtctttcccgtcttgatcacctggagatatgtaattttggaagcagagctagcaaataattcctcttataagcagagctagcaaataattctacttataagtagcataacgtcttgcctgccagaaggagaggtctggcagggggagaaagtgagaatgtgggacttgttgggatgcagggtcctctgggcagggtggccagggtgccaggcccagcagcctgcatgtgggaaggccaggtggagacataggtgatacccgcctggctcactgtgttttctcttcttgaaacagacctagtgaaaccagtgtgtctgcccaacccaggcatgatgctgcagccagaacagctctgctggatttccgggtggggggccaccgaggagaaaggtgaggctgctcctgggcacacaggactgcagggcccacagatggagcattgggttcggaagtgggaggtccaggttttaatcccagttctactactcaatgactggatgactttggttgattcccccagtccttgtgcctcagtttctccatctgctaagtgggagaaatcctgcccagcctacctaatacactgtgttcttatcgtgatcacacagagcagcatgtggaatggcttttgaagtatctgggccatacgagtttagaggtgcaggatctcctgtgttgcactcattgtgagtttagagctgccctggagatcccaccaaggcctgcgtggctgagtgacagggggcttggtgaggacgggcatcctggacccatggtggccacatctaagcctgtcctctgccctgataaccacagagagaggctctctccacccacttcctttgcaatctgcatttctctctgacagtctttcaaatgaagggagcctggctgcttcatttttatggagggttggaagtgcttagtggcaggcacaaaggttcattttacatattgtttatatccttctcaaaagcgtctaggccatacagacaacaaatcctttcaaacaaggggaaaagtacaaaggttgggtgatttctggggagcgtcagggaaggtagtggggggcatcctggctcctcatcagcagaaacttactacagtagagccacaggctgggcaaaagacctcatggaatccaagatgaagggaatatcgacaaatatttgtgcgcacctgcacctagtacaggctgggtgctactcaggtgctgggaatgcagaagtgaacagagtaagacaaatgtctctgctgtcaggagctttacctctcttctggatgtcggtggtggggacggggcaggtgtggtcagacagatgggagacaaacaactgagcgaggtacttccaaacatctgagggtggggatcacaaggtcccggctattttgaaggggtggtcaggaaaggcttctcggaagaggtggcatttgagctgagactcaaatggcaaaaatgtgtacacatcaaaaaggctagtgcatgtatcttcaggtgtggtcaaggggccaaggaggtgggctggggccagattgcataggtccttgtggattatggtgaagacaccagcttctcatctgcttgaggtggggagatcgtgagccggggagtgccatgatctggcagctgcgtggggagtggggatgaatggatggagacgaggatgatggtgacaagtccattgctgtggttccttgagacaggaagccagctcatagcagagtgcgggcgtggatgtgaagagatgagggtacactagggctagagccaccagacttactgatgggttgcatgtctgtgggagagagagtgagaagtcagggacgatggctttccactctgtggctgaagccccagggtggcgggtggtgccatttttcaagccaggaaatattggttggtgagaatttggggtgggagaaggtgtgacggagggttctggttttgcacactaagcccacggtgcccagaagatgcccgaggggaggcagcaaagcgagagtgggaaatgcagaggtggcaagtgcaggccgtgtcttgagaagctctaatgtgcaggggagccgagaagcaggcggcctagggagggtcacgtgtgctccagaagagtgtgtgcatgccagaggggaaacaggcgcctgtgtgtcctgggtggggttcagtgaggagtgggaaattggttcagcagaaccaagccgttgggtgaataagagggggattccatggcactgatagagccctatagtttcagagctgggaatttctttccctgaagctgaactccagagctgcattcagcacaggcaccgccagttgtaaggagaatccaggtttcccaggagaggggttggtgctgggatgagctgaccggggcagggctggaaaatagggctgtgaccatctgtgtagtgcgtgtggaggtctcagggagggaagtgtgctctccctgcgagagctgcaggcaacactgggagctcaacaagtctccctgtccttagggaagacctcagaagtgctgaacgctgccaaggtgcttctcattgagacacagagatgcaacagcagatatgtctatgacaacctgatcacaccagccatgatctgtgccggcttcctgcaggggaacgtcgattcttgccaggtaattcaacatttttattctacctttggtccttaccagatcctactgaaccccccatgagagagagggcattcttggggtcagcagagcctcctcagtgacacggagccagctcggggcagtcatgggaagtgacggccacaaacagtgcgaacgcttctggtggcagaaggaagtacagtcaacaaatcacacacaccctctgaaaaaccggtatttggtaaaagtgccagtggaacagaaacaagtatttagactattttaaattatgaacggcaatttatttagtaacttttagcttgaacagattaaaattcaggatgggggctatctctttgggggttacatctctgttaccatcaccccttgatggtggagattcgaagcccacacagtcactcgtaactcacactgcgacccccgccccccaactcctctaggcctggtcagtggtgtgcggcagattgtgacttgattttctgctctctgtaccttgctgtgtcccacagggtgacagtggagggcctctggtcacttcgaagaacaatatctggtggctgataggggatacaagctggggttctggctgtgccaaagcttacagaccaggagtgtacgggaatgtgatggtattcacggactggatttatcgacaaatgagggtaactatcctgtcctccttctgactgtgttctccgattcctcgagccaaagccagacatctgttaggcgtggttctgctgctggaagctgactggtgaccactggtcagcatgaagcaaactctgcttcctccagccacagccccatccccccagtgtccacccattgcccattgcctctcactggcttcacttgcatatttcccctggtgtttggatgaaaagcgctggggctcagcttgtgtgaaattccttggtgctctgccaaccacacttcgttctggctcagctgactcagctgttccacccaggccacctcacatcaaactttttttttttttttttgagatggagtctcactgtgtcgcccaggctggagtgcagtggcacaatctcgactcactgcaacctttgcctcctgggttcaagtgattctcctgcctcagcctcccaagtagctgggactacaggcatgcgccaccacgcccagctactttttgtatttttagtagagatggggtttctccatgttggccaggctggtctcgaagccctgacctcaggtgattcacccacctcagcctcccacagtgctgggattacaagtgtgaaccacggtgcccggcctcacatgaaacttttgatttatagagagcagagggaagagccggctgtgcccatccttttctggggccatcgagtggctcctgggcagcccccaaggttaggaagggcaggagcagccagggttctctgatgccccagactcaagcacgagggaaggtctcaggggttccatgtgagcctcatggatgtctctgcttagcagagccctggctttgggcattgtccagatagggggtgagaaccagatcttctcatctccaggacctcagacgtatagttttctcagatttctgtgctttctggggctgggctactagtggaagaaagcagtctattctgtcttctcccaaatctcccagatgcccagtctgttgaaggaggagcagaaccagggggcctttcccgctgaggcccgacctgtgtctccttcaaatgacacgcgggactcagggccttcccatgaccatggggcccagggggcgtcacctggcccagggcccagtgctagaaacagatgaccccaggaggaggaggcagggcaggagggaagctggcagggctgggatggtcagccaggctgaggggcggactcgcaccaggatggagctaggaaatgatccaggtgtgtttggcggctgcaggtgggtccgcatggctgtgcagggagggaagggctgcgtggcaggagagcagccgggggaggcccagactctgctgaagagatgcctgttgtgccggcctccacatccgctgcccgctccttccggagctcctgccccgccatgctcagcctgactctgaccaacacgttggagagaagaatgatccctttgtgctattaagcttgcttatttggtttctaagtgcttcatgcgaacctagaggaaaaaattattttccacctttgtttgtcttaagaaaataacacacttttttttttcctatttgaacaggcagacggctaatccacatggtcttcgtccttgacgtcgttttacaagaaaacaatggggctggttttgcttccccgtgcatgatttactcttagagatgattcagaggtcacttcatttttattaaacagtgaacttgtctggctttggcactctctgccattctgtgcaggctgcagtggctcccctgcccagcctgctctccctaaccccttgtccgcaaggggtgatggccggctggttgtgggcactggcggtcaagtgtggaggagaggggtggaggctgccccattgagatcttcctgctgagtcctttccaggggccaattttggatgagcatggagctgtcacctctcagctgctggatgacttgagatgaaaaaggagagacatggaaagggagacagccaggtggcacctgcagcggctgccctctggggccacttggtagtgtccccagcctacctctccacaaggggattttgctgatgggttcttagagccttagcagccctggatggtggccagaaataaagggaccagcccttcatgggtggtgacgtggtagtcacttgtaaggggaacagaaacatttttgttcttatggggtgagaatatagacagtgcccttggtgcgagggaagcaattgaaaaggaacttgccctgagcactcctggtgcaggtctccacctgcacattgggtggggctcctgggagggagactcagccttcctcctcatcctccctgaccctgctcctagcaccctggagagtgcacatgccccttggtcctggcagggcgccaagtctggcaccatgttggcctcttcaggcctgctagtcactggaaattgaggtccatgggggaaatcaaggatgctcagtttaaggtacactgtttccatgttatgtttctacacattgctacctcagtgctcctggaaacttagcttttgatgtctccaagtagtccaccttcatttaactctttgaaactgtatcatctttgccaagtaagagtggtggcctatttcagctgctttgacaaaatgactggctcctgacttaacgttctataaatgaatgtgctgaagcaaagtgcccatggtggcggcgaagaagagaaagatgtgttttgttttggactctctgtggtcccttccaatgctgtgggtttccaaccaggggaagggtcccttttgcattgccaagtgccataaccatgagcactactctaccatggttctgcctcctggccaagcaggctggtttgcaagaatgaaatgaatgattctacagctaggacttaaccttgaaatggaaagtcatgcaatcccatttgcaggatctgtctgtgcacatgcctctgtagagagcagcattcccagggaccttggaaacagttggcactgtaaggtgcttgctccccaagacacatcctaaaaggtgttgtaatggtgaaaacgtcttccttctttattgccccttcttatttatgtgaacaactgtttgtctttttttgtatcttttttaaactgtaaagttcaattgtgaaaatgaatatcatgcaaataaattatgcaatttttttttcaaagtaactactgcatctttgaagttctgcctggtgagtaggaccagcctccatttccttataagggggtgatgttgaggctgctggtcagaggaccaaaggtgaggcaaggccagacttggtgctcctgtggttctcgagataacttcgtataatgtatgctatacgaagttatatgcatggcctccgcgccgggttttggcgcctcccgcgggcgcccccctcctcacggcgagcgctgccacgtcagacgaagggcgcagcgagcgtcctgatccttccgcccggacgctcaggacagcggcccgctgctcataagactcggccttagaaccccagtatcagcagaaggacattttaggacgggacttgggtgactctagggcactggttttctttccagagagcggaacaggcgaggaaaagtagtcccttctcggcgattctgcggagggatctccgtggggcggtgaacgccgatgattatataaggacgcgccgggtgtggcacagctagttccgtcgcagccgggatttgggtcgcggttcttgtttgtggatcgctgtgatcgtcacttggtgagtagcgggctgctgggctggccggggctttcgtggccgccgggccgctcggtgggacggaagcgtgtggagagaccgccaagggctgtagtctgggtccgcgagcaaggttgccctgaactgggggttggggggagcgcagcaaaatggcggctgttcccgagtcttgaatggaagacgcttgtgaggcgggctgtgaggtcgttgaaacaaggtggggggcatggtgggcggcaagaacccaaggtcttgaggccttcgctaatgcgggaaagctcttattcgggtgagatgggctggggcaccatctggggaccctgacgtgaagtttgtcactgactggagaactcggtttgtcgtctgttgcgggggcggcagttatggcggtgccgttgggcagtgcacccgtacctttgggagcgcgcgccctcgtcgtgtcgtgacgtcacccgttctgttggcttataatgcagggtggggccacctgccggtaggtgtgcggtaggcttttctccgtcgcaggacgcagggttcgggcctagggtaggctctcctgaatcgacaggcgccggacctctggtgaggggagggataagtgaggcgtcagtttctttggtcggttttatgtacctatcttcttaagtagctgaagctccggttttgaactatgcgctcggggttggcgagtgtgttttgtgaagttttttaggcaccttttgaaatgtaatcatttgggtcaatatgtaattttcagtgttagactagtaaattgtccgctaaattctggccgtttttggcttttttgttagacgtgttgacaattaatcatcggcatagtatatcggcatagtataatacgacaaggtgaggaactaaaccatgggatcggccattgaacaagatggattgcacgcaggttctccggccgcttgggtggagaggctattcggctatgactgggcacaacagacaatcggctgctctgatgccgccgtgttccggctgtcagcgcaggggcgcccggttctttttgtcaagaccgacctgtccggtgccctgaatgaactgcaggacgaggcagcgcggctatcgtggctggccacgacgggcgttccttgcgcagctgtgctcgacgttgtcactgaagcgggaagggactggctgctattgggcgaagtgccggggcaggatctcctgtcatctcaccttgctcctgccgagaaagtatccatcatggctgatgcaatgcggcggctgcatacgcttgatccggctacctgcccattcgaccaccaagcgaaacatcgcatcgagcgagcacgtactcggatggaagccggtcttgtcgatcaggatgatctggacgaagagcatcaggggctcgcgccagccgaactgttcgccaggctcaaggcgcgcatgcccgacggcgatgatctcgtcgtgacccatggcgatgcctgcttgccgaatatcatggtggaaaatggccgcttttctggattcatcgactgtggccggctgggtgtggcggaccgctatcaggacatagcgttggctacccgtgatattgctgaagagcttggcggcgaatgggctgaccgcttcctcgtgctttacggtatcgccgctcccgattcgcagcgcatcgccttctatcgccttcttgacgagttcttctgaggggatccgctgtaagtctgcagaaattgatgatctattaaacaataaagatgtccactaaaatggaagtttttcctgtcatactttgttaagaagggtgagaacagagtacctacattttgaatggaaggattggagctacgggggtgggggtggggtgggattagataaatgcctgctctttactgaaggctctttactattgctttatgataatgtttcatagttggatatcataatttaaacaagcaaaaccaaattaagggccagctcattcctcccactcatgatctatagatctatagatctctcgtgggatcattgtttttctcttgattcccactttgtggttctaagtactgtggtttccaaatgtgtcagtttcatagcctgaagaacgagatcagcagcctctgttccacatacacttcattctcagtattgttttgccaagttctaattccatcagacctcgacctgcagcccctagataacttcgtataatgtatgctatacgaagttatgctagtaactataacggtcctaaggtagcgagctagctccacgtggctttgtcccagacttcctttgtcttcaacaaccttctgcaagaaaaccaagggcctgaattttaacttcctg

SEQ ID NO: 6 - DNA, 25333 bp, Artificial Sequence
  Recombinant polynucleotide
gcagagtctaagaaatcgctgtgtttagccctcgccctgggcactgtcctcacgggagctgctgtggctgctgtcttgctttggaagttcagtaagtgcagggagcctcgatcccaccatgtgctcctgcagtccccagtgctctgagccagaccctgctctctgggctattgagacctctggaggccctccgtgaggttcctctcttacataacgaggctgtctctcttcccttctcttgtttagctatgagattgacacatcatggggaaagcatttagaatgtacccagtgctttggggtgcttggtgccacccagcactgtgagcacaggttcttctaccttggggccacacccagttacctgtatctcactgcacagcagtggctgttggggaccaggcccacccctccatgtcccacctcctgcaactgcagcctgagccttcccatcagcctggggtggtgcagacccatgtgccattgtggatccttcaagttacctgtgtggcagagaggacgtgtgagtgccgtccaaacccaaacactgagagggtccttcccattgcccccacggaagtaaggtgccccagtgctaattccacttatacttgctggtggcaaggacacttctcctccttattaaagtgggggattggctgggtgaggtggctcacgcctgttatcccagcactttaagaggccaaggcaggtggaccacctgaggtcaggagtttgagaccacaagcctggccaacatgttgaaactccatctctactaaaaatacaaaaattagtcaggcgtggtggcgtgcacctgtaatcccagctacttaggaggctggggcaggaggatcacttgaacccaggagttggaggttgcagtgagccaagattgtgcccctgcactccagcctgggtgacagaatgagacttcatctcaaaaacaaaacaaaacaaaacacagtggggccaggagttggaggctgcagcgagctacagtaatgccacggtgttcctcactccatgaggctcattgcgtttctcagcctgaagggcacctctcttctgttttctctgcaagtgggcagcaagtgctccaactctgggatagagtgcgactcctcaggtacctgcatcaacccctctaactggtgtgatggcgtgtcacactgccccggcggggaggacgagaatcggtgtggtgagtcagccttgaccttgggaagggactcctctgctcaccttggagacagcagccgggtccaggggcctttgggtgactgggcctggcgtgcgtccagtacgctgacacatgatgtcattgaatccctgctccaggctgagccctggggctcagagaggttgtgtttccggcccaacctcacccagcaggtgggagatgacagggccaccgaggactgtgtcattggaaccacacgtgctctgaactgccacaggaagtcagttaagatgagcaaactgtttataaagttggagatgcaggctaggaacggtggctcatgcctgtaatcccagcactttgggaggccgaggcagatggatcacctgaggtcaggagtttgagaccagcctgaccaatatggtgaaaccttatctccactaaaaatacaaaaattagccaagcgcggtggcgggtgcctgtaattccagctattcaggaggctgaggcaggagaatcacttgaacctgggaggcggaggttgcagtgagctgagatcacgccactgcattccagcctgggagacagagctggctcaaaaaataaattaattaattaaaaacaaaattggagatgcactatgttattttcaaaacaagctgcctttaaagatctatctgttgtcacagggtgggctcatctgtttcattttattttctgtggtttatctatttattcattttaatgaactaggaagcattgctcctatttatggcataccacatgatgtttggatacgtgtatgcctgtggcatggctaagtcaagctagaacatgggccttacctcatatacgtgtcttattaagaacacataaaacctactcttgtagtgattttcaaatatgcaacatatagtttattaactgcagtcactatgatgtacaatagattgctcgaacttattcctcctgtctaactaagattttgtgacctctgaccaacatctccccagtgttgtcaccccccgcccccagcctctgatagctgcctttctactctctgcttctgtgagtttgatgtttatacattccacatgtaagtggcctcatgcagtgtttctgtctctgtgtctggcttgttcacttagcgtaatgtcctccagcttcatctatgttgttggaaatgacaggatttccttctttcttgtggctgaatagtattgccttgtgcatatacaccacattttctttatcccttcattcactgatggactcttaggttgatgtcatgtcttggctgttgtgaaaaatgccgcagtgagcgtgggcgtgcaggtccctcttcaacacacggatttcctttcctttggatataaacccagcagtgagattgctggatcacatggcagttctgtttctcaccttttgaggaaactccatactgttttccataatggctgtagcaacttccactcccacccccacggtgcaaagtctccatttctcttctacaacctcaccaactcctgttattttccatctttctgatagtagccatttgaagaggtatgagatgatacctcattgtggttttcatttgcatttttatttgtatttttcatgaatttttgagggtgatttcaagggtagttagtgactcgaacagggaaacgatcctgagtatgagggttgtgctaatcatccccctcctgccagctgcgtacggaatggggctctgcagatggcagggagctggctcgtttctctttaagagctgccttttacttttcttcctcttcctttaaaacttatttcctggccggacgcagtggctcatgcctgtaatcccagcactttgggaggccgaggtgggcggatcacgaggtcaggaattccagaccagcctggccaacatggtgaaaccccgtctctactaaaaatacaaaaattagccagacgtggtggtgcgggcctatagtcccagctactcgggaggctgaggcaggagaatcacttgaacctgggaggagggggttgcagtgagccgagattgcgccactgcactccagcctgggcgacagagccagactccatctcaaaaaacaaaaaaaagttatttcccaagcacagccatgtattccaggcttgtggatcagcgttggtggtggtgtgtgctctcatatcttagttccagctaagcacactctgacatgtttacactagaaccatttgttttttctagaaatagaaatttcagaattgtagagtcagaggacttaccagaaatctcttaggtagttctcctcccctccctcaagtgcagtcctaacctcctggagttttctgtagaaaccacaagcctcagagctggccgagaattctagccaaagatttttccatgccaaagtaatcccccctctcctaagggccatccttggtggggactggtttcctgttaagccctcgctgtcagtcctggctgtggaatttcctggtgaggagcactggcccgtggagctcggccctcgtgccggccttgagcaggcccaagtgttccgtgttcttgatacctttcctccagcacagtcttgcttcccagaaaaaggtttgcacttgaaaatgatgcatttgctgattaaacatagttcttttgctttatttggtttctaaaataaagtgggagtttttgagattgagtaacgtgaggttaagatagcacgtggaatggctttttcttttctttctattttttttttttttttcctggagacagggtttcactctgttgcccaggctggagtgcagaggcatgaccatggctcactgcaacttcgatgtcctggggttaagcgatcccccagcctcagccccccaagtggctgggactacaggtgctcgccaccacacctggctaatttttgtattttttgtagaaaatgggtttcatcaatgttgtccagactggtctcgaactcctgacctcaagcaattctcctgcctcagcctcccagactgctgggattacaggcgtgaactaccacgcctggcctggaatggcttttgatgttctcctatgtgcacatgtgggtgaataaacaccaacaaagtccttatgttacctgaagagttgctctcttcttaatatttaagtcgtatttatttaaatactttaatagttgtacactattaaagtattattaggtcaaaatcaaggaagtacaaaagggtatgctgtgaaaaatctcttcttccttgctctgcttacttacctaccccgcatccccccatacaccccagacacacacacacacacacacacacacacacacacacgcatcactcccatacatgcccacctgtttaccagccaatcacatttcttggggcaactcatctgagttgcttctctttccagagagtttttgcataaagaagcacaggtatttctgcgttaccatgaccctatttcccagtggttcctagccagttgactctcctgcactggataccatcctggacagcattccttagggaaatgagccccctgttttttcccaccatggcacagttggtcctttgcatggacgcaccattattgcccctgtctcttcttggtggaccttaaggttttctccatccttttgctgtaacacacactgctccaagtgtgtgagcatatcagtaggaaacgcttccaggagtagaactgctaggtcagagggcgtgtggatctgtaacctgacagacctagaccggcttcagtttggttttatccagtttccatattgattattcatataaaaggaaacagacaaacataacgctgtgcatgtattctctcttagaccagaacaggcatagggtgcacttttaatttgtccatttcgtagagtagaaattgtttttgctgaaatgaacaccttaggatgctgaagaatatgacccgtcccatggaaaacattcaaaaatgtgtgtagcgctttcttcccaagggtgtgtgtgcgcatattttaacactaattcactttctacttccgttgctatcctttctgtgagtctttctcagaatctcagaaaagaaactaaattgttcactctagttatcaatgctgtactctatacctggaatttgctaaaagggcagattttaagtattctcaccacagaaaagagaaaagaaaatggtaattatgtgacgtggtggacatgttaactagctttattatggtgagcatttcacagcggatatccagtcatcacgctgtacacattaaacatgtacaattgggtttttttgagacaaggtctccttctgtcacccagtctggagtgcagtggctcagtcatggctcattgcagcctcgacctcctgggctcaatccatccttccccctcagcctcctgaaaagctggggccacaggcatgtaccatcatgccaggctaatgcatatatatttatattttttggtggagatggggttggtctcgaactctgggctcaagtgatcctcccgccttgcccttccaaagtgctgagattacaggcatgaaccacagcaccaggcctacatgtaaaatttttatttgtcaactatactttgacaaagctgagaaaaaaaatcctaatatttaaaaaaaaaaaaaaaaggactagcttgagaccttttccagctctctggcttatcagctgccgtctcttccgggtgcagatagctggaagggaaagaaaatccctaaaattacccacaagccaagaatgaagtgtctccctttgagccacagtggcagttttgtttttaatcatagaagtgtattttgagccgggtgtgctggctcacgcctgtaatccccgcactttgggaggccgaggtggggggcggagggggtggggatcgcctgaggtcaggagttcgagaccagcctgaccaacatggagaaaccccgtctctactaaaaatacaaaattagccggcgtggtggtgcatgcctgtaatcccagctactcatgaggctgagtcaggagaatctcttgaacccaggaggtggaggttgcggtgagctgagatcatgccattgcactccagcctgggaacaagaaaaaaaaagaagaagaagaagaagtgtattcatttcagttacttttaaaaaagtgaacagactttatattttagagcggttttaggtttacagaaaatgaaacagacagggcagcgagctccttgtactcctccccagcacacagttgccctgttatgaacatcccacatcagtgctgtgcgttcattaacaccgatgaacctgatgcatacattatgatgaactgaagtcctggacttcaccctttctcttgtacagttctgtgggatttgacaaatgcataatgctgtacagccacaatgatagtatcgtccagagtagttctcctgccttaaaacctcttttgctgcacctgtttctctctccccactcaccccagctatctgatcttcttagtgcctccgaagttttggtcttttcaggatgttgtagcgttggaatcatggagtatgtagccttcaccacatacaccttccttcactttgttggcttcctttacttagtaatatgcattcaagtttcctccatgccttttcatggcttgatagctcatttctttttagcaccaaataatattccgttgtccagatgtagcacaatgtttatccattcatgtaacctgtgaccgactcacagataggatgtggaatcactcaccacagaggcattagacaataatcagacccaagtcatttcatgggggaacaagcccacaggtaccagactgtccagtgagtcagggccactcgtaggaagtaagaagagaggctagagcatagccaggtcctcactttatactttaagcccatgtgtatttctcccaaaccacacagcattgtttccatgctttcagctttgcatgaataacgtgatacttgaacgcatcatttatcacttgctctctttcccacagcgctgttttcaagcttcttcctgttcatgatgctctgcttaacccttaagctgcatgggattctgttctgtgaatacgcccaccccatgtattatcctgcccagcaaaaagtccccaaaactctggatggtggttacctctagggagggagagaagagattgggaatagggagcgacttcaacggtgtttgtaatgttttgtttctttaaataaaagagctgagatcatttcagcagaatgttgatttagagtctcctggacaatttgttgctcaaagtgctctcttaaagagcactttaaaaaaaaaaaccttttatcttattatttatttatttatttattgagacggagttttgctctgtcacccaggctggagtggagtggtgtgatctcagctcactgcaacctttacctcctgggttcaagcaattcccctgcctcagcctcccaagtaggtgggattacagatgcgtgccaccacacttggctaatttttgcattttagtagagatcggtttctccatgttggccaggctgatctcaaacgcctgacctcaggtgatctgcccgccttggcctcccaaagtgctggtattacaggcgtgagctaccatgcctggcttatcttatatatttttaaaaacagcttattgagatctaatttatgtaccataaaattcaagtatataattcagtgcttttatatataaaacatatatatgaaatagcttattgagatataattttttatataaaacagcttattgatatgtaatgtatgtaccataaaatttaaatatataattcactggcttttatatattcacgaatatgtgcaactatcaccacagtcaattttagcatattttcatcagctcataaagaaaccccaagcccttgaactatcaccccatatccctcctcccagcccgtccctcctactcataagcaaccactaatctacttagtgtctatagatttcctactctaggcattccatgtgagcgggatcatgcaatacgtgggctcacacaatataagtggcattccatgtgagtcggctcatgcagtatgtccggctcctttcactgagcataaggtcttcagcactcatccaggttgcagcctgtgtctgaatttcattccctcttctggctgaatcgtattccattgtgtatcttggacatatcctattctgctcacccagccgttggtgggcgtttggagtgttttcgcctttcagctgttttaagagggttgcagtgaacatttgtacaagttttggacccaatgcctgttttcaattctcttgtgtagagagcactttttagcagaaaaagaatagatttgtggcctccctttgtgtgcggtcagtgccttgagaagagtgaactgtgctgccacctccggagccgtggagagcgcggggcttgggtagcagctaggacgatacaagttgggacaaggccaggtgcaatggctcacgcctgtaattccaacactttgggagaccgaggcagggggatcacctgaggtcaggagttcaagaccagcctggccaacatggtgaaaccccatctctaataaaacagaaaaattaactggacggggtggtggacgcctgtaatcccagctactcgggaggctgaggcaggagaatcacttgaacctgggaggcggaggctgcagtgagtggagatcagaccactgcacttcagcctaggtgacagagcgagactccgtctcaaaaaaaagaaaaaaaaagaaagaaactcatggataatcctccctctcgtgcagttcgcctctacggaccaaacttcatccttcaggtgtactcatctcagaggaagtcctggcaccctgtgtgccaagacgactggaacgagaactacgggcgggcggcctgcagggacatgggctataagtgagtatggggcagcacccgccgagtgacagtaacagacagcagaaacacgagaagaccctctctctgcctccctgtgaaagcaccggcacatgagtgctggggacaattgtcaccttccaaaagctgagccctataaccagcaggtggaatttgtcctgctagggctgtgcccagcacacagaccttggctcactgccaccttgccctgcctcctccttggcctctatagactcctggttgctcgggagtgcccagtgctgtggtcatctggtcagaggggtaggctgagggcgttaggtgcctctttttccaaggtgcctctcagccagggtccattcacctccctgggtagaggttggaccagaacagctggcgaggagggttgggctggggagagcagcagagacaaatcctgtgccagtttcacttcattcgggagccatggaagccttttgagctggggagagaatcaatcaatcagactgatacttaaaaaatgtcattcctgctcgtagctctgagggaaggtgggaaggcttaacagggtgtgtgtcgcctgacagtgattcctaacgggggtggggcggtggttaccatttaccagcactgcctggggagatgcggcagccctcaggcatcgggggagagggtggtaggatgctactgccactttgttttccatgggagggtccccaggtgatttctatgcaactttagggtattcaatatgccagttttcagaatgaattaccactcggtgagaaagttggcatcttagctagtcactgtgacatccctaaacagcaggggtgaattacacagcaaagcccccccatcacagtccaggaacctggtggaattgataactggggccatgttaacatctgtaccttttattagattaaatgtgtgtatgattatacaatcctatgtccttctcatagtttcttgatcctaacctggataagaaacacgaccaatgaaggaattttgtctgacactttagggttattgaatcgaaaaatcgttacaatattctagcacttggttagaacgtgtgattttttttcctaaatgctaaggtttttccctcttattctgaatgtcgtatgagcggtattatgacatagtataggatttgtgtttgcttatgccttaaccattatcacaaataaggttttcttttttaggaataatttttactctagccaaggaatagtggatgacagcggatccaccagctttatgaaactgaacacaagtgccggcaatgtcgatatctataaaaaactgtaccacaggtatgcagcaatttcttcttgaaaaattttggaatgaaatcaactaggagacaccatggggaatcgttgtcctgagtctgatttctctgagctgcaatactcggtctggatgggttttgcattgggaggagattagagtctgaccaggcctggttactctaagcagcccttggtttattcataggaagtggctgaggtttctctgctatttcattttcagcctctaccgtctgcccttgttggtagcggctcacacttgcaacatcgacattcaactctatttagttttctttcctcttcagacatttagaggtgtacctattttgtcagggcgtggttctaggaatccaagataatgtctcagtgtcccagccagggtgaccggctcattccagtttgccagggacttcactggcttgagcaagggaagtcctgctccattccaggcagctgggctggctggtcccgttagccccaaccccgggacagcagtgccagagggtgctctgtgagggatgggcagcattctggcggcctgggaatgagttgtggtgtttccagggggtagaagtgggtacaagccacaggtcacatgatgagtggctgacctggctgggagggcagaagaggggatggacttaggctcttccttttgctttgcacatatttaggatgtttgcagacttgctatgattgttgctgttatgtgttttctgatgtgaaagatacacagtgtcctttgcccatgagctctccttgcctcccaggtccccagggcttatgcctggtgtctaggcatcacctccctgcctgccaggtgccaggtgctgcatttcgggggaggatgaactaatcaccccgcgccacctttcctctgagtgggagcctggggcaggtttgcattcctggaggccgctggtggaggggtctgggggcctgacttccactgcagcctgctgtcctggggaatgtggcagggcaagcccagtggggagggctgtgcacggccaggtgcacccatcaaaacagcagggctgcggtttgtccctgtggagaagctaaacacagctgcctgggcactttgtaaatgctgagtggttctttgtctttctgggttacacacggaatcagggagccaagtccagccgggcagggacggggggaggggaggaggtgctgccgtcccttggcaagagccttgggaactcacaaggaggctggagggcttggaagaaagaagagaaggccattgtctggtaggctctattctatctcggtggtggtggtggggggaggcgcacttcttttcctctttctgtgcagcagttgccctttgatgcctgagttcttggcttgttttctgtcgggcttctgtgaataaccacatgtgccctggcgctgtgaccacacagggctatccctaccgaccttaggattcttaggaaatgtcttctcttaaaggggacatgtcttcacttggccgtgtcagtgccccagagccagagtccacctggaatgcacctgtagtcactgagaacccggggggtgtgccttagtaagaaggtgtcaggaaggacctattattgtagggcctgggctcctgcaaggtggtttgggggtggttggaggaagcagagatttgctctggattggatgctgtcaggaagcaggggtaattctgtgaggctgctttattattttttttctaggaggaggttggaatgaggctaggctaaagctgtgattggtaaagaaacgtccgtcgctcaagttagccaggacaggaggagacatcagatcgtgattttgtggttgtgagcacaaggttcctgttctgtctgttcagacatcatttcggaggaggctccttgtgtcttgccccatctcaggcatggaggggcctagtccgatattgacgctcagtgaaataattcaggttccgcagagcacacggcccagctatcagggcgggccagctctgcatgccaggggccgcgtcttcccttctcagcatagcctgggaaattcactgcaggacaaaatgcatcagttacttcctcttcatccataacctgggatgtttgactcccaaatgagtaactcttacgtttcttctaatcctagggaaactattggttatattgctttcaacactacaaatttaaagcagttataggagcccagaggtttccaaatggcttccttaaaaattagaagatgattttaaattccaagaggaaaaacaaaactagcattattgtatacttaccctcacaaccgtcctaggagctggtacaattttaagagaggttaagtaacttgcccaaggtcacactgtggggatgtgagccgcgtaccttggctcagtgtctggtctttgccactgtccctatatggatttacttaccttattggagttgtaactagcagacccttctatgtctcagaagacaggagagggaacatcggaagaaatgactgatttctaagcatgtgagaggcaggtgactccgcactatcgtgaccagaatttcccctgttctttttgcagtgatgcctgttcttcaaaagcagtggtttctttacgctgtataggtaagttcatctggagtcccccttttgatacttctaactaggaaaagctctctactttcagaacagtactccctgtgtctctgggggcgtgggagggaagaaggtggggtcacgggttggaatgtgcccagcggcgtctcgctctttccaaggagctcctggtttagatttccatggcctgtagacaccttcagccttgggtccaagggacaccccctgagatcaggcacgctcaagaagctgacaaagccctacactttatgccacccatgagctggaggcccggcaggtctctttctccagaaagcaaaggggggtggcgttagtgagccctggcagccacctaacgtggacttggagcatctgcggggctgtggtccagcaccaccgtgtggccaccaggtgctcatcagccagtgggacccgggaggagggacaagaccagagaacaacagtgctcttgcctcttctctcctgaattttggacggtggcttagacttgggtgtccccatctctgtgtttagagtgcttacagtttccaaactgtttgcaaatgtggaagccaccgtccctctcctctgggatggcccagtgctgtcgtggggccgtggtcctgagctcagcttttcatttgaagaggtggaaggagctgacaccgtcccatcccggcagggctggctcaggtcttctttaggtcctgagtgggggtccagcacagccccaagggtgcgtggcacccgccctgccctctgcccatgcactcatctcctggtggagaagacactcacacacaggaagcagggaaggcagcagacctcactcacccctcaccccctcactcaccccctactcaccccctcaacctctcattcaccacccaccccctcgccccctcactcaccccctcactccctcaaccctcactcacctcctcactccctcaaccctcactcacctcctcacctcctcactctccccctcatccctccctcaccccaccccgtcacctcctcactcacctcctcaccccctcactcacccttcaccccctcactcaccacctcacctcctcactcaccccctactcaacccctcattcacccctcaccccctcactcacccctgcaccccctcactcaccccttcatccactcacccacctgctcacctcctcactcaacccctcaccccctcactaatccctcactccctcaccccctcacgccctcactcacaccttcacctcctcactcaccccctcaccccctcaaccccttacttaccccctcactcatcccttcacccctcactcaccccctctctcacccattcaccccctcactcatgccttcaccccctcactcacctcctcactcacaccttcacccctcagtcaccccctcactcaccccttcaccccctcaatcatgccttcactccctcactcaccccttcaccctctgaattactccctcatcccctcactcaccccctcactcaccccttcaccccctcacccaccacctcacccacccctcacccaccccctcacctccttacccctcacccccctcactcacccctcaccccctcactcaccacctcacccacccctcacccaccccctcactcactccctcatcccctcactcaccccctcaccccctcactcaccccctcacccacccctcacccaccccctcaccccctcactcaccccttcaccccctcactcaccccctcactcaccccttcaccccctcactcaccacctcacccacccctcacccaccccctcactcactccctcaccccctcactcaccccctcaccccctcactcaccccctcatctcctcactcaccccctcacctcctcactcacccgctcacctcctcactcaccccctcgccccctcactcacccctcaccccctcaccccctcactcacccctcaccccctcgccccctcactcaccccctcgccccctcactcacccctcaccccctcaccccctcactcatcccctcacctcctcactcaccccctcacctcctcactcaccccctcacctcctcactcaccccctcacctcctcacccaccccctcactcactccctcaccccctcaccccctcactcaccccctcacctcctcactcaccccctcacctcctcacccaccccctcactcactccctcaccccctcaccccctcactcaccccctcacctcctcactcaccccctcacctcctcactcaccccctcacctcctcactcatgccctcaccccctcactcaccctttcacctccttgctcatcccctcacttaccccctcacttcgtcaatcacccccccacctcgtcaatcaccccctcaccttttcactcaccccctcactcacccccttacttcctcacttacctcctcaccccccactcaccccctcaccccccactcaccccctcaccccacactcaccccctcaccccccactcaccccctcacccctctcacctcctcactcaccccctcacctcctcacttatcccctcaccccctcaattaccccctcaccccctcaattactccctcatcctttcaattacccactcaccccctcacctcctcactcctcactcactccctcactcaccccttcaccttctcactcacctcctcgtctcctcaccccctcactcacttccagccctgcccctcccatcttccttttctttgtgtgagaatctggggtccctgagtggtgtcagtccctccaagactcaaggagtccccagggccttgttatccagaacacccccacctgggtcccgggagaccccatgggatcacaggagtgttcagggaagtggtgcttcctgggtctgggtgggctggaggggcatcctcccttccccaagaggagacccccaggagccccctaagtccatccccagcagtggtgcccctgccctgtccttgcagcctgggagacccttgggaggggcgggcgctgggtggctgggcggcttctgctggtctcaccccactggcctcctgtttgtcatcctcagcctgcggggtcaacttgaactcaagccgccagagcaggattgtgggcggcgagagcgcgctcccgggggcctggccctggcaggtcagcctgcacgtccagaacgtccacgtgtgcggaggctccatcatcacccccgagtggatcgtgacagccgcccactgcgtggaaaagtatgccaggggcggcgcgggccgggtgggggctcagggctggcctacagccaccctgtgaccttgagcaggtctcaacccttgcagccccggcatccttgtgtttaaatggggagagtattgcacctgcttcctagggctgtgagacatcaagtgcgctcatgccaggcagtgcatggctgtatgcactgagtgtcccctgcacgcagggcacagggtgcaggtggaacattctccacgatgtcgccgtgaccagcgttccttccagccactgtcctctgagctctgtcctgcccttgagcaaagcccctgccccctgaggtatcctgtctccgggacgctagtcccaggagagggcacactcagacaggcttcaggctgccctgctggaaggtccctggggttaagcgttcttggccacagcattgctcatgcagagggttaggtaggggtgaggctagccgtgacagtattagcatttatggacgctaccaccccctccccttttccttaaacacatagtgcttttggtcacatgctgctttggaggaggcctcacttggcggatgtatttttctgccttagagagaggctgaactgggtttgactgttggcccagccctctcttgctgcgtgcccttagacgattcactcaacgtctctgatccatggcatgtacaactataagatgggcatgcccttctcctctcgggctgttatgaaggtcaaggaagcaagggctgttacccaagggtgctcccttctctccccctcttcacacccccaggtgctctgggccctctaggaactgggtttctctcaagggctgttacccaagggtgctcccttctctccccctcttcacaccactgggtgctctgggcccactaggagctgggattctcttaagagggaaactcttggataaaggaaatggtttgattgatatcggacaagtctgttcattagtatccatttattaagcacctaccatgtgccaggaaatgctttggcgtacaaaggaaaataagggccagtcctgctagaaatggccttgaaaccccagggagggatgtcggcccattgtgggtgctgcagattccttgaaggtgatgcaagagccagaaagaaggatgatgtggggggctgaggcagggagtcggggttgggggagtgtgggggagaaggggagaccgagcacctcttccactatctccctgtgtggtttttggtgaaccatcctgcctctgggtgtcttgcctccagcttctgacgttggaagttcatccactgagagctctgtgtttatggctctgagatactgagtccttcttctctcccagacctcttaacaatccatggcattggacggcatttgcggggattttgagacaatctttcatgttctatggagccggataccaagtagaaaaagtgatttctcatccaaattatgactccaagaccaagaacaatgacattgcgctgatgaagctgcagaagcctctgactttcaacggtacgtgtggctcaggcttggcaagcaggttggcagaatcttaaagagatgttgattggaaatgacacttgtgctatgccaaatggaagggaggcatttgcgttgagcgagggtagcgtgcagcgggtggccaatgggagaggctcacagaggctaagagcacctgccgcattttgggggaggcagcagccaccacatctgttctgtactgtactgagtggtggtgattcaagccaggcatggaaaaggctagaacagggctttcccactgcagcacccttgacatctgggtggttctctgttgtagggctctcttgtgccttgtaggatgtttaacagcgtccccagcctctacccactggaggccagtagctaccaagctgtgacaaccagtgttgcctgctgacattgccaaacatccgctttgaggcaaagtcacttccagttgagaactactggcctaaaatgtgtaaagatccttgatttttaaagatacattctaaaaccaagttgcttaattcaggacaaacatgctttctcttagcctcttattcggtcccactctggtccatccaagggtctggaatgttctagccccatgtggatacagaagaagcaaaacctcagccctccctacagcatgtctgtattcacattgggaaatggttcacatatagaagagcgaatgcctgagcaatggcgtggtgcctctggggcgaaagctgactccattgactccatcggctttttggctgttgcctcctgtgtgtctttcccgtcttgatcacctggagatatgtaattttggaagcagagctagcaaataattcctcttataagcagagctagcaaataattctacttataagtagcataacgtcttgcctgccagaaggagaggtctggcagggggagaaagtgagaatgtgggacttgttgggatgcagggtcctctgggcagggtggccagggtgccaggcccagcagcctgcatgtgggaaggccaggtggagacataggtgatacccgcctggctcactgtgttttctcttcttgaaacagacctagtgaaaccagtgtgtctgcccaacccaggcatgatgctgcagccagaacagctctgctggatttccgggtggggggccaccgaggagaaaggtgaggctgctcctgggcacacaggactgcagggcccacagatggagcattgggttcggaagtgggaggtccaggttttaatcccagttctactactcaatgactggatgactttggttgattcccccagtccttgtgcctcagtttctccatctgctaagtgggagaaatcctgcccagcctacctaatacactgtgttcttatcgtgatcacacagagcagcatgtggaatggcttttgaagtatctgggccatacgagtttagaggtgcaggatctcctgtgttgcactcattgtgagtttagagctgccctggagatcccaccaaggcctgcgtggctgagtgacagggggcttggtgaggacgggcatcctggacccatggtggccacatctaagcctgtcctctgccctgataaccacagagagaggctctctccacccacttcctttgcaatctgcatttctctctgacagtctttcaaatgaagggagcctggctgcttcatttttatggagggttggaagtgcttagtggcaggcacaaaggttcattttacatattgtttatatccttctcaaaagcgtctaggccatacagacaacaaatcctttcaaacaaggggaaaagtacaaaggttgggtgatttctggggagcgtcagggaaggtagtggggggcatcctggctcctcatcagcagaaacttactacagtagagccacaggctgggcaaaagacctcatggaatccaagatgaagggaatatcgacaaatatttgtgcgcacctgcacctagtacaggctgggtgctactcaggtgctgggaatgcagaagtgaacagagtaagacaaatgtctctgctgtcaggagctttacctctcttctggatgtcggtggtggggacggggcaggtgtggtcagacagatgggagacaaacaactgagcgaggtacttccaaacatctgagggtggggatcacaaggtcccggctattttgaaggggtggtcaggaaaggcttctcggaagaggtggcatttgagctgagactcaaatggcaaaaatgtgtacacatcaaaaaggctagtgcatgtatcttcaggtgtggtcaaggggccaaggaggtgggctggggccagattgcataggtccttgtggattatggtgaagacaccagcttctcatctgcttgaggtggggagatcgtgagccggggagtgccatgatctggcagctgcgtggggagtggggatgaatggatggagacgaggatgatggtgacaagtccattgctgtggttccttgagacaggaagccagctcatagcagagtgcgggcgtggatgtgaagagatgagggtacactagggctagagccaccagacttactgatgggttgcatgtctgtgggagagagagtgagaagtcagggacgatggctttccactctgtggctgaagccccagggtggcgggtggtgccatttttcaagccaggaaatattggttggtgagaatttggggtgggagaaggtgtgacggagggttctggttttgcacactaagcccacggtgcccagaagatgcccgaggggaggcagcaaagcgagagtgggaaatgcagaggtggcaagtgcaggccgtgtcttgagaagctctaatgtgcaggggagccgagaagcaggcggcctagggagggtcacgtgtgctccagaagagtgtgtgcatgccagaggggaaacaggcgcctgtgtgtcctgggtggggttcagtgaggagtgggaaattggttcagcagaaccaagccgttgggtgaataagagggggattccatggcactgatagagccctatagtttcagagctgggaatttctttccctgaagctgaactccagagctgcattcagcacaggcaccgccagttgtaaggagaatccaggtttcccaggagaggggttggtgctgggatgagctgaccggggcagggctggaaaatagggctgtgaccatctgtgtagtgcgtgtggaggtctcagggagggaagtgtgctctccctgcgagagctgcaggcaacactgggagctcaacaagtctccctgtccttagggaagacctcagaagtgctgaacgctgccaaggtgcttctcattgagacacagagatgcaacagcagatatgtctatgacaacctgatcacaccagccatgatctgtgccggcttcctgcaggggaacgtcgattcttgccaggtaattcaacatttttattctacctttggtccttaccagatcctactgaaccccccatgagagagagggcattcttggggtcagcagagcctcctcagtgacacggagccagctcggggcagtcatgggaagtgacggccacaaacagtgcgaacgcttctggtggcagaaggaagtacagtcaacaaatcacacacaccctctgaaaaaccggtatttggtaaaagtgccagtggaacagaaacaagtatttagactattttaaattatgaacggcaatttatttagtaacttttagcttgaacagattaaaattcaggatgggggctatctctttgggggttacatctctgttaccatcaccccttgatggtggagattcgaagcccacacagtcactcgtaactcacactgcgacccccgccccccaactcctctaggcctggtcagtggtgtgcggcagattgtgacttgattttctgctctctgtaccttgctgtgtcccacagggtgacagtggagggcctctggtcacttcgaagaacaatatctggtggctgataggggatacaagctggggttctggctgtgccaaagcttacagaccaggagtgtacgggaatgtgatggtattcacggactggatttatcgacaaatgagggtaactatcctgtcctccttctgactgtgttctccgattcctcgagccaaagccagacatctgttaggcgtggttctgctgctggaagctgactggtgaccactggtcagcatgaagcaaactctgcttcctccagccacagccccatccccccagtgtccacccattgcccattgcctctcactggcttcacttgcatatttcccctggtgtttggatgaaaagcgctggggctcagcttgtgtgaaattccttggtgctctgccaaccacacttcgttctggctcagctgactcagctgttccacccaggccacctcacatcaaactttttttttttttttttgagatggagtctcactgtgtcgcccaggctggagtgcagtggcacaatctcgactcactgcaacctttgcctcctgggttcaagtgattctcctgcctcagcctcccaagtagctgggactacaggcatgcgccaccacgcccagctactttttgtatttttagtagagatggggtttctccatgttggccaggctggtctcgaagccctgacctcaggtgattcacccacctcagcctcccacagtgctgggattacaagtgtgaaccacggtgcccggcctcacatgaaacttttgatttatagagagcagagggaagagccggctgtgcccatccttttctggggccatcgagtggctcctgggcagcccccaaggttaggaagggcaggagcagccagggttctctgatgccccagactcaagcacgagggaaggtctcaggggttccatgtgagcctcatggatgtctctgcttagcagagccctggctttgggcattgtccagatagggggtgagaaccagatcttctcatctccaggacctcagacgtatagttttctcagatttctgtgctttctggggctgggctactagtggaagaaagcagtctattctgtcttctcccaaatctcccagatgcccagtctgttgaaggaggagcagaaccagggggcctttcccgctgaggcccgacctgtgtctccttcaaatgacacgcgggactcagggccttcccatgaccatggggcccagggggcgtcacctggcccagggcccagtgctagaaacagatgaccccaggaggaggaggcagggcaggagggaagctggcagggctgggatggtcagccaggctgaggggcggactcgcaccaggatggagctaggaaatgatccaggtgtgtttggcggctgcaggtgggtccgcatggctgtgcagggagggaagggctgcgtggcaggagagcagccgggggaggcccagactctgctgaagagatgcctgttgtgccggcctccacatccgctgcccgctccttccggagctcctgccccgccatgctcagcctgactctgaccaacacgttggagagaagaatgatccctttgtgctattaagcttgcttatttggtttctaagtgcttcatgcgaacctagaggaaaaaattattttccacctttgtttgtcttaagaaaataacacacttttttttttcctatttgaacaggcagacggctaatccacatggtcttcgtccttgacgtcgttttacaagaaaacaatggggctggttttgcttccccgtgcatgatttactcttagagatgattcagaggtcacttcatttttattaaacagtgaacttgtctggctttggcactctctgccattctgtgcaggctgcagtggctcccctgcccagcctgctctccctaaccccttgtccgcaaggggtgatggccggctggttgtgggcactggcggtcaagtgtggaggagaggggtggaggctgccccattgagatcttcctgctgagtcctttccaggggccaattttggatgagcatggagctgtcacctctcagctgctggatgacttgagatgaaaaaggagagacatggaaagggagacagccaggtggcacctgcagcggctgccctctggggccacttggtagtgtccccagcctacctctccacaaggggattttgctgatgggttcttagagccttagcagccctggatggtggccagaaataaagggaccagcccttcatgggtggtgacgtggtagtcacttgtaaggggaacagaaacatttttgttcttatggggtgagaatatagacagtgcccttggtgcgagggaagcaattgaaaaggaacttgccctgagcactcctggtgcaggtctccacctgcacattgggtggggctcctgggagggagactcagccttcctcctcatcctccctgaccctgctcctagcaccctggagagtgcacatgccccttggtcctggcagggcgccaagtctggcaccatgttggcctcttcaggcctgctagtcactggaaattgaggtccatgggggaaatcaaggatgctcagtttaaggtacactgtttccatgttatgtttctacacattgctacctcagtgctcctggaaacttagcttttgatgtctccaagtagtccaccttcatttaactctttgaaactgtatcatctttgccaagtaagagtggtggcctatttcagctgctttgacaaaatgactggctcctgacttaacgttctataaatgaatgtgctgaagcaaagtgcccatggtggcggcgaagaagagaaagatgtgttttgttttggactctctgtggtcccttccaatgctgtgggtttccaaccaggggaagggtcccttttgcattgccaagtgccataaccatgagcactactctaccatggttctgcctcctggccaagcaggctggtttgcaagaatgaaatgaatgattctacagctaggacttaaccttgaaatggaaagtcatgcaatcccatttgcaggatctgtctgtgcacatgcctctgtagagagcagcattcccagggaccttggaaacagttggcactgtaaggtgcttgctccccaagacacatcctaaaaggtgttgtaatggtgaaaacgtcttccttctttattgccccttcttatttatgtgaacaactgtttgtctttttttgtatcttttttaaactgtaaagttcaattgtgaaaatgaatatcatgcaaataaattatgcaatttttttttcaaagtaactactgcatctttgaagttctgcctggtgagtaggaccagcctccatttccttataagggggtgatgttgaggctgctggtcagaggaccaaaggtgaggcaaggccagacttggtgctcctgtggttctcgagataacttcgtataatgtatgctatacgaagttatgctagtaactataacggtcctaaggtagcgagctagctccacgtggctttgtcccagacttcctttgtcttcaacaaccttctgcaagaaaaccaagggcctgaattttaacttcctg

SEQ ID NO: 7 - protein, 491 aa, Artificial Sequence
  Recombinant protein
MALNSGSPPGIGPCYENHGYQSEHICPPRPPVAPNGYNLYPAQYYPSPVPQYAPRITTQASTSVIHTHPKSSGALCTSKSKKSLCLALALGTVLTGAAVAAVLLWKFMGSKCSNSGIECDSSGTCINPSNWCDGVSHCPGGEDENRCVRLYGPNFILQVYSSQRKSWHPVCQDDWNENYGRAACRDMGYKNNFYSSQGIVDDSGSTSFMKLNTSAGNVDIYKKLYHSDACSSKAVVSLRCIACGVNLNSSRQSRIVGGESALPGAWPWQVSLHVQNVHVCGGSIITPEWIVTAAHCVEKPLNNPWHWTAFAGILRQSFMFYGAGYQVEKVISHPNYDSKTKNNDIALMKLQKPLTFNDLVKPVCLPNPGMMLQPEQLCWISGWGATEEKGKTSEVLNAAKVLLIETQRCNSRYVYDNLITPAMICAGFLQGNVDSCQGDSGGPLVTSKNNIWWLIGDTSWGSGCAKAYRPGVYGNVMVFTDWIYRQMRADG

SEQ ID NO: 8 - DNA, 2267 bp, Mus musculus
ccggttgtgttataggacttgaccagccccaatagtcctcaagtcactcctagatacagtggcaggtggtagctggcttgcggaaggaagaggaagaagagaatgtgggccatcaaggagcaaggccagccttgcacttgggccccctctgctcagtgctgaccagggctttctgagccgcttcctaatgaggctcatttgaagacccccccccacccccctcctgctgtcttgggtggcagagctagctccaggctgtaagaaaattaggaggattaccaaagcagtatggagtcagacagtggccaacccctcaacaaccgtgatattgttccctttcgcaaaccccgaaggccccaggagaccttcaaaaaggtggggatccccatcattgcagtgctgctgagcctgatagccctcgtgattgtggcccttctcatcaaggtgattctggataaatactacttcatctgcggcagtcccctgaccttcattcagaggggccagttgtgtgacggccaccttgactgcgcctcaggggaggatgaggaacactgtgtcaaggacttccctgaaaagcccggagtggcagtccggctctccaaggacagatccaccctgcaggtgctggatgcagccacagggacctgggcctcagtctgtttcgacaacttcacagaagcactggccaagacagcctgcagacagatgggctatgacagccagcccgctttcagagcagtggagatccgtccagatcagaacctccctgttgctcaagtcacaggaaacagccaggaacttcaggtgcagaatggaagcagatcctgcctctcaggctccctggtttccttgcgctgccttgactgtggaaagagcctgaagactcctcgtgtggtgggtggggtggaggcccctgtggattcttggccgtggcaggtcagcatccagtacaacaagcagcatgtctgtggtgggagcatcctggatccccactggatcctcacagcagcccactgcttcaggaagtatcttgatgtgtcaagctggaaggtcagggcaggctcaaacatactgggtaactctccatccttgcctgtggccaagatcttcatcgctgaacccaatcctctgtaccccaaagagaaggacattgcccttgttaagctgcagatgccactcacattctcaggctcagtcaggcccatctgcctgcccttctctgatgaggtgcttgtcccagccacaccagtctgggtcattggatggggctttacagaagaaaacggaggaaagatgtctgacatgctactgcaggcatcagtccaggtcattgacagcacacggtgcaatgcagaggatgcctacgaaggggaagtgaccgctgagatgctgtgtgcaggtaccccacagggtggcaaggacacctgccagggtgacagtggtgggcctttgatgtaccattctgacaagtggcaggtagtaggcatcgtgagctggggccatggatgcggcggcccaagtactcctggagtgtataccaaggtcactgcctatctcaactggatctacaatgttcggaagtctgagatgtaacgctgccgtcccccacatccagaagctgcttcccttcagacctacctacggcatgacccctcaaagtcagatatgggacaagagcctccttgaacaaactctggtatccctgcagcaagcaaggatacattgcagaggtgcccggagtggagtcagatgggctagctcagccacccctgcatctcccaaaccctgggagacatgtggcccatgggagtaaatccaggacattgactcaactctcagaagtgttattcagtcaaggaggctctcccttccactgaaggaaggaaagtcagctctctcctgaaaggccagatcactggctgagtagatgagacaagggtatgaaaggcctttgccatcttctttgcccagtcctgaaagcactgacgtaagagaccagtcagttctaatgtaaggtgtatattttagtgtcagggtattgcaattgtcacctctgtggtcaatatcattaaacaggtatgagaattcgctggcatagacttcctggtctgcttaataagaatccaactaaggatgtcacatgacagtttcccagaaaatgtgaacaagtgtccatctgacacacggcaccaatgacaaaccaaagaagttattctgcctgagtctcagttgctgaactaataaattagctgcggtttcttgca

SEQ ID NO: 9 - protein, 435 aa, Mus musculus
MESDSGQPLNNRDIVPFRKPRRPQETFKKVGIPIIAVLLSLIALVIVALLIKVILDKYYFICGSPLTFIQRGQLCDGHLDCASGEDEEHCVKDFPEKPGVAVRLSKDRSTLQVLDAATGTWASVCFDNFTEALAKTACRQMGYDSQPAFRAVEIRPDQNLPVAQVTGNSQELQVQNGSRSCLSGSLVSLRCLDCGKSLKTPRVVGGVEAPVDSWPWQVSIQYNKQHVCGGSILDPHWILTAAHCFRKYLDVSSWKVRAGSNILGNSPSLPVAKIFIAEPNPLYPKEKDIALVKLQMPLTFSGSVRPICLPFSDEVLVPATPVWVIGWGFTEENGGKMSDMLLQASVQVIDSTRCNAEDAYEGEVTAEMLCAGTPQGGKDTCQGDSGGPLMYHSDKWQVVGIVSWGHGCGGPSTPGVYTKVTAYLNWIYNVRKSEM

SEQ ID NO: 10 - DNA, 3543 bp, Homo sapiens
atcattccagtttggcaacttcacttgtagggctgttttaatcaagctgcccaaagtcccccaatcactcctggaatacacagagagaggcagcagcttgctcagcggacaaggatgctgggcgtgagggaccaaggcctgccctgcactcgggcctcctccagccagtgctgaccagggacttctgacctgctggccagccaggacctgtgtggggaggccctcctgctgccttggggtgacaatctcagctccaggctacagggagaccgggaggatcacagagccagcatggatcctgacagtgatcaacctctgaacagcctcgatgtcaaacccctgcgcaaaccccgtatccccatggagaccttcagaaaggtggggatccccatcatcatagcactactgagcctggcgagtatcatcattgtggttgtcctcatcaaggtgattctggataaatactacttcctctgcgggcagcctctccacttcatcccgaggaagcagctgtgtgacggagagctggactgtcccttgggggaggacgaggagcactgtgtcaagagcttccccgaagggcctgcagtggcagtccgcctctccaaggaccgatccacactgcaggtgctggactcggccacagggaactggttctctgcctgtttcgacaacttcacagaagctctcgctgagacagcctgtaggcagatgggctacagcagcaaacccactttcagagctgtggagattggcccagaccaggatctggatgttgttgaaatcacagaaaacagccaggagcttcgcatgcggaactcaagtgggccctgtctctcaggctccctggtctccctgcactgtcttgcctgtgggaagagcctgaagaccccccgtgtggtgggtggggaggaggcctctgtggattcttggccttggcaggtcagcatccagtacgacaaacagcacgtctgtggagggagcatcctggacccccactgggtcctcacggcagcccactgcttcaggaaacataccgatgtgttcaactggaaggtgcgggcaggctcagacaaactgggcagcttcccatccctggctgtggccaagatcatcatcattgaattcaaccccatgtaccccaaagacaatgacatcgccctcatgaagctgcagttcccactcactttctcaggcacagtcaggcccatctgtctgcccttctttgatgaggagctcactccagccaccccactctggatcattggatggggctttacgaagcagaatggagggaagatgtctgacatactgctgcaggcgtcagtccaggtcattgacagcacacggtgcaatgcagacgatgcgtaccagggggaagtcaccgagaagatgatgtgtgcaggcatcccggaagggggtgtggacacctgccagggtgacagtggtgggcccctgatgtaccaatctgaccagtggcatgtggtgggcatcgttagttggggctatggctgcgggggcccgagcaccccaggagtatacaccaaggtctcagcctatctcaactggatctacaatgtctggaaggctgagctgtaatgctgctgcccctttgcagtgctgggagccgcttccttcctgccctgcccacctggggatcccccaaagtcagacacagagcaagagtccccttgggtacacccctctgcccacagcctcagcatttcttggagcagcaaagggcctcaattcctataagagaccctcgcagcccagaggcgcccagaggaagtcagcagccctagctcggccacacttggtgctcccagcatcccagggagagacacagcccactgaacaaggtctcaggggtattgctaagccaagaaggaactttcccacactactgaatggaagcaggctgtcttgtaaaagcccagatcactgtgggctggagaggagaaggaaagggtctgcgccagccctgtccgtcttcacccatccccaagcctactagagcaagaaaccagttgtaatataaaatgcactgccctactgttggtatgactaccgttacctactgttgtcattgttattacagctatggccactattattaaagagctgtgtaacatctctggcataggctagctggaatgcttgataagaactgagctgggatgattgaactttcattctttggcttggggagaaaagaagtcctggggaagcaattgagtctcaaagtagaggcaggggaaaaaagagttagggagaccagatctgctgagtggcagcaagagtgagctgcagattacagaaaccagggtgagcaagtttgagtcccacacagggccttctccctttgcctctttccctccctccctgcctgtgataatcagccaggagccagggataacctatgacttgggaaagagatgagttaggcagtcaagggtgacattcaatcagggatccacaagtggctggaaagaaatgctggtcctgtgtcctaactttttccgcctggagagccctcagtgtggcttcttacatttaaaaaacaaaaaggatcagctgccaggtgtgaggcagtccccaagctgagttgtgaggatgtaagcatgaataagtccctgcactcaaaatggtcaaagaattaaaccccatggacttttttggcatctgtatgaaagcttgggttttctgaggactgtcttgctatagttaagtcagatcctagatgaaatatacttgttcatactgtactaggttcttaggaaacaacagaattcctcaaatgccaaaaacaaagaaaatagaaacccagaaaacaaaacaaaataaaacaaaaccatcagaactgtgagtggaaactaaggtgatgatctgggagcaatacactaaaatcttgggtcgagacctatatgaaggctggcagtggagctaaacctggacacactgaagacaagggagctgaaccagggctcctacatgaagcagggataactgatggcagtaaatgtggtctcaaattgcagatggtctggaggaaaatttcccaaatttagagcctcaggattcccaaagatcctccaaatatgagctcacaatcaaagatcagagacgttgaaaaataaaaaacaccttaagtgggcagcataaaaaacagctaatttagaaccccaaaggcttcagatgtcagaatattagagacttatgataataagcaatatttgcagagtatttgtatgtgccagacactattgtaagtgcttcatcatgtactgattcatttaatactcacagaaatctgtgagatgggtattattcttatcctcactctatggattaaaaaaactaaggcacaaagtggttaagctccttgcctgagattatagactgtaagttgaacgtgagcacttggaatacagagttcatgctgtaaactaccacactatagggcctccaatatgataatttataaaatatttgaataaaaaatgaatactagttccacattttaaaaaaaaaaaaaaaaaa

SEQ ID NO: 11 - protein, 437 aa, Homo sapiens
MLQDPDSDQPLNSLDVKPLRKPRIPMETFRKVGIPIIIALLSLASIIIVVVLIKVILDKYYFLCGQPLHFIPRKQLCDGELDCPLGEDEEHCVKSFPEGPAVAVRLSKDRSTLQVLDSATGNWFSACFDNFTEALAETACRQMGYSSKPTFRAVEIGPDQDLDVVEITENSQELRMRNSSGPCLSGSLVSLHCLACGKSLKTPRVVGGEEASVDSWPWQVSIQYDKQHVCGGSILDPHWVLTAAHCFRKHTDVFNWKVRAGSDKLGSFPSLAVAKIIIIEFNPMYPKDNDIALMKLQFPLTFSGTVRPICLPFFDEELTPATPLWIIGWGFTKQNGGKMSDILLQASVQVIDSTRCNADDAYQGEVTEKMMCAGIPEGGVDTCQGDSGGPLMYQSDQWHVVGIVSWGYGCGGPSTPGVYTKVSAYLNWIYNVWKAEL

SEQ ID NO: 12 - DNA, 20078 bp, Artificial Sequence
  Recombinant polynucleotide
ccacccgcacacactacagtcgagataacttcgtataatgtatgctatacgaagttatatgcatggcctccgcgccgggttttggcgcctcccgcgggcgcccccctcctcacggcgagcgctgccacgtcagacgaagggcgcagcgagcgtcctgatccttccgcccggacgctcaggacagcggcccgctgctcataagactcggccttagaaccccagtatcagcagaaggacattttaggacgggacttgggtgactctagggcactggttttctttccagagagcggaacaggcgaggaaaagtagtcccttctcggcgattctgcggagggatctccgtggggcggtgaacgccgatgattatataaggacgcgccgggtgtggcacagctagttccgtcgcagccgggatttgggtcgcggttcttgtttgtggatcgctgtgatcgtcacttggtgagtagcgggctgctgggctggccggggctttcgtggccgccgggccgctcggtgggacggaagcgtgtggagagaccgccaagggctgtagtctgggtccgcgagcaaggttgccctgaactgggggttggggggagcgcagcaaaatggcggctgttcccgagtcttgaatggaagacgcttgtgaggcgggctgtgaggtcgttgaaacaaggtggggggcatggtgggcggcaagaacccaaggtcttgaggccttcgctaatgcgggaaagctcttattcgggtgagatgggctggggcaccatctggggaccctgacgtgaagtttgtcactgactggagaactcggtttgtcgtctgttgcgggggcggcagttatggcggtgccgttgggcagtgcacccgtacctttgggagcgcgcgccctcgtcgtgtcgtgacgtcacccgttctgttggcttataatgcagggtggggccacctgccggtaggtgtgcggtaggcttttctccgtcgcaggacgcagggttcgggcctagggtaggctctcctgaatcgacaggcgccggacctctggtgaggggagggataagtgaggcgtcagtttctttggtcggttttatgtacctatcttcttaagtagctgaagctccggttttgaactatgcgctcggggttggcgagtgtgttttgtgaagttttttaggcaccttttgaaatgtaatcatttgggtcaatatgtaattttcagtgttagactagtaaattgtccgctaaattctggccgtttttggcttttttgttagacgtgttgacaattaatcatcggcatagtatatcggcatagtataatacgacaaggtgaggaactaaaccatgggatcggccattgaacaagatggattgcacgcaggttctccggccgcttgggtggagaggctattcggctatgactgggcacaacagacaatcggctgctctgatgccgccgtgttccggctgtcagcgcaggggcgcccggttctttttgtcaagaccgacctgtccggtgccctgaatgaactgcaggacgaggcagcgcggctatcgtggctggccacgacgggcgttccttgcgcagctgtgctcgacgttgtcactgaagcgggaagggactggctgctattgggcgaagtgccggggcaggatctcctgtcatctcaccttgctcctgccgagaaagtatccatcatggctgatgcaatgcggcggctgcatacgcttgatccggctacctgcccattcgaccaccaagcgaaacatcgcatcgagcgagcacgtactcggatggaagccggtcttgtcgatcaggatgatctggacgaagagcatcaggggctcgcgccagccgaactgttcgccaggctcaaggcgcgcatgcccgacggcgatgatctcgtcgtgacccatggcgatgcctgcttgccgaatatcatggtggaaaatggccgcttttctggattcatcgactgtggccggctgggtgtggcggaccgctatcaggacatagcgttggctacccgtgatattgctgaagagcttggcggcgaatgggctgaccgcttcctcgtgctttacggtatcgccgctcccgattcgcagcgcatcgccttctatcgccttcttgacgagttcttctgaggggatccgctgtaagtctgcagaaattgatgatctattaaacaataaagatgtccactaaaatggaagtttttcctgtcatactttgttaagaagggtgagaacagagtacctacattttgaatggaaggattggagctacgggggtgggggtggggtgggattagataaatgcctgctctttactgaaggctctttactattgctttatgataatgtttcatagttggatatcataatttaaacaagcaaaaccaaattaagggccagctcattcctcccactcatgatctatagatctatagatctctcgtgggatcattgtttttctcttgattcccactttgtggttctaagtactgtggtttccaaatgtgtcagtttcatagcctgaagaacgagatcagcagcctctgttccacatacacttcattctcagtattgttttgccaagttctaattccatcagacctcgacctgcagcccctagcccgggcgccagtagcagcacccacgtccaccttctgtctagtaatgtccaacacctccctcagtccaaacactgctctgcatccatgtggctcccatttatacctgaagcacttgatggggcctcaatgttttactagagcccacccccctgcaactctgagaccctctggatttgtctgtcagtgcctcactggggcgttggataatttcttaaaaggtcaagttccctcagcagcattctctgagcagtctgaagatgtgtgcttttcacagttcaaatccatgtggctgtttcacccacctgcctggccttgggttatctatcaggacctagcctagaagcaggtgtgtggcacttaacacctaagctgagtgactaactgaacactcaagtggatgccatctttgtcacttcttgactgtgacacaagcaactcctgatgccaaagccctgcccacccctctcatgcccatatttggacatggtacaggtcctcactggccatggtctgtgaggtcctggtcctctttgacttcataattcctaggggccactagtatctataagaggaagagggtgctggctcccaggccacagcccacaaaattccacctgctcacaggttggctggctcgacccaggtggtgtcccctgctctgagccagctcccggccaagccagcaccatgggtacccccaagaagaagaggaaggtgcgtaccgatttaaattccaatttactgaccgtacaccaaaatttgcctgcattaccggtcgatgcaacgagtgatgaggttcgcaagaacctgatggacatgttcagggatcgccaggcgttttctgagcatacctggaaaatgcttctgtccgtttgccggtcgtgggcggcatggtgcaagttgaataaccggaaatggtttcccgcagaacctgaagatgttcgcgattatcttctatatcttcaggcgcgcggtctggcagtaaaaactatccagcaacatttgggccagctaaacatgcttcatcgtcggtccgggctgccacgaccaagtgacagcaatgctgtttcactggttatgcggcggatccgaaaagaaaacgttgatgccggtgaacgtgcaaaacaggctctagcgttcgaacgcactgatttcgaccaggttcgttcactcatggaaaatagtgatcgctgccaggatatacgtaatctggcatttctggggattgcttataacaccctgttacgtatagccgaaattgccaggatcagggttaaagatatctcacgtactgacggtgggagaatgttaatccatattggcagaacgaaaacgctggttagcaccgcaggtgtagagaaggcacttagcctgggggtaactaaactggtcgagcgatggatttccgtctctggtgtagctgatgatccgaataactacctgttttgccgggtcagaaaaaatggtgttgccgcgccatctgccaccagccagctatcaactcgcgccctggaagggatttttgaagcaactcatcgattgatttacggcgctaaggtaaatataaaatttttaagtgtataatgtgttaaactactgattctaattgtttgtgtattttaggatgactctggtcagagatacctggcctggtctggacacagtgcccgtgtcggagccgcgcgagatatggcccgcgctggagtttcaataccggagatcatgcaagctggtggctggaccaatgtaaatattgtcatgaactatatccgtaacctggatagtgaaacaggggcaatggtgcgcctgctggaagatggcgattgatctagataagtaatgatcataatcagccatatcacatctgtagaggttttacttgctttaaaaaacctcccacacctccccctgaacctgaaacataaaatgaatgcaattgttgttgttaaacctgccctagttgcggccaattccagctgagcgtgcctccgcaccattaccagttggtctggtgtcaaaaataataataaccgggcaggggggatctaagctctagataagtaatgatcataatcagccatatcacatctgtagaggttttacttgctttaaaaaacctcccacacctccccctgaacctgaaacataaaatgaatgcaattgttgttgttaacttgtttattgcagcttataatggttacaaataaagcaatagcatcacaaatttcacaaataaagcatttttttcactgcattctagttgtggtttgtccaaactcatcaatgtatcttatcatgtctggaataacttcgtataatgtatgctatacgaagttatgctagtaactataacggtcctaaggtagcgagctagccaagtctgtgtgctaccaagtagcaaaactgagcctggaactcacacatgcgtgtctgagagcccagcactatcgccaggaaaacccagcgtctccctgctcaagcctgaccctcagccctctctgcctctccctgcacttgccttccagtcaaggtgattctggataaatactacttcctctgcgggcagcctctccacttcatcccgaggaagcagctgtgtgacggagagctggactgtcccttgggggaggacgaggagcactgtgtcaagagcttccccgaagggcctgcagtggcaggtgagtgcagggtctgaggcacaagagaagtgggcccagcaggaggtctgctcaggcccccacggcccactgcatagtatctgccccctacttgtcacttttcatccttgttgtataaggttctttgtttgtttgtttgttgttgttttgaggcagagtgctctgtggcccaagatggagtgcagtgtcttggtctcggctcactgcaacctctgcctcccagtttcaagtgattcttctgcctcagcctcatgagtagctgggattacaggtgccagccaccacgcctggctaatttttatatttttagtagagacggggttttgccacattggtcaggctgatcttgaactcctgacctcaggtgatctgcccgcctcagcctcccaaagtgctgggattacaggcgtgagccaccgtgcccagctgtgtaagtttcttgagagcaggaccctgtcttgtctacctttaaatcctagtacttaacacacagcaaacagtaactatttgatgaccaaatgtgagccagaaaggacaggaaattgtaactgaggctgccccatgcgtgctgcgcctggtggatttcaggcagagggctagactgggtgaccttggggcattcctcctttctatgaaatttgttatttcaaggagactagaaaagagacttctcagccacttcgccagctattggtccttctattcattagtgtttgctgagacatgctatgtgacaggactgagccaggtcctttcaatggataggagatgttttgagcataaaatccacgttctctcttgggctgggctcttctaccttcttccccctggtgcttgggctctgaagaaaaaaagataggtaggagatgagtgatggggcttctgagggcagggctgagtgactttctgtgtatttgctctttctttatcagaagtcaaatgcccacaggcacctgtcatcctactgccagtaggacttctcactcaaccttcccctctgaccttacttggagaaggacttaggtccctctctcagacatttccccaggctgggcaagttgtgtggaccatggatgggtatgtggtccatacaatttaaacaagctgtatatggtcgctgggtagagtgaccacataattgatcatcaaaactgatacctgtaagagcaaaagggggcactattaaccattgggtcagggcaacaggtcaaaatggagacctaccctgggacttctggtcacactagctactgtcaaaatggggcccaaatagacaaagccaaatggaagaaattcccttgacattgaaagtgttggggctctgtggcacccccagttctaggttgggggagcttgggctggtctcatgatgagttctgagggggatgggccagttgggccccccgttccatctaactcaggttcctttcctcccagtccgcctctccaaggaccgatccacactgcaggtgctggactcggccacagggaactggttctctgcctgtttcgacaacttcacagaagctctcgctgagacagcctgtaggcagatgggctacagcaggtaaccaacctgggcctctctcctttttccctccttcctccttcctcctcttcctcctttccttcctcccttcttctctctttcctaaaaattacgggcattggagccaggcagaatggcttttgaatcccagcatttcacttataagcaacatgaagttaaatttcctaagcctcaggttcctcaggagttaattgggggaactaatgccaacctcataggatagttttgcaatgccagtgagagaatgtgtgctgccctccaacacacacacacacacttctagcgtctatgcagtcctctcctttcctttactcctcaaccttcactcctttgtgctggctttgcaagaaactgttcctgcccagtaatacaaaagctaagttaacttattcaaagtttcgttagttaagatttagcttaagtgagcctagtttcagtggggccccatcttcagcaatcccagctctctctgcaaatttcaaaagcagttccaaatctggagtggatgaaaaggtgtaagatgatagtaagagtaatttgcattctatatatttatattcacttgattttggcagaaaaccaaaaagatagttattatatcttatatatagatatatattatatctatttcataaataggctcaaacaaagtaagtaacttgctagggtactagctgggaggtagagggctagaatttgagcccaagacccctaattcttgcgcattaggagttcccacattgtttctgtttctagactgagtaattctttattctcatgtaggacatcatctctaagggaaggggctaatgagatggttgatcactcagagagtttagctggagaggatggaaaagaacccatacattcagttgcagattgagatagcctatctctggcaggcctcagatttcttcaggattctaacagactggacccagagactaggccaaacaaacaaacaaacaaaaactctactaggcagacatcaccaaccaatcacagaactctctcccatggatccctaatacagcctcaaagtccttttcagtaaatgctccaggcagccattacaaatcaatcagaattatttgcctttctcttctctgctcaacgggcttctgctgctctctactttccatagggggcaacttccattaccctctagaaagcacaccccaccaccttcatttcaaggagagtgaggaactcatgcccagcacctgctattctcccctcttcctgcagccacggagcccagcctcgctgcagccagccctgcctccccactgtagtccagtcaactgctgcatcagccgttcctggcacagcaggctgagccttgattatgaaacctgggtgtctccaggggttcttaagatgataggctcctggaatttctgtccttttggagctcagtaaggcaccaaaccacctgagtcttgtgcttcacaaaatcaaagttcatcagaatcattcattgggatggaattggtgaacagaagttaactttcctgggaatgtccatttccaccatattccgtccttctaggtctcagacttctctactttctttcctctctctagatcggaggcccttcttgtcctagaaccataggcatttcaagatgtgggagaccctagggatcatctagtccacgcatcttttttttttttttttgacagagtctcactctgtcacccaggctggagtgcaatggcaccatctctgcttactgcaacctccacctcccaggttcaagtgattctttcgcctcagcctcccaagtagctgggattacaggcacgcaccatcatgcccagctaatttttatatttttgtagagaccgagtttcaccatgttggccaggctggtcttgaactcctgacctcaggtgatccacccacctcggcctcccaaagtgctgggattacaggcgtgagccactgcacccagccccgtgcatctttttatagagggggaaactgaggcttggagagacccagaaaaagaatatgacctgcccaaggccacacatcaaactagtgccagagccagggacagaacctagatcatgaggactcttaaaatgcactctagtcctcccaggtctgagacttgggtccttccaggaagtgccagcattcctgcctgagaatgtgccaatccaccagtattgccaatgactcagccctccatggagagcttctactaacattactagcatagttagggatggaaggaaaagatttagaagaggcagattcagtaaaggaacaatcagagagatggaattaatcaaggaaggcttcctggaggaggaaaaacttcaacccaaggtttgaaagtagcaagcatggattagcagggagaaagagggagagtggtccagttgagagaaacgtttgtctggattcatatgaagacagatctagtcctgttctattaaatatctctaagggggccaaaaacatacccccgctatcaaagtcagaccagatgctttgtttggagaacgaaatatccacattccaactccctcccaggtgagaagggagctaacctgagcccctatgcctctttgtttccctgctgtgaaccagaagacattgctgggatatttgaaatagggacagagctgggaatatggaaaggagacccctaacatttctccagggctctgggttctggatttggattccccacccaagaaagcaagttacatcagcaatgcactgagggttgagtcctgggatgccaagggtcggttctttattgtatagcaaagcaggccccatcttcactgactaagaccatctccactccctggccactccccaccaagcattctctgccactctttctcctgaaagtgggggccaactctaccatcttgttctaaccccctgccccagctcacaactctctctccctcttgatgtgagcagcaaacccactttcagagctgtggagattggcccagaccaggatctggatgttgttgaaatcacagaaaacagccaggagcttcgcatgcggaactcaagtgggtaagtgaggggacaccttctggcctacagaaggcccccacatggacgctgctcttcaggttgcaaccagctcacctggaaccccaagcagccaggggaatgtaagcagacatcaggaagaactcctagccagatggatcattcaatgccaagagctatagactcacattttggagaggttttctgtgttgacttgtttttaatacaatggacagctggacaaagtgtgttgtcctactcagagccagagggatggataatgtgacctttccatcaatctggatagtaaatagtttttgctactgctgtaggttttctaataaattgcccaataggcaagattccaaagtcactttgtccttccctaccacttacccagccagagctccccaccttcttgatgctccagggaagaggctccatggcccttgtgggtggcctgttcctgagcctcgccaccctgtgttagagcagagcatccagatgaaatctgtcacactgtggcaaagtggctcagagaggaggctggcttcctagcattcagggacgttgctgagggccgcttattcaccgaaaataaatcttgaaaaggacagggctggtagcagaatgatcctttacctaaaattctatcaaaatcccattcttccatttggaaagcccacagtgtcacagactctgttccgggctctgtcctcttccctcttgggtcccaggagcccaggctgggctttgaagcaggcagggcccagcacacagtaggtactcagcagtgggggtgttgaatccaatcaaacggaagtgtcaatgcaggaaatgcaatggatgtcaatgcagtctccaaatgttccccactgtgcagcttccacattcccgaggtattgggaggggacttgaattaacagcttcgggaggcctgagtccctgcctcccagctgaggaagaagcttaaatcacagggcgctgtgtctgtcttccaggccctgtctctcaggctccctggtctccctgcactgtcttggtgagtacccccaatctctgagggtttggggcctgggccagcaatgagcagggaggaagaccttcatcttcactcctaaatttctgggactccaagtttcattctgccttggtctacagcccttgggcttgtcggtcaatgccccctcgagttgttggtggccttgggcaggtcacattctttttctgggtctttccaagccccagtttcccccttctaccatctgtgcatggctccatgacctaagtggagacctgggagagagtgttaggaagaccgaaaagggcaggacggggcctccactgcctcccatccctggtccgggcccacatagccttctttgtcacaatcagctcaggtatccaagatcagattacccacattcattatttgagcaactattcattgaacagttagaatatgtctcactctgtcagttgctggctagaagtagaaagtaccagatgagtgaaataattggccactatccttggtagctgatgactaagtaagagagagatgcaagacaacatgtggaaaatgccaaactgagtagcagtcacagttgacatgctgcagagagagctggccgggggtcagaagacctgggcaccagtcctgttcatttccagtgtggcctcgagtcattcacctgacctccctgaagttcattttcccaagaagttgtttagtccaactgcccatcaaggatctttagggacccttctagctctaacagaggagatcagaaaagaaaacaagcaatgtggctcagctcatcctacaagcttcatagagaactgagactggcctggaagcatagccagaaattagaacgcctaagggaagaaggtcacaacgctgcctctgcaatttaggagtgtatatgctttcctgcaggatgttgagagtttcattcattatcgtatgccccctaccccggccccacaatacctagtgcgtgggatctgacacgtggtggctggtcaatgaatgaatgaatgaatggtcacaccatctgaggttctgcactgagtagccctgaaggcttgaagcagcataagtgacaggtcctcccttgaggggcctctgttttaccaataagccaagacctaagctcaacaacactgaaagggtggccaatacccaggacagcctgtgggaattccagagaaagggagattcccagggactgggggcccaggctaaacactgaaaaatgcatctgtaggctcaaggaggaaaagcccatgtctgtctgtcttgcccaccactctctcccagcacccagcactgccccaggacagagagcacttgacacaagttggttagattaatgaatgatttagagttcagtggtccccaacctttttggcacaagagactggttgcatggaagacaatttttccgcaaaccaagagggggatagagagcattagattctctcttttttttttttttgagaccaagtctggctcttgtcactcagcctggagtaaagtgttgcgatctcggctcactgcaacctccgcctcctggattcaagcgattctcctgcctcagccccctaaatagctgggattacaggcacccgtcaccagcccagctgggactataggcatgtgccaccatgcccggctaatttttgtatttttagtagagacggcgtttcaccatgttggccaggctagtctcgaactcctgacctcaggtgatctgcccgcctgagcctcccaaagtgctgggattacaggcatgagctgcctcacccagcctaaagtctcataaggaacgtacagcatagatccctcacatgtgcagttcacaataaggttgtgctcctacaagaatctaacgccacctctgatctgacaggaggtgaagctcaggtggtcatgctcgcttgtccctgccactcacttcctaatgtacagccaggttcctaacaggccacgaaccagtgggaagggcatctttttggatcaaaaacagaattactttttagagaactacaagcagatcaatttggctagacagagactttatatgaaacagcaggaggctgctaggaggagtggaaactctactttgccctcaagggagatcccgaagggctttgcaggagcgggcaaggtggcatgaagaaagcagtgtttgaaatcaggtggtatttgaaaagcccagcccttccccttagaatggcccttctaccatctgtgcatggctccacaaccgtggtggtggctgccagaagaattggaaaggcagagcatgggtggagaggggggacctgagggctttacaggagttccgggggtggtgagggtgtgaaagccaggtcagtcagtaggaagacaggatgtcagattgagagactcccctggccggggaaacagacttggagaagggggagttttggatgagacagtccacttccgagtcacaaaatagcttgtgggtgtctgtttactgttactcagtgggagtggctggggacacgccacctgggcagggctttcgtaattctgcatcacttgtgaaggtcacagattcccagcacaacggacacacccatgttcatagtctgaactcctaaacacatcttaaaccaaaataaaaaaaaaagaaagaaagaaagaaaaaggagagggaggtttgaggaaagcctatggtctgggacactcaatacctcccatgaatatctcatattgggctggtcctctctccactctggccccagccataagggccctgcttagagcagattttgggtgctgagtggaggcagcctcatccccaacagcctgacttcctgcctcctccctgcctctgcctgtgtccagcctgtgggaagagcctgaagaccccccgtgtggtgggtgtggaggaggcctctgtggattcttggccttggcaggtcagcatccagtacgacaaacagcacgtctgtggagggagcatcctggacccccactgggtcctcacggcagcccactgcttcaggtaagaccccagctgtaaggaggtctctggggaccaaggccagtcagggaccagagagcttggggtcctgtctcctggcaccgtccttctcttcactctcccactagagacgttttccaggttgtggtggccccaatgagacaatggccatgatgccctttgttaggcttttgggtgtctgagcagagggtgctggtcaccaagcatggcctcttcctggtgggacaccagcagatacccagagtcctcaccccacccccatatcgttcaagctacaaaagctcttcccacctgcctcaacttccaagaactcactctctttttgcttgtttccaggaagttgttccagggtctagagtcatagccacgtcctcattatgtctggaaactttaaaaaaattaaagagcataggttcctttcagtccacagagaagcctggccttacctcagggaagggctactcccagacccccttcactttttttttttttttttttttttttttttttgagacagagtcttgctctgttgcttaggctggagcgcagcagcatgatcttggctcactgcaacctccgcctcctgagttcaagcaattctcctgcctcagcttcccaagtagctgggactataggcatgggccaccatgcccggctaatttttgtatttttggtagagacagggtttcaccatgttggccaggctgatctctaactcctgacctcaagtgatctgcccacctcagcctcccaaactgctgggattacaggcatgagccagggcatccggcttttatttattcattcattcaatatctaatgagcacctaccaggtaccaaacaccagatgatgcgcccaagttcattagaccccaccgctgtcttcaaggcactcatgatctaggccagcgttttttaaccactttttttttttttttttttgagattctggtgagagctataaattctttcctggaaaaacatctctgcacactaagctgtgcctggcattgggaaaaagaaagcacgtaatgtaactgacagcatgagtaacacagtgagaaaggttggaggagagagcgccaggacctcagaactcaggcattagaggagccccttccccagccctccttgaggtttcgttgggcaggtttcactgaggaaaaagggtcaaatccctttttcgaatttgacttcttgtaagtgccagaagactgccccttctccaccatccctgcctcaccatcatctttcctcccaaggcagtgacatccagcaccccgatccctagggccctggggacccagcctttggcaaagtctcctcaggcttggatcaggcctgaacccagctgtctctacccccaggaaacataccgatgtgttcaactggaaggtgcgggcaggctcagacaaactgggcagcttcccatccctggctgtggccaagatcatcatcattgaattcaaccccatgtaccccaaagacaatgacatcgccctcatgaagctgcagttcccactcactttctcaggtgagaagcagggcccaaggccactcaagcctcttacatcagttttcacgcccactctgctattagctcactgaccgcccttggcacataatgtctcctctcaagtcctcagcttgcccatttgtctctaatacgtcagcctaacatcactgatgccatgaggcctcctcaagctgtcagctaacacctccactccattccctgccagagattcttccaaggcctgtcttccctatgtggagcccctcgagtgagaactggagtttcatccaatcttggagttttaggagaccttttaaaaagattatcgagctaattccccaccactgaccaacacgcaagagcctgctcagtatccctgccaaggagtcattgtgcccctgtttgctctcctccaggggcagggaacccattacctgtgaggcagcccacagagtctttgaacagctctgttggatgccttgtgcttatactgaaatgtatttagatcaggattcccaactgtggggtccacaagacactggccccttggagaagagaggattccattgtcaaataagtttggggaacattttcatactacagctcccttcttggaacacattagtttattaaaggtaggagaagtttttaaaataatctgttttattgcgtttaacctacattttttaaatttatttgaccacagaatccttttttcatgctacttctattagcatcccatagaacaagtgttctagagaccctggtgtgacccctttcagagagcttaactgccaggctctcctgagccctggtgtgtgtttcaagatttgtgcctgggaattgttttaatcaggtatggcaaggtgacagatacagacacagctatctttgaaagaagagtttattatttataattcctgagagaaagggacataccccaccccccaacacagggacacccggggaagcagctgggtccaccaggaggcaggagtgaggggaaggcatggcccagagccacctgtggcttccatgggcaggtctggccaaggtagggtaggcaagattgagcatgctcaggattggatagtgtggacaattctctaggctatagatgtcagcctctggttgtctagtatctgtccctggggtgatttagggcagggaaaatattggcttggtgtctgagagtcagataaaggaagtggttggggatatgggctttgggttggctggtttgcctattaaaggcgtgcccaaagccaagttgtttactatctgcaggaattagctaacccagtctctcccagaccagcaagatccccataatcataaagcatcataatttacagaaaattaacacttatgatgaataaaagatctccttcttcctctgtgctcctggcaggcacagtcaggcccatctgtctgcccttctttgatgaggagctcactccagccaccccactctggatcattggatggggctttacgaagcagaatggaggtaagtcctgggtgcaggaccacagggcaggagatgcccttgtatgagggagcagcttccagaagtaatgggaaggaggaccacccttcagagaaacccatcctggaggaccaagcaccaaggcgccaggcagaaagcaaagtggtttggcaatccagggctgggggatagaaggcaaggatgggaatgtgagtgtttttaccctcccagggaagatgtctgacatactgctgcaggcgtcagtccaggtcattgacagcacacggtgcaatgcagacgatgcgtaccagggggaagtcaccgagaagatgatgtgtgcaggcatcccggaagggggtgtggacacctgccaggtggggcctccaagaatcatggggagttctaagaatagggtttaggtcctagagagatgagaaaacccagaggctgcatgccctacaggaagccttgcatatcatgggcactcaatgtgtgatgatgggaggaagagagggagggaaggaaaggatagtcagataaaagtgtaccaatagatgagtgggtggatggatggatgcagacaagcagagagatttcaaatgtctctttcacattcgaagatgatgttactggcctggcatggtggctcacgcttgtaatcccagcactttgggaggctgaggcgggcaggtgatttgaggtcaggaattcaagaccagcctggccaacatggtgaaatcccatctctactaaaaagaatacaaaaattagctgggcgtggtggcacgtgcctgtaatcccagctacttgggaggctgaggcaggagaattgcttgaacccaggaggcagaggttgcagtaagctgagattgcgccactgcactccagcctgggtgacccagcaagactccatctgaaaacaacaacaacaacaaagatgacattactcatccaccccacccacccttctcactagctacagaatgattagccccttgaggtcaggaatcccaggtctattttctctgtgactctccccaagctgctgaactacactaggaaagaattaccgcctgcagaatgctggaagcacatctgtgtgtgccctcaccccggcctcattggccatcaggactgcttagcaatccctgtagaccttcttcctcccccatacttccagaggatcttctgaactattttctttttttattttttcttttatgttttttaacagagacagggtcactatgttgcccagtctggtctcaaactcctgggttcaagggattctcccacctcagctttccaaaatgctgggattacaggcatgagccatcgtgcttggcctgaaccattttcattaaaacccctaccctactctcacctccatttccagtcattaaattccttcatttaagaggcatctcttagtcatcgcatgtgtgccatgaacatggtagtctttggagacccctcagggagctcacagtggttgggggaaaggggggcattaaacagacatttaagctatagttttgggttcagagggaggaagccccaggggctaaaacagctgataaggactcccagataagtgcacttttcactatctggcattttcttgttttgttatttgcttgttcactgtctctcaccccatttgatcctaagctttctgagggcagggatctttgttttttttcatcagttggatcccaattgcttagaacactacctggcacaaaataggcactctataagtgattacacaaattttggaacgactaggttaaacaatgataaccaggcttttttttttttttttgagactgagtctcactctgttgcccaggctagagtgaagtggtttgatctcggctcactgcagcctccgcctctgggttcgaatgattctccacctcagcctcctgagtagctgggattacaggtgcctgccactatgcccagctaatttttgtatttgtagtagagacgggtttcaccatgttggccaggctggtcttgaactcctgacctcaagtgattcacccgcctcagcctcccaaggtgctgggattacaggtgtgagccaccgctcctggccaacaaccaggcttttttaagacatcactcagagcctttaatttgctaatgtgagttgtgaatctctgagagaaggctaacggcatgcttgcaacttacttgtccacagacaagcctttctgccccagaagagaagaccattctagggtgctaatgagcaaagagggtgagggtggaatatcggagagcagcagggagtgcaggggaacagataggccagttcagggagcagagaaggagaagcccccccacctcacctgccctccccagcagtctctgttctggtctctcacagggtgacagtggtgggcccctgatgtaccaatctgaccagtggcatgtggtgggcatcgttagttggggctatggctgcgggggcccgagcaccccaggagtatacaccaaggtctcagcctatctcaactggatctacaatgtctggaaggtaaggtacctttgccctacccactgtgccttccctccagtcctctacctggggggtgccaatccatcctcaggtttgatttaaatggttctgacaactctttacatcccaaataactttccctccaagcaagggacagcctgagattgcactattaaggctgaaattccttaggtcagagatttctgataaatgcaaataccttagggaatagaacacaccaagcctttctttctcttttctgacagaatgagactatcagatcctttctagagagaagattctgataaggaagagagtggaaaggctcatgagacctcctggccctctgcagggtagggagagaagcaaagtgtttcagaaaaggaagactcacgttacacatgtcaccactttgtccagtttcagataatctgactttctcttcatcggtctctcttattctaggctgagctgtaacgctgccgtcccccacatccagaagctgcttcccttcagacctacctacggcatgacccctcaaagtcagatatgggacaagagcctccttgaacaaactc

SEQ ID NO: 13 - DNA, 15159 bp, Artificial Sequence
  Recombinant polynucleotide
ccacccgcacacactacagtcgagataacttcgtataatgtatgctatacgaagttatgctagtaactataacggtcctaaggtagcgagctagccaagtctgtgtgctaccaagtagcaaaactgagcctggaactcacacatgcgtgtctgagagcccagcactatcgccaggaaaacccagcgtctccctgctcaagcctgaccctcagccctctctgcctctccctgcacttgccttccagtcaaggtgattctggataaatactacttcctctgcgggcagcctctccacttcatcccgaggaagcagctgtgtgacggagagctggactgtcccttgggggaggacgaggagcactgtgtcaagagcttccccgaagggcctgcagtggcaggtgagtgcagggtctgaggcacaagagaagtgggcccagcaggaggtctgctcaggcccccacggcccactgcatagtatctgccccctacttgtcacttttcatccttgttgtataaggttctttgtttgtttgtttgttgttgttttgaggcagagtgctctgtggcccaagatggagtgcagtgtcttggtctcggctcactgcaacctctgcctcccagtttcaagtgattcttctgcctcagcctcatgagtagctgggattacaggtgccagccaccacgcctggctaatttttatatttttagtagagacggggttttgccacattggtcaggctgatcttgaactcctgacctcaggtgatctgcccgcctcagcctcccaaagtgctgggattacaggcgtgagccaccgtgcccagctgtgtaagtttcttgagagcaggaccctgtcttgtctacctttaaatcctagtacttaacacacagcaaacagtaactatttgatgaccaaatgtgagccagaaaggacaggaaattgtaactgaggctgccccatgcgtgctgcgcctggtggatttcaggcagagggctagactgggtgaccttggggcattcctcctttctatgaaatttgttatttcaaggagactagaaaagagacttctcagccacttcgccagctattggtccttctattcattagtgtttgctgagacatgctatgtgacaggactgagccaggtcctttcaatggataggagatgttttgagcataaaatccacgttctctcttgggctgggctcttctaccttcttccccctggtgcttgggctctgaagaaaaaaagataggtaggagatgagtgatggggcttctgagggcagggctgagtgactttctgtgtatttgctctttctttatcagaagtcaaatgcccacaggcacctgtcatcctactgccagtaggacttctcactcaaccttcccctctgaccttacttggagaaggacttaggtccctctctcagacatttccccaggctgggcaagttgtgtggaccatggatgggtatgtggtccatacaatttaaacaagctgtatatggtcgctgggtagagtgaccacataattgatcatcaaaactgatacctgtaagagcaaaagggggcactattaaccattgggtcagggcaacaggtcaaaatggagacctaccctgggacttctggtcacactagctactgtcaaaatggggcccaaatagacaaagccaaatggaagaaattcccttgacattgaaagtgttggggctctgtggcacccccagttctaggttgggggagcttgggctggtctcatgatgagttctgagggggatgggccagttgggccccccgttccatctaactcaggttcctttcctcccagtccgcctctccaaggaccgatccacactgcaggtgctggactcggccacagggaactggttctctgcctgtttcgacaacttcacagaagctctcgctgagacagcctgtaggcagatgggctacagcaggtaaccaacctgggcctctctcctttttccctccttcctccttcctcctcttcctcctttccttcctcccttcttctctctttcctaaaaattacgggcattggagccaggcagaatggcttttgaatcccagcatttcacttataagcaacatgaagttaaatttcctaagcctcaggttcctcaggagttaattgggggaactaatgccaacctcataggatagttttgcaatgccagtgagagaatgtgtgctgccctccaacacacacacacacacttctagcgtctatgcagtcctctcctttcctttactcctcaaccttcactcctttgtgctggctttgcaagaaactgttcctgcccagtaatacaaaagctaagttaacttattcaaagtttcgttagttaagatttagcttaagtgagcctagtttcagtggggccccatcttcagcaatcccagctctctctgcaaatttcaaaagcagttccaaatctggagtggatgaaaaggtgtaagatgatagtaagagtaatttgcattctatatatttatattcacttgattttggcagaaaaccaaaaagatagttattatatcttatatatagatatatattatatctatttcataaataggctcaaacaaagtaagtaacttgctagggtactagctgggaggtagagggctagaatttgagcccaagacccctaattcttgcgcattaggagttcccacattgtttctgtttctagactgagtaattctttattctcatgtaggacatcatctctaagggaaggggctaatgagatggttgatcactcagagagtttagctggagaggatggaaaagaacccatacattcagttgcagattgagatagcctatctctggcaggcctcagatttcttcaggattctaacagactggacccagagactaggccaaacaaacaaacaaacaaaaactctactaggcagacatcaccaaccaatcacagaactctctcccatggatccctaatacagcctcaaagtccttttcagtaaatgctccaggcagccattacaaatcaatcagaattatttgcctttctcttctctgctcaacgggcttctgctgctctctactttccatagggggcaacttccattaccctctagaaagcacaccccaccaccttcatttcaaggagagtgaggaactcatgcccagcacctgctattctcccctcttcctgcagccacggagcccagcctcgctgcagccagccctgcctccccactgtagtccagtcaactgctgcatcagccgttcctggcacagcaggctgagccttgattatgaaacctgggtgtctccaggggttcttaagatgataggctcctggaatttctgtccttttggagctcagtaaggcaccaaaccacctgagtcttgtgcttcacaaaatcaaagttcatcagaatcattcattgggatggaattggtgaacagaagttaactttcctgggaatgtccatttccaccatattccgtccttctaggtctcagacttctctactttctttcctctctctagatcggaggcccttcttgtcctagaaccataggcatttcaagatgtgggagaccctagggatcatctagtccacgcatcttttttttttttttttgacagagtctcactctgtcacccaggctggagtgcaatggcaccatctctgcttactgcaacctccacctcccaggttcaagtgattctttcgcctcagcctcccaagtagctgggattacaggcacgcaccatcatgcccagctaatttttatatttttgtagagaccgagtttcaccatgttggccaggctggtcttgaactcctgacctcaggtgatccacccacctcggcctcccaaagtgctgggattacaggcgtgagccactgcacccagccccgtgcatctttttatagagggggaaactgaggcttggagagacccagaaaaagaatatgacctgcccaaggccacacatcaaactagtgccagagccagggacagaacctagatcatgaggactcttaaaatgcactctagtcctcccaggtctgagacttgggtccttccaggaagtgccagcattcctgcctgagaatgtgccaatccaccagtattgccaatgactcagccctccatggagagcttctactaacattactagcatagttagggatggaaggaaaagatttagaagaggcagattcagtaaaggaacaatcagagagatggaattaatcaaggaaggcttcctggaggaggaaaaacttcaacccaaggtttgaaagtagcaagcatggattagcagggagaaagagggagagtggtccagttgagagaaacgtttgtctggattcatatgaagacagatctagtcctgttctattaaatatctctaagggggccaaaaacatacccccgctatcaaagtcagaccagatgctttgtttggagaacgaaatatccacattccaactccctcccaggtgagaagggagctaacctgagcccctatgcctctttgtttccctgctgtgaaccagaagacattgctgggatatttgaaatagggacagagctgggaatatggaaaggagacccctaacatttctccagggctctgggttctggatttggattccccacccaagaaagcaagttacatcagcaatgcactgagggttgagtcctgggatgccaagggtcggttctttattgtatagcaaagcaggccccatcttcactgactaagaccatctccactccctggccactccccaccaagcattctctgccactctttctcctgaaagtgggggccaactctaccatcttgttctaaccccctgccccagctcacaactctctctccctcttgatgtgagcagcaaacccactttcagagctgtggagattggcccagaccaggatctggatgttgttgaaatcacagaaaacagccaggagcttcgcatgcggaactcaagtgggtaagtgaggggacaccttctggcctacagaaggcccccacatggacgctgctcttcaggttgcaaccagctcacctggaaccccaagcagccaggggaatgtaagcagacatcaggaagaactcctagccagatggatcattcaatgccaagagctatagactcacattttggagaggttttctgtgttgacttgtttttaatacaatggacagctggacaaagtgtgttgtcctactcagagccagagggatggataatgtgacctttccatcaatctggatagtaaatagtttttgctactgctgtaggttttctaataaattgcccaataggcaagattccaaagtcactttgtccttccctaccacttacccagccagagctccccaccttcttgatgctccagggaagaggctccatggcccttgtgggtggcctgttcctgagcctcgccaccctgtgttagagcagagcatccagatgaaatctgtcacactgtggcaaagtggctcagagaggaggctggcttcctagcattcagggacgttgctgagggccgcttattcaccgaaaataaatcttgaaaaggacagggctggtagcagaatgatcctttacctaaaattctatcaaaatcccattcttccatttggaaagcccacagtgtcacagactctgttccgggctctgtcctcttccctcttgggtcccaggagcccaggctgggctttgaagcaggcagggcccagcacacagtaggtactcagcagtgggggtgttgaatccaatcaaacggaagtgtcaatgcaggaaatgcaatggatgtcaatgcagtctccaaatgttccccactgtgcagcttccacattcccgaggtattgggaggggacttgaattaacagcttcgggaggcctgagtccctgcctcccagctgaggaagaagcttaaatcacagggcgctgtgtctgtcttccaggccctgtctctcaggctccctggtctccctgcactgtcttggtgagtacccccaatctctgagggtttggggcctgggccagcaatgagcagggaggaagaccttcatcttcactcctaaatttctgggactccaagtttcattctgccttggtctacagcccttgggcttgtcggtcaatgccccctcgagttgttggtggccttgggcaggtcacattctttttctgggtctttccaagccccagtttcccccttctaccatctgtgcatggctccatgacctaagtggagacctgggagagagtgttaggaagaccgaaaagggcaggacggggcctccactgcctcccatccctggtccgggcccacatagccttctttgtcacaatcagctcaggtatccaagatcagattacccacattcattatttgagcaactattcattgaacagttagaatatgtctcactctgtcagttgctggctagaagtagaaagtaccagatgagtgaaataattggccactatccttggtagctgatgactaagtaagagagagatgcaagacaacatgtggaaaatgccaaactgagtagcagtcacagttgacatgctgcagagagagctggccgggggtcagaagacctgggcaccagtcctgttcatttccagtgtggcctcgagtcattcacctgacctccctgaagttcattttcccaagaagttgtttagtccaactgcccatcaaggatctttagggacccttctagctctaacagaggagatcagaaaagaaaacaagcaatgtggctcagctcatcctacaagcttcatagagaactgagactggcctggaagcatagccagaaattagaacgcctaagggaagaaggtcacaacgctgcctctgcaatttaggagtgtatatgctttcctgcaggatgttgagagtttcattcattatcgtatgccccctaccccggccccacaatacctagtgcgtgggatctgacacgtggtggctggtcaatgaatgaatgaatgaatggtcacaccatctgaggttctgcactgagtagccctgaaggcttgaagcagcataagtgacaggtcctcccttgaggggcctctgttttaccaataagccaagacctaagctcaacaacactgaaagggtggccaatacccaggacagcctgtgggaattccagagaaagggagattcccagggactgggggcccaggctaaacactgaaaaatgcatctgtaggctcaaggaggaaaagcccatgtctgtctgtcttgcccaccactctctcccagcacccagcactgccccaggacagagagcacttgacacaagttggttagattaatgaatgatttagagttcagtggtccccaacctttttggcacaagagactggttgcatggaagacaatttttccgcaaaccaagagggggatagagagcattagattctctcttttttttttttttgagaccaagtctggctcttgtcactcagcctggagtaaagtgttgcgatctcggctcactgcaacctccgcctcctggattcaagcgattctcctgcctcagccccctaaatagctgggattacaggcacccgtcaccagcccagctgggactataggcatgtgccaccatgcccggctaatttttgtatttttagtagagacggcgtttcaccatgttggccaggctagtctcgaactcctgacctcaggtgatctgcccgcctgagcctcccaaagtgctgggattacaggcatgagctgcctcacccagcctaaagtctcataaggaacgtacagcatagatccctcacatgtgcagttcacaataaggttgtgctcctacaagaatctaacgccacctctgatctgacaggaggtgaagctcaggtggtcatgctcgcttgtccctgccactcacttcctaatgtacagccaggttcctaacaggccacgaaccagtgggaagggcatctttttggatcaaaaacagaattactttttagagaactacaagcagatcaatttggctagacagagactttatatgaaacagcaggaggctgctaggaggagtggaaactctactttgccctcaagggagatcccgaagggctttgcaggagcgggcaaggtggcatgaagaaagcagtgtttgaaatcaggtggtatttgaaaagcccagcccttccccttagaatggcccttctaccatctgtgcatggctccacaaccgtggtggtggctgccagaagaattggaaaggcagagcatgggtggagaggggggacctgagggctttacaggagttccgggggtggtgagggtgtgaaagccaggtcagtcagtaggaagacaggatgtcagattgagagactcccctggccggggaaacagacttggagaagggggagttttggatgagacagtccacttccgagtcacaaaatagcttgtgggtgtctgtttactgttactcagtgggagtggctggggacacgccacctgggcagggctttcgtaattctgcatcacttgtgaaggtcacagattcccagcacaacggacacacccatgttcatagtctgaactcctaaacacatcttaaaccaaaataaaaaaaaaagaaagaaagaaagaaaaaggagagggaggtttgaggaaagcctatggtctgggacactcaatacctcccatgaatatctcatattgggctggtcctctctccactctggccccagccataagggccctgcttagagcagattttgggtgctgagtggaggcagcctcatccccaacagcctgacttcctgcctcctccctgcctctgcctgtgtccagcctgtgggaagagcctgaagaccccccgtgtggtgggtgtggaggaggcctctgtggattcttggccttggcaggtcagcatccagtacgacaaacagcacgtctgtggagggagcatcctggacccccactgggtcctcacggcagcccactgcttcaggtaagaccccagctgtaaggaggtctctggggaccaaggccagtcagggaccagagagcttggggtcctgtctcctggcaccgtccttctcttcactctcccactagagacgttttccaggttgtggtggccccaatgagacaatggccatgatgccctttgttaggcttttgggtgtctgagcagagggtgctggtcaccaagcatggcctcttcctggtgggacaccagcagatacccagagtcctcaccccacccccatatcgttcaagctacaaaagctcttcccacctgcctcaacttccaagaactcactctctttttgcttgtttccaggaagttgttccagggtctagagtcatagccacgtcctcattatgtctggaaactttaaaaaaattaaagagcataggttcctttcagtccacagagaagcctggccttacctcagggaagggctactcccagacccccttcactttttttttttttttttttttttttttttttgagacagagtcttgctctgttgcttaggctggagcgcagcagcatgatcttggctcactgcaacctccgcctcctgagttcaagcaattctcctgcctcagcttcccaagtagctgggactataggcatgggccaccatgcccggctaatttttgtatttttggtagagacagggtttcaccatgttggccaggctgatctctaactcctgacctcaagtgatctgcccacctcagcctcccaaactgctgggattacaggcatgagccagggcatccggcttttatttattcattcattcaatatctaatgagcacctaccaggtaccaaacaccagatgatgcgcccaagttcattagaccccaccgctgtcttcaaggcactcatgatctaggccagcgttttttaaccactttttttttttttttttttgagattctggtgagagctataaattctttcctggaaaaacatctctgcacactaagctgtgcctggcattgggaaaaagaaagcacgtaatgtaactgacagcatgagtaacacagtgagaaaggttggaggagagagcgccaggacctcagaactcaggcattagaggagccccttccccagccctccttgaggtttcgttgggcaggtttcactgaggaaaaagggtcaaatccctttttcgaatttgacttcttgtaagtgccagaagactgccccttctccaccatccctgcctcaccatcatctttcctcccaaggcagtgacatccagcaccccgatccctagggccctggggacccagcctttggcaaagtctcctcaggcttggatcaggcctgaacccagctgtctctacccccaggaaacataccgatgtgttcaactggaaggtgcgggcaggctcagacaaactgggcagcttcccatccctggctgtggccaagatcatcatcattgaattcaaccccatgtaccccaaagacaatgacatcgccctcatgaagctgcagttcccactcactttctcaggtgagaagcagggcccaaggccactcaagcctcttacatcagttttcacgcccactctgctattagctcactgaccgcccttggcacataatgtctcctctcaagtcctcagcttgcccatttgtctctaatacgtcagcctaacatcactgatgccatgaggcctcctcaagctgtcagctaacacctccactccattccctgccagagattcttccaaggcctgtcttccctatgtggagcccctcgagtgagaactggagtttcatccaatcttggagttttaggagaccttttaaaaagattatcgagctaattccccaccactgaccaacacgcaagagcctgctcagtatccctgccaaggagtcattgtgcccctgtttgctctcctccaggggcagggaacccattacctgtgaggcagcccacagagtctttgaacagctctgttggatgccttgtgcttatactgaaatgtatttagatcaggattcccaactgtggggtccacaagacactggccccttggagaagagaggattccattgtcaaataagtttggggaacattttcatactacagctcccttcttggaacacattagtttattaaaggtaggagaagtttttaaaataatctgttttattgcgtttaacctacattttttaaatttatttgaccacagaatccttttttcatgctacttctattagcatcccatagaacaagtgttctagagaccctggtgtgacccctttcagagagcttaactgccaggctctcctgagccctggtgtgtgtttcaagatttgtgcctgggaattgttttaatcaggtatggcaaggtgacagatacagacacagctatctttgaaagaagagtttattatttataattcctgagagaaagggacataccccaccccccaacacagggacacccggggaagcagctgggtccaccaggaggcaggagtgaggggaaggcatggcccagagccacctgtggcttccatgggcaggtctggccaaggtagggtaggcaagattgagcatgctcaggattggatagtgtggacaattctctaggctatagatgtcagcctctggttgtctagtatctgtccctggggtgatttagggcagggaaaatattggcttggtgtctgagagtcagataaaggaagtggttggggatatgggctttgggttggctggtttgcctattaaaggcgtgcccaaagccaagttgtttactatctgcaggaattagctaacccagtctctcccagaccagcaagatccccataatcataaagcatcataatttacagaaaattaacacttatgatgaataaaagatctccttcttcctctgtgctcctggcaggcacagtcaggcccatctgtctgcccttctttgatgaggagctcactccagccaccccactctggatcattggatggggctttacgaagcagaatggaggtaagtcctgggtgcaggaccacagggcaggagatgcccttgtatgagggagcagcttccagaagtaatgggaaggaggaccacccttcagagaaacccatcctggaggaccaagcaccaaggcgccaggcagaaagcaaagtggtttggcaatccagggctgggggatagaaggcaaggatgggaatgtgagtgtttttaccctcccagggaagatgtctgacatactgctgcaggcgtcagtccaggtcattgacagcacacggtgcaatgcagacgatgcgtaccagggggaagtcaccgagaagatgatgtgtgcaggcatcccggaagggggtgtggacacctgccaggtggggcctccaagaatcatggggagttctaagaatagggtttaggtcctagagagatgagaaaacccagaggctgcatgccctacaggaagccttgcatatcatgggcactcaatgtgtgatgatgggaggaagagagggagggaaggaaaggatagtcagataaaagtgtaccaatagatgagtgggtggatggatggatgcagacaagcagagagatttcaaatgtctctttcacattcgaagatgatgttactggcctggcatggtggctcacgcttgtaatcccagcactttgggaggctgaggcgggcaggtgatttgaggtcaggaattcaagaccagcctggccaacatggtgaaatcccatctctactaaaaagaatacaaaaattagctgggcgtggtggcacgtgcctgtaatcccagctacttgggaggctgaggcaggagaattgcttgaacccaggaggcagaggttgcagtaagctgagattgcgccactgcactccagcctgggtgacccagcaagactccatctgaaaacaacaacaacaacaaagatgacattactcatccaccccacccacccttctcactagctacagaatgattagccccttgaggtcaggaatcccaggtctattttctctgtgactctccccaagctgctgaactacactaggaaagaattaccgcctgcagaatgctggaagcacatctgtgtgtgccctcaccccggcctcattggccatcaggactgcttagcaatccctgtagaccttcttcctcccccatacttccagaggatcttctgaactattttctttttttattttttcttttatgttttttaacagagacagggtcactatgttgcccagtctggtctcaaactcctgggttcaagggattctcccacctcagctttccaaaatgctgggattacaggcatgagccatcgtgcttggcctgaaccattttcattaaaacccctaccctactctcacctccatttccagtcattaaattccttcatttaagaggcatctcttagtcatcgcatgtgtgccatgaacatggtagtctttggagacccctcagggagctcacagtggttgggggaaaggggggcattaaacagacatttaagctatagttttgggttcagagggaggaagccccaggggctaaaacagctgataaggactcccagataagtgcacttttcactatctggcattttcttgttttgttatttgcttgttcactgtctctcaccccatttgatcctaagctttctgagggcagggatctttgttttttttcatcagttggatcccaattgcttagaacactacctggcacaaaataggcactctataagtgattacacaaattttggaacgactaggttaaacaatgataaccaggcttttttttttttttttgagactgagtctcactctgttgcccaggctagagtgaagtggtttgatctcggctcactgcagcctccgcctctgggttcgaatgattctccacctcagcctcctgagtagctgggattacaggtgcctgccactatgcccagctaatttttgtatttgtagtagagacgggtttcaccatgttggccaggctggtcttgaactcctgacctcaagtgattcacccgcctcagcctcccaaggtgctgggattacaggtgtgagccaccgctcctggccaacaaccaggcttttttaagacatcactcagagcctttaatttgctaatgtgagttgtgaatctctgagagaaggctaacggcatgcttgcaacttacttgtccacagacaagcctttctgccccagaagagaagaccattctagggtgctaatgagcaaagagggtgagggtggaatatcggagagcagcagggagtgcaggggaacagataggccagttcagggagcagagaaggagaagcccccccacctcacctgccctccccagcagtctctgttctggtctctcacagggtgacagtggtgggcccctgatgtaccaatctgaccagtggcatgtggtgggcatcgttagttggggctatggctgcgggggcccgagcaccccaggagtatacaccaaggtctcagcctatctcaactggatctacaatgtctggaaggtaaggtacctttgccctacccactgtgccttccctccagtcctctacctggggggtgccaatccatcctcaggtttgatttaaatggttctgacaactctttacatcccaaataactttccctccaagcaagggacagcctgagattgcactattaaggctgaaattccttaggtcagagatttctgataaatgcaaataccttagggaatagaacacaccaagcctttctttctcttttctgacagaatgagactatcagatcctttctagagagaagattctgataaggaagagagtggaaaggctcatgagacctcctggccctctgcagggtagggagagaagcaaagtgtttcagaaaaggaagactcacgttacacatgtcaccactttgtccagtttcagataatctgactttctcttcatcggtctctcttattctaggctgagctgtaacgctgccgtcccccacatccagaagctgcttcccttcagacctacctacggcatgacccctcaaagtcagatatgggacaagagcctccttgaacaaactc

SEQ ID NO: 14 - protein, 435 aa, Artificial Sequence
  Recombinant protein
MESDSGQPLNNRDIVPFRKPRRPQETFKKVGIPIIAVLLSLIALVIVALLIKVILDKYYFLCGQPLHFIPRKQLCDGELDCPLGEDEEHCVKSFPEGPAVAVRLSKDRSTLQVLDSATGNWFSACFDNFTEALAETACRQMGYSSKPTFRAVEIGPDQDLDVVEITENSQELRMRNSSGPCLSGSLVSLHCLACGKSLKTPRVVGVEEASVDSWPWQVSIQYDKQHVCGGSILDPHWVLTAAHCFRKHTDVFNWKVRAGSDKLGSFPSLAVAKIIIIEFNPMYPKDNDIALMKLQFPLTFSGTVRPICLPFFDEELTPATPLWIIGWGFTKQNGGKMSDILLQASVQVIDSTRCNADDAYQGEVTEKMMCAGIPEGGVDTCQGDSGGPLMYQSDQWHVVGIVSWGYGCGGPSTPGVYTKVSAYLNWIYNVWKAEL

SEQ ID NO: 15 - DNA, 2046 bp, Mus musculus
cagaaacaaggacctcttcattattcaagagtaaaatgtataggccaagaccaatgctatcaccgtcaagattcttcactccctttgcagtagctttcgttgtcataataacggtagggctcctggccatgatggcaggtctacttattcactttttagcttttgacaagaaagcttacttttatcatagcagctttcaaatcctaaacgttgaatacactgaggctttaaactcaccagctacacacgaatacagaaccttgagtgaaagaattgaggctatgattactgatgaatttcgaggatcaagtctaaaaagtgagtttatcaggacacatgttgtcaaactaagaaaagaagggactggtgtggttgcggatgttgtcatgaaatttcgatctagtaaacgtaacaacagaaaggtaatgaaaaccagaattcaatctgtgctacgaagactcagcagctctggaaacttggaaatagccccttcgaatgagataacatcactcactgaccaggatacagaaaatgttttgactcaagaatgtggagcacgtccagaccttataacactgtcagaagagagaatcattggaggcatgcaagctgagcccggtgactggccctggcaagtcagtctacagctcaataatgtccaccactgtggaggtgccctgatcagtaacatgtgggtcctgacagcagctcattgcttcaaaagctatcctaatcctcaatattggacagccacctttggggtttctacaatgagccctaggctgagagtgagagtaagggctattttagcccacgacgggtacagctccgtaactcgtgacaatgacatcgcagttgtacaacttgacagatctgtcgccttttccagaaatatccatagggtatgtctcccagcagcaacccaaaatatcatccctggttctgtcgcatatgttacaggatggggatctctcacatatggaggcaacgcagtcacaaatctacggcaaggagaggtcagaataataagttcagaggaatgcaatacgccagctggttacagtggaagtgtcttgccaggaatgctgtgtgctggaatgcgttcaggggccgtggatgcatgccagggtgattcaggtggcccgctagtacaagaagactcaaggcggctttggtttgttgtgggcattgtgagctggggatatcagtgtggcctcccaaataagccaggcgtgtatactcgagtgacagcctaccgcaactggatcagacagcagacgggaatctagtgcaaccgaggaaaaaacgtgccatgaggtctctgtatccaagtgtgactgactcggatgccatggcttcacatttcaactgcaaaggagactggaaatgccccttctgaacgtcccattacataaatatggtttaactgtttagtatttctttgtcggtacagatttttactttcttgaggaaaaaaaaaacatgaacatggctaagtaagaattatgttaggctagtaacaggaagacatttattacatgggtggtcaggtgtagtagtgagaagtcaggtaagttaagtcaataatttacagaaaataatgtcaggtagtcctaacgttaaatatgtgaggccacagaacaaatagtgttagaactgaagccatcccaagtatttaacatttgttttcaagtgaaactaagaaacagacttacatatagttttaatggtgaattttcattttaaatattttatctacatagaaaagacatatctccttcatgaagaagctgaggtgatgaatcaacacagcctcttcagctatgtttgcaaccacaagatttgtgggaaagaaatccctactaccaacttcctactgttggcattattttttagagtaacacgacgcacaatagcaaaatttaagtaacaaattaaaagttaatgatgaagaagaagtaaagagtttgtttgcaaagacaaaaattaaacagattaatatcaataaatctggagacagaagggtctcagattcatattctctct

SEQ ID NO: 16 - protein, 417 aa, Mus musculus
MYRPRPMLSPSRFFTPFAVAFVVIITVGLLAMMAGLLIHFLAFDKKAYFYHSSFQILNVEYTEALNSPATHEYRTLSERIEAMITDEFRGSSLKSEFIRTHVVKLRKEGTGVVADVVMKFRSSKRNNRKVMKTRIQSVLRRLSSSGNLEIAPSNEITSLTDQDTENVLTQECGARPDLITLSEERIIGGMQAEPGDWPWQVSLQLNNVHHCGGALISNMWVLTAAHCFKSYPNPQYWTATFGVSTMSPRLRVRVRAILAHDGYSSVTRDNDIAVVQLDRSVAFSRNIHRVCLPAATQNIIPGSVAYVTGWGSLTYGGNAVTNLRQGEVRIISSEECNTPAGYSGSVLPGMLCAGMRSGAVDACQGDSGGPLVQEDSRRLWFVVGIVSWGYQCGLPNKPGVYTRVTAYRNWIRQQTGI

SEQ ID NO: 17 - DNA, 2800 bp, Homo sapiens
atttgagtgggaatctcaaagcagttgagtaggcagaaaaaagaacctcttcattaaggattaaaatgtataggccagcacgtgtaacttcgacttcaagatttctgaatccatatgtagtatgtttcattgtcgtcgcaggggtagtgatcctggcagtcaccatagctctacttgtttactttttagcttttgatcaaaaatcttacttttataggagcagttttcaactcctaaatgttgaatataatagtcagttaaattcaccagctacacaggaatacaggactttgagtggaagaattgaatctctgattactaaaacattcaaagaatcaaatttaagaaatcagttcatcagagctcatgttgccaaactgaggcaagatggtagtggtgtgagagcggatgttgtcatgaaatttcaattcactagaaataacaatggagcatcaatgaaaagcagaattgagtctgttttacgacaaatgctgaataactctggaaacctggaaataaacccttcaactgagataacatcacttactgaccaggctgcagcaaattggcttattaatgaatgtggggccggtccagacctaataacattgtctgagcagagaatccttggaggcactgaggctgaggagggaagctggccgtggcaagtcagtctgcggctcaataatgcccaccactgtggaggcagcctgatcaataacatgtggatcctgacagcagctcactgcttcagaagcaactctaatcctcgtgactggattgccacgtctggtatttccacaacatttcctaaactaagaatgagagtaagaaatattttaattcataacaattataaatctgcaactcatgaaaatgacattgcacttgtgagacttgagaacagtgtcacctttaccaaagatatccatagtgtgtgtctcccagctgctacccagaatattccacctggctctactgcttatgtaacaggatggggcgctcaagaatatgctggccacacagttccagagctaaggcaaggacaggtcagaataataagtaatgatgtatgtaatgcaccacatagttataatggagccatcttgtctggaatgctgtgtgctggagtacctcaaggtggagtggacgcatgtcagggtgactctggtggcccactagtacaagaagactcacggcggctttggtttattgtggggatagtaagctggggagatcagtgtggcctgccggataagccaggagtgtatactcgagtgacagcctaccttgactggattaggcaacaaactgggatctagtgcaacaagtgcatccctgttgcaaagtctgtatgcaggtgtgcctgtcttaaattccaaagctttacatttcaactgaaaaagaaactagaaatgtcctaatttaacatcttgttacataaatatggtttaacaaacactgtttaacctttctttattattaaaggttttctattttctccagagaactatatgaatgttgcatagtactgtggctgtgtaacagaagaaacacactaaactaattacaaagttaacaatttcattacagttgtgctaaatgcccgtagtgagaagaacaggaaccttgagcatgtatagtagaggaacctgcacaggtctgatgggtcagaggggtcttctctgggtttcactgaggatgagaagtaagcaaactgtggaaacatgcaaaggaaaaagtgatagaataatattcaagacaaaaagaacagtatgaggcaagagaaataatatgtatttaaaatttttggttactcaatatcttatacttagtatgagtcctaaaattaaaaatgtgaaactgttgtactatacgtataacctaaccttaattattctgtaagaacatgcttccataggaaatagtggataattttcagctatttaaggcaaaagctaaaatagttcactcctcaactgagacccaaagaattatagatatttttcatgatgacccatgaaaaatatcactcatctacataaaggagagactatatctattttatagagaagctaagaaatatacctacacaaacttgtcaggtgctttacaactacatagtactttttaacaacaaaataataattttaagaatgaaaaatttaatcatcgggaagaacgtcccactacagacttcctatcactggcagttatatttttgagcgtaaaagggtcgtcaaacgctaaatctaagtaacgaattgaaagtttaaagagggggaagagttggtttgcaaaggaaaagtttaaatagcttaatatcaatagaatgatcctgaagacagaaaaaactttgtcactcttcctctctcattttctttctctctctctccccttctcatacacatgcctcccccaccaaagaatataatgtaaattaaatccactaaaatgtaatggcatgaaaatctctgtagtctgaatcactaatattcctgagtttttatgagctcctagtacagctaaagtttgcctatgcatgatcatctatgcgtcagagcttcctccttctacaagctaactccctgcatctgggcatcaggactgctccatacatttgctgaaaacttcttgtatttcctgatgtaaaattgtgcaaacacctacaataaagccatctacttttagggaaagggagttgaaaatgcaaccaactcttggcgaactgtacaaacaaatctttgctatactttatttcaaataaattctttttaaaataaaaaaaaaaaaaaaaaaa

SEQ ID NO: 18 - protein, 418 aa, Homo sapiens
MYRPARVTSTSRFLNPYVVCFIVVAGVVILAVTIALLVYFLAFDQKSYFYRSSFQLLNVEYNSQLNSPATQEYRTLSGRIESLITKTFKESNLRNQFIRAHVAKLRQDGSGVRADVVMKFQFTRNNNGASMKSRIESVLRQMLNNSGNLEINPSTEITSLTDQAAANWLINECGAGPDLITLSEQRILGGTEAEEGSWPWQVSLRLNNAHHCGGSLINNMWILTAAHCFRSNSNPRDWIATSGISTTFPKLRMRVRNILIHNNYKSATHENDIALVRLENSVTFTKDIHSVCLPAATQNIPPGSTAYVTGWGAQEYAGHTVPELRQGQVRIISNDVCNAPHSYNGAILSGMLCAGVPQGGVDACQGDSGGPLVQEDSRRLWFIVGIVSWGDQCGLPDKPGVYTRVTAYLDWIRQQTGI

SEQ ID NO: 19 - DNA, 38992 bp, Artificial Sequence
  Recombinant polynucleotide
gagggagggtggtgctttgctaatggtgaattactaactcctcaataaagaatattatttgaaataatttttgaaatttcataattactttgggttctttcttaatgataaataaataatagtatattacaaacatacattaatatttcctgaatgaatacaccacaaatctcccttaaaatatagcaagaataaaaattatactatttctgacaatttttaatttctcaaataataataccactctgatttttaaacatctacaccactctggctttgccaatctttttaaaaattgaaaagataataattttatcataattacactgaagcatagaactttttctttcaaggaaagcaaatttttgaaattctataatataacctcccataatcctgaataaattaaaggttcaacaacttagtaaagtaagactgaccttcccttttatttctttttcagatcaaaaatcttacttttataggagcagttttcaactcctaaatgttgaatataatagtcagttaaattcaccagctacacaggaatacaggactttgagtggaagaattgaatctctggtaagttaatatttgtctttgctctttattccattataaaatgaatatgataataaacctaatgttttgtaatatattttcagttgctaagtgctctacatattttccttccttgaatggtgaaacatgtgtttctctctgcttttatccagttagtttactcatatactggttcttattcacatctttgtcatgagtaaaaagtgttagaaaggccacgagtaaatatgcattttatttgtttatgaattcaaatactaaaagttttttatttgtttaattaagcattgacattgtctttttaaattcttttcattttaccttcttccctcttccttatccaactaaagacgcaaagcaggaggtgttaaaaaacaggtttaccatatcagcagtaacatagtttggacaacattacactttggttcaatgatagacatagaagtttgaacagaaatatgcaaagcaagtttgagctctaacttgaagagagcctctgggtgcctgccaggaaacctcacgagtggacccttaacattcatgtgtcaccacaaactaggggctgccctttagttttgaccagtctcagtgtcactcacttacccttaccttttcaaaaaaaagtcctaagaatataaagtaattcaatggttctacaattttagcatgtaactgagtcacctggcagggttgctttggtgagctcaagataaaattttatcagcatttctacattttctggaatattccttaatccaggcttttaatcccttggtgcttttctgaaccactgcaatgagcttctaactgttctcactgtgtgcaggctcttttccttctaatctaatttacacacttctgaacacaaatctctcacagcctgtttccttcatgttacctccagctcaagactttttgcctacaaaataaaattcaaacttgttagctaagcaccttctcatgtctatgctttggctcatatttcagccatcgtgtgccccacttattcttatagccaacctgaaaagccatcttttataagaaactacctctgctctccatgattggatataattaatcctccttccacatcacctcgccacaaaattgtatctgtgttgatctcatgccacatacctgtatgtattttatattataaatatttgcagacttgtttaatttgccatgttagactaagttccatgaagacagctccatatccattccatttttatatatccacaacatttggtcgggttgatgcttaataaatgtttattgaaggaacaggagtctcccacttctgacataatgaacttatttcccccagtgttaaccctacatctggttcctgtccaagagtctcttcccaaatcattctgattcaactgttcattctgatctcattaaacatttaaatgatatatctaacttcgcttgctttattctatgctcatcctgcagtctcctcataacttggtttcaatgatgcttgcttctagagaaaaaaatgtattaaataagcttatgattcagtcctccagctgtgatggttctcactgaacattagctcagtggttttcgaagtatggtctctagcataacctagaaacttgttagaaatgcaaattcttgggctcaccaagacatactaaatcaaaaattctgacattggggcctagaaatctgtgttttaacaagcctgccagtgcagcctggtcccttttcttctcggagccccactcaaagctttcagtgctcatctcccaccaatgacagggtcctctatggaaaccggcaggacggtttccaactctaactacgttttagagtttgcttcctagggctatccaggcaccaagtatcacaggttagtttcccagggaagcagactctgagacttgcatgcagggagtgtctctggggtgctctcaaccaacaccttcaggaagagaaggaagcagcattgggcagaggcatagtcaaactacagtgctgttggcacagaagactgaagggagtcagagccagggggtagaggtgggcccttagcatccatccttcaccattaggtgtgagttgccccacctccttgatggtgtaacctcagtcccaaggtgggtgggagtgcagcagagcagcccctacaagggccaaaccagagatacaccaggcgccagaagtgctgccagggaatagagaggaaaggatgggcttaaggtaggatccacagaacttggcaatggattagaagacaggatgagaagtgacaggttaacactaacacagaaatgtctaacttcggtagataatggtgccattggctagaagaggaaaccgaaatgaaagcaggttgttcagggagacaaaagttcactgtggacatctcagcagagtgattcagtggggaaaggaatggatgcccagaccacctcagaggaagatctaagctggagccagcaataaagatacaagatgaacaatccctaacgaactgctcctcagccatgctccccagacacgctgcttcagatttatagtccgggtgaggctaggaggtgcgcctccctcagtggaggacagcaaagcaccagtggctccagggagttaaaatcttttgataatttttgttctagcatctgtctgcagagctgtctctcagccattgcctgcctttacacaggagtgcagtccgaaattgggagatgagtgaaatttattatgcctagagatctggatccccagttgtttgggagtatattttctgaaccacttgttggtttaagtaatgcagatttattgatgccacttctcttgaatctgtgactctggacccaccatctaagtgaatgtgcagagggaacggaatggctgcaatagatctccattaaaaccagtgcatcctcccagacacatacagtagtagggaggtgagtcaatgtcaggacagcaccagctcccgcttcggtacatttccaaagttctcagtctgtgtacaaaggtttgctctggggcagcagaaatagccctgggcaggtagtcaaaggcctggtttgatttcctccacttccaggcaagtcactcgaaggctcacaggctttttcctcacctgccacatgggtccagtgagatctactgagctgtaaataatgaaatgagtgtgtgtgcagtcatctataagttgtaaagtactagaaaatggtgaaactttgggatttgggctatttaaggctgaatgctaaaaatgtcaggcattgtggagaaaggaatttaaatataagattgattgactgggatttaaagacaaatgaaggcacacacgcaagtgcacacccacactgacactgcacagctcccgttggaggcatatcctgaccatgcagacctggggctctgcctgtccaagtgcactcctttactacataaaccctccttctcttttggggctgtcaccccaccagagctggcaccgagcccttgctgctgcgcttccctggggtgtcagcttttgacagggtgtttcctccctctgcaggagccttaacatcccttggacttccttccccccacccacccccagcagttttatctcttcctaactcgggaccctttttttcccacacaaagtttattgtcagttgctggtttcatctgtttgagcggctgcaacaaaataccatagactgggtggcatatgcacgacaaaaatttatttctcacaggagaagtcaaagattaatgcaccagcagatctggtgtctgaggggccaccttctggtttgtagatgatgctttctagttaaaacacctatttaacacactattaaacactaagtgtgttaaatagtgcagttgatgtatttgtcatgtcacctttatcatacactaaatccttctttgtctttttttctgtactctaatctctttctgtaagtaatctttgcttgcagcagtaggatatttagagtactgtggcttgacaatatatttagtatttcaagatttccatgaaattcttctgatgtatgagttccctagttaatcttacatatgtatccctttgtaaaaacactttgaacatttaaaatgatacatgaatagtactctaatacaatgccataaaaattataaatcatttgtatagactggtaagtaaagattgtgagattaagaaacgcatcaaaggccattgagctggaaagtggtataatgagaattcaaaccagggtctcttgactcaaaatctaaggatcataccatttctcatgataatatgagtattattgttatctctatcccatagacaaagtgttaacactgaatgagcagtgaaatagtctcagaattttttattttatttagcaattcacttgtcatttctggtcctcagtttattcacgagtaaaataaaatagttggactagataatttctatagtacattcttacacaaaaaatctatgattttgttatttttaatgtgatatactcatggcactcattcacctcattttcccagcctgcctcactggtcattacttctctgtgttctttacaggctccccctcctctacactgccattaaatattgaaacacctcaaagctttacttatgtccacctctcctctgacactatcattctgtctagatgatcccatacatacatgcccattacttcaacctgtatttatacgccaatgattcactatatttccagcctagacattcttttgtactctagttaccagcttgatatccttacatggctgtttcaaaacaactcaaatatattatctctcaaaatcaaactcatgatgtccccacaccatcctagctttccaccaacaatacctatccctattaatagcaataccatttattcagttatccaaatcaaaaacctagaattcatccttaaaattctactatcattccaaatatcctatccatcagcagccactgtattcttaatcccctgtatttccttcaaatccattcacctctctccatatccattgctgcatgactatccaagccatcgcctctaccctagggtaccaaaatagcaacaaacctaatctgttcatttgcattattttttctccaaaactgattatctatatgtagcaagacagattgttctcaaattgcaaatcccactatattatcctcttgcttcaaacacttccatggtttcccattgtttatgataaaaccaaatgcttcaagttcgaagaccggcatgattgggaatttcctgtcaccctagcctacttgctctccatggtacagttgcactggctttctttcattccttaagtacaacctgtttcctcccacctcaggactgtgcatgtgccattcattctgctgaggagcctttttccttccacttcaatcagctaagtctgattcttcctgacaatctcagctcaataagcatttcctctaagaaatgtctctaatatcattaattggctcaggtccctctactgtattgctgcacttttcacagttataattttacttaattatgaatgattatttgattaggtctatttccatccattagacataagcttcatgatggccagattactgttttctatccatcgttgtattccaatacctgacagaaggagggcgggaggtggtggcacacaagagatgctcaaaaacaattgttgaataagtaaatgaatgaggccatttagaaataacgaaagtacctgtttacaaagtacatgtatcaaaactatgaatgcattctacttacatggttttctccaaataaaacaaaagacttcaatcaggattaatacctgggataaactgagtcattaaatctctcctttgccatcaggagtgacattgaaacaaatgtctgcaaacaacaaatacttttttcccaaaatatattgaatggcatttccataaacaaactagaacatgggaggagaaagaaagcaatattaatttaaaattaatcttatcacataacttataccatcagggatttcgggtaaaattcctttcaggcacatccatttaacaagaattgattgttactgaaagcctagaagagaatttggcacatacttggtgttcaaatatttgttgactgagtgaataaatgatgcaagtgtctaagaaacacaaaataaggacatgattacagtcacggtggagttcacagtcatctccaaaatgaggatatgcatcccagggaggaccaacaattcattggagtgctgaaataaaatactcaaaggtcattttacatgtattttttctctaaattacttttcttaagacacagaaaacaaaaaaagaaacttagctttgttactttctaacaaatagttaaatcattaaacaggattgacactagcatccttgtttggtcttatgccttaggggaacatgaaatgtgtgaagacattctgagatctgagggaagggtagacagtaatacagtgggactgaccaggcttcagcacacctttacctcctctcagcagatttcagtgatgagcagtttacaactagattgaaagattatattatctagttctaaaagaaaactaagcctcccaaaagcaacaagggaactgagaggaatcctgcaaaacaaaaacaaattttaaaacttgcactttgtaataaccctaatatgtaatcacagtaatgaacagtaagataatgacagaactgacatatttccttatctattaaagccatattaacaggtaaagcaatgccagtcagtggtacacttcttagaagatatttaatacatactagacacatacacacacacaacattttccttcaaggtgtatgtatcagaaaatcactttttaaggccggatgcagtggctcaggcctgtaatcccagcactttgggaggccgacgtgggcggatcatctgaggtcaggagttcaagaccagcctgcccaacatggcgaaaccccatctctacaaaaatacaaaaattagccagggatgatggtggatgcttgtagtcccagctactcaagaggcagaggcaggagaatcacttgaacctgggaggcagaggttgcagtgagccaagatcacccattgcactccagcctgggcaacagagtgagactctgtctcaaaaaaaaaaaaatcactttttagataaaattcatgctatagagagaagactatgaaaatatgtttagcaatgtgtccatcattaggtgattgagtttccttttgttttgttttactgaaaatcatataaagtatgttatctgtaaaagttctctgacatgcacacataaaaatttgggagaaaagattaactataatgtttaatagattttgtacacatttctttaaaaatatataaaacacaacacctttcaattggtttgcaagaataaccaattgacatcatggaaaatggaaattcacttgctgaattttaacaaaaatttgcatgatgagtgagactgacaacttagtgtcatgatttaatgaattatgccaatggtaaacttcatgcacatggggccaggtaattatgtggaaactttttcaatgcttaaagccaagtattgaaattaaacttagaatcagacctttgaaccattttatgacaatgttcaaaaattataaattctatccacttatattataatattaaaaatatcattacaaaaaaaacctgtgtttattttataactcagcctttttaatttctaatttcataaatatattataatggatattgttagtaatgtagtattattacatgtatataatttataagtaaatatacatgttttggctactcatgcataaaatgtttcacccataggagcacataatcagaaatgtctggagaccattatagtaatagatagatcatattgccacatattttatctcctccttgacaactgagctttccagatcttctggtgaaacgaaagagaaagttgtaacagaagagtgattaaaatgacaaaagcattacttctattacttctattctaataatatgagcaaagctataactatcaagtaataatgcactaaagaaggtgattaatctgatatattcacaggcaactaataagacctttctattgcagccatgaaaaatatgtgacaattatagatatcctgtgtgcagtgtttcaacctttatgtgacctgttctactaacagatttagtgatgttcactttgttagaattttcttacacatgccataacttgcttcagtcttttgattatgaatattatggatattaaggattctagactattctagatttaaaaaataatattgtcacctcaatcagaagggaaatattaaatagttctcattttttcaatgtttactcagtttttgtccaatgtaatgaaagtgtcagcagtacaggttacaaaataaaatgtgtattaaagtaaactcatttgaacaggttaataattgtagagggagggaaaaggctaaaagattgaatgtaaaacttatgaaaagtagatacatcgtctctatgatttgcagtagtcaactgcatacagatgaatcattttaatacacgttaactactttccttttacagatggagaaactgagaggaagaaagtttatatggttcattaaactttgtgatgcaagctaaactaacctgtctctgtattttccatctactgcccttatcactatctcattagaatactcttcaagcatctccttactgattttcttaccaagcatttgttaagttctaatgagagttggtagtaacattttcacccactctgtgaaatatgaaatcttattcataggcctcttcttttattcttgtatttgcatatcaaccaattaatcaacttgctttctttatgttgcttattatcttagtccttactaaattgcctcttaatgttgtccacataacagaaatgttaaggtggatacttaacattttagtccagtctagccggtgccagtgcaatgccaaatcatgaattaaaatataattacaagaaccacttatcaaattttaacaattccttcagctttgtgacagttttttctacttcgattaaagtcaagtaaaattaaagttaaatatttttattaaaatatctcctttaacattccatattaataaacatattaaagctcatgcttctaagtagattactagaagttactttatcgaattacagcaatggttaattctagatcatagaatttagaatgactttttgccttcttcttttttttccttttttttaaacagagtcttgctctgttgtccaggctggagtgtactggcgcgatcttgactcactgcgacctctgccctgcaggttcaagtgattctcctgccccagcctcttaagtagttgggattacaggtgcctgccaccacacctggctaattttttttttgtatttttaggagagacagggtttcaccatgttggccagactggtctcgaactcctgacctcaagtgatccacttgcctcagcctcccaaagtgctgggattacaggtgtgagccactgtgcctggcctgactttttgctttcttcttaatacttactagtatttcttgaatttttaaaaaagaaacataaagtactttgataaaaccaacagtctcattgttcttaaaattgttcaaaggttctctggaaaaaaaaaagaaaattatcatttggttaagaatcatgttggtctgacatcaatcatcctataggagtgaatattgaaaaagtaagatatattgtggtataatcgagattgcataaattttaccatttttgagaagaatctgctccaaatcctggcttaatgtaatatccagcatgctacttaattttcttgtcttcaccttttcatatccacatccacctaggtgccacctcacagtataagccagcataatccattcttctcaatgaaaccacaatacatctgaccctgcatctcaggagaactgtatcagccacagcacttccagttgactatgaatctgaatgttatgcctcaggagaaacatccttgctgggactgagtagtgattcaaggagatagttatgattcagtcaagaaattaataattagtgttatttttattattgagacagagtctcgttctgtagcccaggctggagtacagtggcatgatctcggctcactgcaacctctacctccccggttcaagtgattctcctgcctcagcctcccaaataactgggacagcaggcacttgccaccacgcctagctaattttttgtatttttagtagagacggagtttcaccgtgttagccaggatggtctcgatctcctgacctcaaggtccacctgcctcagcctcccaaagtgctgggattacaggcgtgagccactgcgcccggccataaattattaactgagccaggcacagtggtacacacttatagtcccagatactcaggagactgaggttggagtatccttttttatgttattttatttttaattattatgggtacataataggtgtacatacccatggagtacaagtcatgttctgatacagacacataatgtttaataatcacatcagggtaattgggatatccatcacctcaagcatttatctttctttgtgttaggaacattccacctccactcttggaataggcaccctgttgtgctattaaatacgaggtcttattcatttcatctaactatatttttctacccattaaccatcacctcttttcccctcttccccactacctttcctgtgaggctgcaggattcttaagcacaacagttagaggccagcctggacaacatagtgagactcaatttctaaaaaataaaaaagaaattaccaactaatgctaaaaaaatagtctctgatgcttaggtatgaattagaaatgaccaaaaaaaaaaaaaaaaaaaagactgccctttgcttccttctccccttctcttcaagttttccattgctactcattttagtctggtttaatcaggtttcatccattaaaagcaattgttgggatcacacattttgagttgtgtcagtggacttccctcatgctggcatgattcctgccccaagcccttagtaaaagccaccaagccatataacataatctctcattgagtaaaacatctgatgtgtttagaatgacttctagcaaaaaaccagcctgtccagcatcatctctgtataacagataaaggaataggtactgcatcaaaaggttatagaacctgcccaaatcaatcccatgtgttttgcaatggaattaggttgaactaaagtgaaaattcagttttctactcctcattaacatgtctcatgttgcaaggttgagaggaaggagaagaagaactgtatttacagagagattccccctctctttctttctacagattactaaaacattcaaagaatcaaatttaagaaatcagttcatcagagctcatgttgccaaactgaggtgagtggaactgtagaaaaaatatttaagtatagatacaatgtggcatacttgactttttgtcacagaatgaatagtaaatgacatgttcagataagttgttgtaatattatgaaaatagtattttagtcagcttaaaaaccaatgccaaaaaagccaaacatatgatctatttagctactaatgtaaataaccatattatatctattcttattgggaagaggaagaaggggtggagagagagttggggtgaaggtacagtaacaaggccatcctattgtaaaactccagtggatatcattcacagtgcagcctatgtaaacagtccctcctggagttgtacaatgctgtggtttgggtgtatccatccaagatcaagacactatgaccaacatcaaaagtggctttttggttttatctgcctgatgtgctataataaaagggtattatggccaaatccaaggcatgtctatcatgaattaataataggaggagtagcagcatgcatgctagttatttgccattcctgccttagttaaatatgatgtgataaaaccagcctttccaactgaaatagtcacctttactgactctcccgcaaatgtctcaaatgaccacattgctctagtctttaaataatatgcaatagttctttggtagaagaggaattatactaattctttctcaaatactagcatcacaagaaaattaattcttgttctctggagagtcacctagtaagtatctggagcacagatgtctggtcaggtaagttttgatgaggagttaaagggataagaagagtccatgagaagggtattttccaaaacacctttcggtcaattcagtgcacattcacttagtactttcttgtcagtatctgtatcagccactaatgttcaaaagtgagtaagccctgaaaacctgtaggactacatgagccttctgccttttctctccttttgttcacttcccacttatcactcaatcctctgcaacctggcttcaataccaccataaaatatcaactgctcttgccgattcaacaatgacatccagataacaaaatccaaagaaaccacatcagtcctattcttggacctttcaacagtatttggtcctgttggcctgtcactccttgaaataggactatcccttggtttgcatggccttgtataccctgattttccccttacctccctagctattccttcttagtttcctttactaggtcttacttctttgtatattccttaaatgttgctgaacatcaggctgtgctctaggcctctcatcttctcaggtcacactctctcctttccttggccttcactgccacccatatgctgagtgctctcaaagttgtatctctaggccagtcctcttttgcctccaaacatgaatatatgcagccatctacttggtaccatcacatggataattctcatgatctcttccagtatgactgcttctttatttttttctgggctcttttttagcattgctttacatggaactttatcatgtctctcaacctctattttatcttttatctatgtatgtagagtctgtgtaatttcttcatctcttttagataactaatatctcttcagctttgacttgtattctgtgtaacccatttattgcgttttcaatttcaatgagtatgttttcctatctgcaagttctatttgtttcttttgagaatcttcctggtcttttaaacacatttcttattttaatttttgggggtacctagtagttgtatgtatttttggagtacatgagatgttttgatacaagcaaacaatgcataataatcacattgtgtaaaatggggtatccatcccctcaagcatttatcctttgtgttacaaacaatccaattatattcttttagttatttttaaatgtacaattaaattattattgaccatagtgactctgttgtgctatcagatactaggtgatcttttaaaaataatgttttctacttaatctcatttttatgattccctcttttacgtcatttgtcatttcaaatacagtcacttgtctgttgattctattatgtgaagtttttgaggataatctttttgttactttgattccaccttggtatggtttggctgtgcccccactaaaatctcatcttgaactctggttcccataatacccacatgttgtgggagggaccttgtgggaggtgattagattatagggacgtttcccccctttgctctgttctttttcctgccaccatgtaagaaagatgtgtttgcttccccttctgccatgattgtaaatttcctgaggcctccgcagccatgcaggacctcttttctttgtaaattacccagtctccggcggttctttatagctccgtgagaaaaaactaatacacacctcatgatgtattgtttaccactgaaattgtatgcttaaatttaatctcacttgggaccctgtacaacctagacttaacatatctacctccagagcagttacatctgtcagacattctagaggaatcagcagcacatggactttgttgttgttaatttgttgtcgggggaggggggagggatagcattaggagatacacctaatgctaaatgacgagttaatgggtgcagcacaccaacatggcacatgtatacatatgtaacaaacctgcacgttgtgcacatataccctaaaacttaaagtataataataataaaattaaaaaaaaaaaggttctgggagtattcaggtagtattaatgaagattcagacatcgtgcagccaggcccatgcttatgaattttcaggtgatacttctttttcttttttcttaatttaaagctggatctcggaaacagataaatttatttttttatgacatgacgagcatttttttcattctagttcatgctgttattgggtgtttagttctttgagactcctggcctttttctaaaacctcaagttcaacttcctattttgcactggcccaaggtcccatctccagtctctatgtaaatgctaaacataagcctgtggaatattctagtctcaccacatactattcacattcttctttgtttttggtcttccaggattttccttacttttctatgaacccagtcttgcatttgaaatggaatttattatatattatctatcctttctatttgttttatgcagaaagtgttttctaaaattatttaggcttccatattgctagacatggaagttgtaattatttgttcagtgcctgtttctacatctaaactgcaagacccatatggcaactgtgaatcttagtcccagctaatttctgaagcttagaatagtgcctagcacaagaagttgtttatctaacatttttaaaaataaatattaaattcatatctggaatgaatattaagttagagctggtcattgaggtgagaggaggaagccaagagagaatatgagagcctcaaagccaaatatctttaatgtactttttcagaaaagaagacagccaatgtcaggtggaggaactggtttatgaggtaactttcctggaagaaaatagaaattactgaggttttagataatccaaatatttaatcaagtcaccaaggtttattgtggggaatctttattattaattaaaatgagtgatgaaatcttaatatacgacaaaagttaaaatttgcttttgcaggcagatgaatggtctaggtatcaaaaaattaagttgagtctctaactcacacaaatttacaaccctatcactttatgaatttgtttaggagattatttttaataacactggtgaagtctaagaatagctaaaatttatagtacacttattgtgtgctattgactcttctttgaagttttgcatatagtgattcatctaatcttcataacccattttacatgtgaagaaacttagatatagaaagattaagaaacttacataacttatccaaagttacacagtaaaactctggcattataacttcaaaatcagctatcctacagtgagtacagtgttctgtgcattgaaatcaaataagtgagatagcatcgtgatatagtattacgtatgcaaacactgttacagagatctgtctaaagttaaattccacaaatgaattctttaaaagggtttaatcaagaagaatatataaacaggatggtgaaaaattgtcatattatttgttttttaaaatatctttatgatttacaggcaagatggtagtggtgtgagagcggatgttgtcatgaaatttcaattcactagaaataacaatggagcatcaatgaaaagcagaattgagtctgttttacgacaaatgctgaataactctggaaacctggaaataaacccttcaactgagataacatgtaagtataatttttcataaacaattttatttcaatatatccctcaagtttaccaattcaaattcatattttaattgagaggctgacttttctttctttgaaactaaactgtgaaaacaatccattaaaaagctaaatataccatatagctccctaacgtaaatcattctaagacttaaagaatcatttggcatttatatagtaaattttatttgctaaaaattctcattaattatccctgcaacattccttatgagtgatgttactgtcagatgtcattagtggataggccataggaggggtacatagatgctcaaggtcagagaactatttaattaatgatccacctcagaggcttcttcatttttctttgtaacatttatcacaattgaaattacaaagttatctgtgtaaattttgtattgtttggcttcatcctacactgtaatcatcctaaaagaaagaaccagtcaaccttcttcatcctactaccctcctaccacccagtctccatcatataacacatattcaataaataattcttgcatgactgaaagaaaagaaataatatatgcatagaatttaaggacattcctccaagttggttacattctgctagtttaataagccattatttcttctcgatgagctcaagattaaaaggattttgatgattcccatactagactggtaggtaccagttacagatgtactaactgttaaatattgaaatgctttcctatttgttggtaaacaattactgcatcaggcccacaaagttgtcttccgagatgtttcaaatccactgcccctgctgctaaagagttatgcttagcaaagcaaagcactctaagacactgctccaactccatggcctgattgcatcttttatgactggccaatgctcacgcactgcagtttgttaggtagttgaatattacctctgcttccacacattaaggaatgctcccgaacgcacttcccaagtgtttatttatttatcattatactagacaatatggtgatacgatggtcacagaatagcggtttccacctccagagcccataatctagttgaagggaaagatattccaacacaagagtgttgacaatcaagatagaatatgatcaagggcccagtgtgaggcccaggcaatgatcactgcaggaatctggggaagaaagagaccagcgtgcttgggatatctagcaaaagtttcatgaaggagaatggactttgactttgaaatatgggtaggatttacatattttgagatgagaaaaagaaagttcccagagaaggaaagcatgaaaaggcaaacagtctgtactgaacgcgatgctttgacagaataatgaagaaagggacctgctggaatgattgatcagtgttcatcattcacaccatcatcatcaaaacacttatttaatgagaacttactgttttttaggcatggctttaatgccctatatgaatttttttcttgattaatccttacaacaaacatatcccatagatagttttattgtcccccttagaaaagataaattgcctaggctgacacagtcagtatatgaggcagtcaggattcaaactaagtctgtttgttcaaaaaattaagaatggccagctttttaaaattttctgtctccagaagtatgatttggctccactgaagtttgcaaaacaaatgtgatacccaaaccttgtgaaacttttagtgggaaataactttgcataagtcggtttgagagagcgtggaaacctgtcttgaaaagttttaatttaacttgcaggaaataaaaatgatgggtttctcaattaaaaatttcaatcaaggaaggatatgagctaacataacatttttttaaaaagatcagtctggtaaggtagaggtgcataaactgaaaaggagcaaaagtggtggaattcagttagaaaattattgtaactgtactgatgtcaaatgatgaaaccatgaactaaagtagtaccaaaaggagtgaggaggatggaataattcaaaagatagaggacagatgtgcagaacctggagattataagatgtgaaaggaggagtttgagaaaatttcagattttggaagtggtgtcattttactaaaaggatataataagtagcaaattttggataaagttgggtcccactgagtttgagatggctgttggacatgcagagaaaactgtcttgtatgctgttcttaaattgaaatagacagacctttaccctctgatactgacatattttcctttccaggctcaccctccatttccctaaacacaacacatgcactagctctccttactttattgctccacaaacatcttacacctccaagcatttgtgcccactgtaccttctatctggaatctcttttgtcctcttgtgtgcctgaaaaattcctttcagatcttcaaaatacagtgcagatgctatttcttctagctcaaatattatctcctccatataatttaattactctcttttttcttttctctactttgcacttacatttatttgaatgattgcttgattaatttctacctgtaaattatgtgagggcaggtcctctatattttgctcgcagttaaatctgcagcacttattatagagtggtatcattagagtaatatacatatatttgaggacatgataaattaacttcccctatagtatttatcacattgcatctcaatgacttgcttatgtttctgttttcccatataaattgagtaacttgaaaaaagagatatctattaagtatttaatgagaaattaaagtacaaactttagtatgcataacaacaaattgggaaaaggttgtaaacaaagagatttgtagggcccatgagttagagatcgtttcagcaggtctgaaaggaagcctaggaatctgcattttagaggaccacctcccaaccccaacaagtaattctgcttcttgttgtctgggtactgtactttaagaaattatggtgaaatgatatcagcctttattgtatttatcttattctcattttttaatactagcacttactgaccaggctgcagcaaattggcttattaatggtaagttttaatattattttgtaactgtaatttgccaaatcataaagagtaaaagtgcaagtcttttgtgtacttttggccaaggcagtatctatcaagttgatgtctttgttcttagttcgctcaggtggtgttgaaacaagacagtgctgatcccaagtgtcccatggagtggactttaggtttcccctttccttttagaaaaaggaagaagttgtagtggaggactacccactctgcactcaaaattgccctcatgaaaatttctttggcagctttgagaaccttttactgccctggttctaaggtggcatttctgtagacttacaaattatgtttgatgacaccgtttatgtagcttctcctaaccaccagagtagcttgctttgttgtgaattcaggttaatcacaaagtataataaaaaagaattgtcagaagtcttcccagctttgggtctataacctgaaggaaaagtcactactcttcaacatcatcctatgtactctcaggctaggatagcagaaatgcaatccctagaaaacagcaacttacttctctgaccaaaaaaatgcagttaaaaattagttcaatgtacctggtagctggcctatcttaggtacttcagtgattttacaaagtgatggtagtcctatgggtgtttttcagcttcactacgtatttaattcatgcttattgttaatgaaactgtgataagcaatttactagggtatttgtttgggagatgccacaaaggaacacatgtatctcttaatggaagcctggtcctcctttatccaggaaatttgctaggaaaaaaaagcctttaggtggttgtgctattaaaccagggcactacttaaaagccagcccagcaatagttgtgtgatttaccattaatttcttagtaatagaccacacaaaagaagaaaattatgggaatgcgagttgagaggaattgggtgatcagcctaccccagcccgtttcagctctggccagtagactattcacgagctctttgaaaacatttaaataaaccttatttagatactagaaaccctctgtcaccctcaagaatattctgtggtatagcgactcctttatgagggcatgtttggtaatacagcatcagtcttggaggtggactggattctacaaggtgaactgcagtcactaaggagtcttttggatgagaccagttttcctccaacttcaatgtgtgcatgaacctcacatcaaaatgtagctttagatttgtcccatgatgtggttccaagaatcagcacttctaataagtttccaggggatgcccatgctgcaggcccacaaaccacactgagcatagcaagactattgagaaaaaggaaatttcccaggagtctgtggcctgagctggcacatccaataatgacctatcttaacctcaactcatgaggaattccagggaactctgaagctgctcaaaatttgaagcctatatgccaactaaattcagaaatgttctccaaaatgctatctataagcaacagtagtcacaaatgcattgtagaaatatatcgatcatgctttttggaaaatccagcatgtcctgaggaagaatgtataagacataaaagtcataaattatggaaagactcttcagcttcttccaaatgtaaaggaatcatgatcttcccagcacattaatgccctttctcattagaatgtggggccggtccagacctaataacattgtctgagcagagaatccttggaggcactgaggctgaggagggaagctggccgtggcaagtcagtctgcggctcaataatgcccaccactgtggaggcagcctgatcaataacatgtggatcctgacagcagctcactgcttcagaaggtgaggccaccactacctacccatctgggaacaattagaatagacaggtcatgaagactgcaccctctaccctaggattgaattgagccagaaataattcaatgcaaaaaaatcagtaagaattttcttcctattcatgaaaggaaaaggatttttcccctttagcatgctaatttagtgctatttctctgtttcaggtaataatatattagcacagtaaagaacaaagatttatatgtcagaatgttttttaaatcctagctataaaagcttaagaaatttactaaatctccataagctttattttttttccaaattaagggacaacactgttatctgtgacttagtgttactggtagcattgagtacactaatgtaaacatacgttaaatgttagcgaaacgaattgctgtggaagatttgcacattatatcatgggagctgatggctaacctagagactgccccatgccattaatttattcattcataaagattattgagtatctagtatgagcacagtgttatatattgtagaagctactagtataaacaaagtattgcctctgccttcaaagagcttacactcgaatgttggaatcagaatgcacaaaaataatgatcaattacaatgagtagcataaataaaattaatgtaggcaacttacaagaattcttaattgaggtgactaaactattgccaacactagggtgatatgctaccagtggcgagtaggttgcataaacttaccttattggtaaaaagaaaagttcacattgctcataaaagaaggattttagatttcagcataactaaaatctgtttcaaacctgccttgttactggggcatcgcagaccacaacagttgttgggaacttaactcaaaaagttcacccagaaaaataatggagatttgaactcgtgtgcccctgaccatatcaattttcttctcagactcttactctaaactggacctccttatcacacacacaaagccttccataggcagatcaatccagtcttatttctcaaagcatgtaccttgagcttcagataaacagcattgttctcttcccctggactcttcctacatttccctacctatgagtatctgatcaatctgcttatccttgaaatgttaatatatttaccacatctctatttgaattttatgaaatttttgataatttctaagtagttttttcagatttataggcactacttcatggtacagtgactgttacaaacgtatttgttaaatttagaaggaataaagatttaaaagactagggtagttactgaactaaagttttaggaaatcccaaattatttcaaatttttcttatggtaattttatgacttaatatttttatatgcagtgaacaaatttgaaactttaaaagatactcccagaattatcagttttctgatgtagattggcaaatttattactatatcccaaataacccaagagacaaaattcacaaaaacatttcaattttcattgccacttgaaaggccaaaaagcagaaatggcacgcattgatttcaatcgtactcttgagtgtgggaaccaggaattaaaatacctggacttatcaggcacttagcataaccaagaacggaatagaaacctccctggattctaagccctattcagtcccaatcaccaaaaaccaagtaaacgatatcactataatgaaagccacagttataaatatcgacaacgattaccaaaggaatccatggaactttgaattttgccaccccacatccttctattcattaccatgattgatccactaaagctaacagactctgtgaaccttgtattggacccctccctaaagacctgattgtcactgagaaccatcagtgaggatttgtttggggcatgaccagccttacatcaaagtacatagaagtgatgaggtcttatcaaagaggattattgaattatcacctcttctatgtagctttccctgatactctctttcctctccattgagttccacagaaatttttttatctgcctttaacagttgtcctcatgatttgtgatatttgacttacctcttgtcagtttccttcactagtgtagagttcctcaaagaaagagaccataattacttatatttttattcctggagactcatactattccttatacaaagtagacacttaacaatggcttgttgaactataattaatgaaaataatagctaccttcatgaaagttcactttgtgccaaacactatagttgacataatacatttgtctcattaatacttaacaattgtgtgagaaggtatcaccaatcacattttatatgtaaataaaccccagagctattaattaacttgtcataaataacacttttcatatgtggcatagccaagatttaaatataaatgttactggttccaaaatgatgctctaattcacttgctggaaagaaggaaaggaagaaaataaacgagtggaaggaagagagggagggaagagagaaaaggaaggaaagaaaaaagagtctcttcagaaccttcactgtaaagactccgagcaaaagaagttgaatataaaaacaacataggtttgtttgttttctaatattttttcttcaaaatttttaactcaggttcactcttacacaaactactgtgtcttataaaagtatttccggtcatagaatttttattttctgtattaactccactatctaatctccataaaactcctaaattggtattatcggtaacattttgtttttactcaacccttaggaacaatgttaagttaatcagccctccacatcacagatccttattttcatcagtctgtacaaggcatttctctcattttaattttttttcctcctgtcatccctggatttcactttcactgccctccttccacccatatgcctcatactaatatattcgaaatatacatgtcttaaaggtacatgcacgcacctacaaaacctatagtgtttttttgtatgtatatgtctttaatttaaataagtagcattgtgtaaaagtctaatattgtttcttactgttttcactcaattcttggaattttcatctgatgcactgctgcatagcaccccatggtatgcagccaccatatttccttcatccaattaggttgcatgacctaccttcccattgccacaaagagtacacacaaaatatttgtacttatctttctgtaaaccttcaggaatttcagaagcacacatgcaggctgctaaatataccagaatactttccagccacttaaatctttaccagtattgcaaaagaggccccatttccctccacatcaacatttagtattattcttttgtttaagttttatcaatcttttaaatgtacacaagatgctcatttttataattttaatttctcagattactagtttgagtatcttttcatatatctaagagctgttttgatctcccctaccatgaactgccactaatattctttgcctattttacaatggtttttctgcttatttattactggtttacagacttttaaaatatattctacaaaaattttagacattaaacattaccaatattttcccatggttcctcatccatctggtaaacttgtctatggtatatctaattttgatttaatagaattcattctatttttaccttttagtttgtgtttttgttgtttagccaaaaagtccccattcctaggtcataaaggtaatgtcctttttttttttttaacgctactgttctctctctgtctccccctatgtatataggtgcacatatacttgtacacacatacatatacctatatatgaggggagttcgataagtttatggaaaataaaattaaaagataaaataaaaaattataaactttatttctcaacataagctccttcaagttcaagacacttttgtaagcaataataccagccatatcgtccatccctaaagaactgagggtcctgagaatttaactatgtcaatgcagtcttttttacattacttttttacagtacttattgatgaaaaatgggtgccttttaaagattgttttaagattagggaacaaaaataagtcagaggaagtcaaatcaggactgaaaggtggatgcctagtgatttattgctgaaactttcataaaactaaccttatttgatgagaggaatgagcatgagcatggttgtgatggagaagaactctggtggagctttcctggacactttttctactaaagctttggctaactttcttactctcataagaagaagatgttatttttcactgaccctttagaaggtcaacaagcaaaatgccttcagcatcccaaatgtctgttgtcatgacttttgttcttgactagtctggttttgctttgactggaccacttctacctctttatagccattgctttgatggtgctttgtcttcaagattgtattagtaaagccatatttcatcttctgttacaattcttcaaagaaatacttcagaatcttgatctgacatgtttaaaatttctattggaagctctgaccttgggtgcagctgatctgggcgaaacagttttggcatccatcaagtagaaagtttgctcaactttagtttttcagtcagaattgtataagctgaaccagttgagatgtctatggtgttgtctattgtttctcacagttaattgttggtcctctttgagacatgaacaagatgaaatttttcctagcaaactgatgtggatgatctgttgctgcgggcttcaccctcaacaacatctctttctttcttgaaacaaattatccattagtaaactgatgattgggggagatgctgtccccataaactttttgtaaggcataaataatttcaccattcttccagtttcaccataaatttgacgtttttttgcttcaattttagcagcattcatgttgctttgataagagctcttttcaaattcatgtcttattcctcttagtgcctcaaactagatcttgttcagtatgacaagttagtatgagtttatctgcatgcaaaaatctttgaaatccatgcatagtttgtttataatatacattttcaatgaacttttgaagaccccatacatacatatgtatatatatgcacacacacacacacacacacaccaaaatcttcaaccattatcagacttagtgcagaaaaattattcatccattaacaagataagaatgccccttatcatcactactatttaaatggagctcctggctaaaggaaaagacagggattgaaaaaaattagttaaatctaaaatgtttattatttcaggtttcttagttgcttaaatgggaagggaggtatggacaaaagagaaatcaaagatatttgtgttatgctacttatcattaaagtatcagaataacttcattggaatagaaaaacaccaagatcaccccacgatatgttttctaaaatcttctccatttctttagacaagtgaccatgtattcggccagtgaagaattaaactcacttgccagcttataatgcaggaaaatatagcaaagagatgtggatccaatagtttctagatagtggtacaggatggctaagatgaatttatatatctgaaatgttcacaaattccctactcatatagcatgttttcataatgttttagcaactctaatcctcgtgactggattgccacgtctggtatttccacaacatttcctaaactaagaatgagagtaagaaatattttaattcataacaattataaatctgcaactcatgaaaatgacattgcacttgtgagacttgagaacagtgtcacctttaccaaagatatccatagtgtgtgtctcccagctgctacccagaatattccacctggctctactgcttatgtaacaggatggggcgctcaagaatatgctggtaagtgtctcggaaaaaaaaattaacaatagaaatgtcttatatttgctattaggtaattttttaaattaggaaacatctggaataggtgtttctattcttctacagacagaaccattctatattctgctcagcccaagctctggctacccctgagtctccttagcaaagcaaagcaatgctccagaaactatgggaattctcaaatatagtaataggaaaatgtaaaagaaagttatgaagacacgagttctttaataatccagagattctataagattcaaatagcttccctataaacaataaaaaagattttgtttgtttgtttgtttgcttgttttttagagacaaagactttctcagactggagtgcagtggtgcaatcatggcttactgcagcctcaaactctggtcttaagaaatcctcttgcttcagcctcccaagtagctagaattataaataagtgtgtaccaccatacccagctttttttttttttttctacagacaggttcttgctctgttgcccaggctggtctggaattcctgccctcaagccatcctcctgccttgttggcctcccaaagcaatgggaggatttagattagacattgtatgagggcttaataatccttaaggtattaactgccctttaaagtattctgggatatggcaaaaactcgatgtgtatataaacattggtcatatttgtttattgaatgaataaaatggaaactaaaatgaggacaatgcacaagagctactagaaccagtaagagtatcagcgaaggagtggaagggtagcattgacaatttccctgggcttttacccatgttgtagattgtctctccaaggaataatacaaagccttaatagtcctagaacacattctattgtgttcttatggcccaaagtaaattggtgtagtagataacatttgcaccagtcatgaaaaactattggtgtcattctgagagtacatcaatataaaatagactagttctttagccttgaaactagactggtttctcttttgctgctaggttaaaggttattcaatatgtaatcttccaatccaaaatctgtcagtggataatttaaaagcttttagtcaattttaagatatttgttttcttaaaattttaaggggcactgtgtcacaaagctaaagaaaaaaaagaaaaaaaaactgatctgtgaaaggggttatcctcatctacttggggaattttggctgcgaagaaactccaaagtaaatctttagaagccttcattgttaaatatgaaataatgtttggagtacatttatttcttctcaaatttattatagggtcaataatgtacacatcttgaagtccatttttttcctgcttttataacaaacaggccacacagttccagagctaaggcaaggacaggtcagaataataagtaatgatgtatgtaatgcaccacatagttataatggagccatcttgtctggaatgctgtgtgctggagtacctcaaggtggagtggacgcatgtcaggtaagctcaagacaatctcatccatgtcatcatccaagaagtgtataagcacttcctagtatgtgataatgtgatagacataagtgtaacagttacaatacacagccctgttcctctaaaatttataatctagattttagaaataaatttttttatgaatgaagtttatctatcatgaaagcattaactctgagaggccaaattacagagtagttaaccatccaaagctcaagaatcagaaagacctcgatttgaattccttaacctctattaccaagtctctaactaaaagctggggataatcataatagcacctaactttttgggtactaagaaaagttaaatgaagactaaatatatcaggcacatggtaaacaacaaagaaatctcatctatttcactattattaatgtagaccatggtcactcgtgttaataactttaacctcaaccttttaactgctgtgaaggattaaataaaaaattaatcactatattataaaaattaattgatatataataaatgaattttaagagatacgtaataattcatggactccttgaagatagaaaatttatacaaaatcctagtaatttgagtcacaaaagctcctacaataatgaaacagtatgaatgaaaaagaaaagaaataactattatatttggatctagcccataatttttaaccaaatgcacaaaaacaaacaacaaatatgaaattctcactgtaaagtgattaaaatcaaatttgaattctaaaattttaaattaaattatctaaacataattgatgcagttatatgttttaataggttttgttcacatatctgaaatccaactccacacagtagcaggaacagctggtgtcagaaattaaatattcttttagtctggagttttaaaaaatcaatctgtttacttgagtaatttgttgctgttttcatgggtgaattgtatacagaaggataagaattattcttcgcatcaaaaggtcactgactttcatatttagtgctcatggtctttaaaaagtggataaaaagtagttctcacatttcatggaaagcccccaatccatgagcacatttcccaaaatgaaacatttttatcaactgcaagttgtgtgtaggtggagatttgtttttcaattgtcaagatactgttaattacccagtcctttatctccttttggtggagatgtctctgtgctaggaaacccttcttgctctccttcctgtttctcttttactactggccctgaaacaacaaattctcaagtttcatgacagctttccaaagaatccatcaatcaaataagcaacacaactcgacactgacaattccagacctactaagagcattaattaagacttaaaaataaacatgagttttaaaagggtgttattcattattttcccatttataacgtcccttaccttctgtccttcagtgcatacaaattattatcttccttgaagcccagttcaagccgtacctcaccatgataccttccatgtatattccactctaggcctcactgatttttaactgaaatactataatgcatagttcacacttaaaaaaaaaaaaaaaacacagcactttacataagagcttacaggatcctatttgttttatccattcttttgttcatttttacaatcattaattcaaaggaattatattaattactttctatgcacccgacgttgtgttaacacaacaatactatccctgcattcagcaagtctatggtctacaagagaggacacaaattcaaatgtctgtagtcaagcagtgaagctggctagatatggaaaaattacaagtccctcttgctttaacatttgcttgcccacatttggtcagacatcatgcaaaataatttctcactatagaaaaaaaaacactacaaaaacaataatataaagaactgagaactggttaactgaagcatgcatatgtcatctaaaagaagcaggtgacgaccagcttcatgaagtacttgccatgcatattggcacttcacacactgacccttctccccacctagaccagtaattaaacaggtatggatgagctagctactaagagcagccaactgaatagctgactaacttagaagcacacttggtaataatagctgacttttattagtactgactatactatatgctaagctgtactcaaagtgctttgagttttaaactgatacaaacattatatgaggaaacagaggtacagagagctattcaccagcttaccaaaggtcacatagctggtaagtggaggacttaaacccagactatctagtttcagaacccacagacttaatccatcgtgcagaacataagacatactccatctgtctccccaactaggttattatgtgcacaaatatttattggttggttggttcattattatgactgggtggtaagtatgtcattaggagtgttttgcttatgactatataaatttcttcaccaaaagaagactttctgatgatatactatgcatcagacaccacgcagggtgctaaggttaggaagataagtgagacttctagaaactcattcattcaacaaatatctcctaagggctagaagcttaggtttcagcagtgaacagaataggtatgttctctttcgtgttggaccttatagtatatctgggaaaacagacattgaataaatatcacaaatgcaagtgagtgtttcagagacatgcagctgctacatcaaaacaaaacagaacaaaacaaacaaacaaaaactgaccagtgggattaagtgtaaataggcacacaaatgcacaaatatgcttttataaaatagtgaagcagtgacagagacacacacaagatataaagacacaatgaagaacaattgagcccaaagctggaaagggtgagagtgtgaaggaaaaaggttgatcagagaagttttcccgaaggagagaaagcctggatgattaggaggcaaccactcggtgactgagggaaatctgaaaaatgtatttgtcatcttctcagacttgctgaaggaatgacttgggtactttgaggatttcagtaatttttccatgacttggtataatatttcaaaaggaaataggctgactttatttgtataatgaatgtgactccttcctcgactgccatagaaataaactccttaatattttgggtttgtctttgcacttaagtaatcagtcattctgtttttttacagggtgactctggtggcccactagtacaagaagactcacggcggctttggtttattgtggggatagtaagctggggagatcagtgtggcctgccggataagccaggagtgtatactcgagtgacagcctaccttgactggattaggcaacaaactgggatctagtgcaacaagtgcatccctgttgcaaagtctgtatgcaggtgtgcctgtcttaaattccaaagctttacatttcaactgaaaaagaaactagaaatgtcctaatttaacatcttgttacataaatatggtttaacaaacactgtttaacctttctttattattaaaggttttctattttctccagagaactatatgaatgttgcatagtactgtggctgtgtaacagaagaaacacactaaactaattacaaagttaacaatttcattacagttgtgctaaatgcccgtagtgagaagaacaggaaccttgagcatgtatagtagaggaacctgcacaggtctgatgggtcagaggggtcttctctgggtttcactgaggatgagaagtaagcaaactgtggaaacatgcaaaggaaaaagtgatagaataatattcaagacaaaaagaacagtatgaggcaagagaaataatatgtatttaaaatttttggttactcaatatcttatacttagtatgagtcctaaaattaaaaatgtgaaactgttgtactatacgtataacctaaccttaattattctgtaagaacatgcttccataggaaatagtggataattttcagctatttaaggcaaaagctaaaatagttcactcctcaactgagacccaaagaattatagatatttttcatgatgacccatgaaaaatatcactcatctacataaaggagagactatatctattttatagagaagctaagaaatatacctacacaaacttgtcaggtgctttacaactacatagtactttttaacaacaaaataataattttaagaatgaaaaatttaatcatcgggaagaacgtcccactacagacttcctatcactggcagttatatttttgagcgtaaaagggtcgtcaaacgctaaatctaagtaacgaattgaaagtttaaagagggggaagagttggtttgcaaaggaaaagtttaaatagcttaatatcaatagaatgatcctgaagacagaaaaaactttgtcactcttcctctctcattttctttctctctctctccccttctcatacacatgcctcccccaccaaagaatataatgtaaattaaatccactaaaatgtaatggcatgaaaatctctgtagtctgaatcactaatattcctgagtttttatgagctcctagtacagctaaagtttgcctatgcatgatcatctatgcgtcagagcttcctccttctacaagctaactccctgcatctgggcatcaggactgctccatacatttgctgaaaacttcttgtatttcctgatgtaaaattgtgcaaacacctacaataaagccatctacttttagggaaagggagttgaaaatgcaaccaactcttggcgaactgtacaaacaaatctttgctatactttatttcaaataaattctttttaaaataatttccctgcctaattatttatggaagttatgacttttgaaggacaattcaaaaccatttatttaattggttctgcaatgaaagaactgccccatatactctactaaaggcttggcactttctgctgccttttaatccagcgctataattgaggcaagcgtccagcttgacacctcgagataacttcgtataatgtatgctatacgaagttatatgcatggcctccgcgccgggttttggcgcctcccgcgggcgcccccctcctcacggcgagcgctgccacgtcagacgaagggcgcagcgagcgtcctgatccttccgcccggacgctcaggacagcggcccgctgctcataagactcggccttagaaccccagtatcagcagaaggacattttaggacgggacttgggtgactctagggcactggttttctttccagagagcggaacaggcgaggaaaagtagtcccttctcggcgattctgcggagggatctccgtggggcggtgaacgccgatgattatataaggacgcgccgggtgtggcacagctagttccgtcgcagccgggatttgggtcgcggttcttgtttgtggatcgctgtgatcgtcacttggtgagtagcgggctgctgggctggccggggctttcgtggccgccgggccgctcggtgggacggaagcgtgtggagagaccgccaagggctgtagtctgggtccgcgagcaaggttgccctgaactgggggttggggggagcgcagcaaaatggcggctgttcccgagtcttgaatggaagacgcttgtgaggcgggctgtgaggtcgttgaaacaaggtggggggcatggtgggcggcaagaacccaaggtcttgaggccttcgctaatgcgggaaagctcttattcgggtgagatgggctggggcaccatctggggaccctgacgtgaagtttgtcactgactggagaactcggtttgtcgtctgttgcgggggcggcagttatggcggtgccgttgggcagtgcacccgtacctttgggagcgcgcgccctcgtcgtgtcgtgacgtcacccgttctgttggcttataatgcagggtggggccacctgccggtaggtgtgcggtaggcttttctccgtcgcaggacgcagggttcgggcctagggtaggctctcctgaatcgacaggcgccggacctctggtgaggggagggataagtgaggcgtcagtttctttggtcggttttatgtacctatcttcttaagtagctgaagctccggttttgaactatgcgctcggggttggcgagtgtgttttgtgaagttttttaggcaccttttgaaatgtaatcatttgggtcaatatgtaattttcagtgttagactagtaaattgtccgctaaattctggccgtttttggcttttttgttagacgtgttgacaattaatcatcggcatagtatatcggcatagtataatacgacaaggtgaggaactaaaccatgggatcggccattgaacaagatggattgcacgcaggttctccggccgcttgggtggagaggctattcggctatgactgggcacaacagacaatcggctgctctgatgccgccgtgttccggctgtcagcgcaggggcgcccggttctttttgtcaagaccgacctgtccggtgccctgaatgaactgcaggacgaggcagcgcggctatcgtggctggccacgacgggcgttccttgcgcagctgtgctcgacgttgtcactgaagcgggaagggactggctgctattgggcgaagtgccggggcaggatctcctgtcatctcaccttgctcctgccgagaaagtatccatcatggctgatgcaatgcggcggctgcatacgcttgatccggctacctgcccattcgaccaccaagcgaaacatcgcatcgagcgagcacgtactcggatggaagccggtcttgtcgatcaggatgatctggacgaagagcatcaggggctcgcgccagccgaactgttcgccaggctcaaggcgcgcatgcccgacggcgatgatctcgtcgtgacccatggcgatgcctgcttgccgaatatcatggtggaaaatggccgcttttctggattcatcgactgtggccggctgggtgtggcggaccgctatcaggacatagcgttggctacccgtgatattgctgaagagcttggcggcgaatgggctgaccgcttcctcgtgctttacggtatcgccgctcccgattcgcagcgcatcgccttctatcgccttcttgacgagttcttctgaggggatccgctgtaagtctgcagaaattgatgatctattaaacaataaagatgtccactaaaatggaagtttttcctgtcatactttgttaagaagggtgagaacagagtacctacattttgaatggaaggattggagctacgggggtgggggtggggtgggattagataaatgcctgctctttactgaaggctctttactattgctttatgataatgtttcatagttggatatcataatttaaacaagcaaaaccaaattaagggccagctcattcctcccactcatgatctatagatctatagatctctcgtgggatcattgtttttctcttgattcccactttgtggttctaagtactgtggtttccaaatgtgtcagtttcatagcctgaagaacgagatcagcagcctctgttccacatacacttcattctcagtattgttttgccaagttctaattccatcagacctcgacctgcagcccctagcccgggcgccagtagcagcacccacgtccaccttctgtctagtaatgtccaacacctccctcagtccaaacactgctctgcatccatgtggctcccatttatacctgaagcacttgatggggcctcaatgttttactagagcccacccccctgcaactctgagaccctctggatttgtctgtcagtgcctcactggggcgttggataatttcttaaaaggtcaagttccctcagcagcattctctgagcagtctgaagatgtgtgcttttcacagttcaaatccatgtggctgtttcacccacctgcctggccttgggttatctatcaggacctagcctagaagcaggtgtgtggcacttaacacctaagctgagtgactaactgaacactcaagtggatgccatctttgtcacttcttgactgtgacacaagcaactcctgatgccaaagccctgcccacccctctcatgcccatatttggacatggtacaggtcctcactggccatggtctgtgaggtcctggtcctctttgacttcataattcctaggggccactagtatctataagaggaagagggtgctggctcccaggccacagcccacaaaattccacctgctcacaggttggctggctcgacccaggtggtgtcccctgctctgagccagctcccggccaagccagcaccatgggtacccccaagaagaagaggaaggtgcgtaccgatttaaattccaatttactgaccgtacaccaaaatttgcctgcattaccggtcgatgcaacgagtgatgaggttcgcaagaacctgatggacatgttcagggatcgccaggcgttttctgagcatacctggaaaatgcttctgtccgtttgccggtcgtgggcggcatggtgcaagttgaataaccggaaatggtttcccgcagaacctgaagatgttcgcgattatcttctatatcttcaggcgcgcggtctggcagtaaaaactatccagcaacatttgggccagctaaacatgcttcatcgtcggtccgggctgccacgaccaagtgacagcaatgctgtttcactggttatgcggcggatccgaaaagaaaacgttgatgccggtgaacgtgcaaaacaggctctagcgttcgaacgcactgatttcgaccaggttcgttcactcatggaaaatagtgatcgctgccaggatatacgtaatctggcatttctggggattgcttataacaccctgttacgtatagccgaaattgccaggatcagggttaaagatatctcacgtactgacggtgggagaatgttaatccatattggcagaacgaaaacgctggttagcaccgcaggtgtagagaaggcacttagcctgggggtaactaaactggtcgagcgatggatttccgtctctggtgtagctgatgatccgaataactacctgttttgccgggtcagaaaaaatggtgttgccgcgccatctgccaccagccagctatcaactcgcgccctggaagggatttttgaagcaactcatcgattgatttacggcgctaaggtaaatataaaatttttaagtgtataatgtgttaaactactgattctaattgtttgtgtattttaggatgactctggtcagagatacctggcctggtctggacacagtgcccgtgtcggagccgcgcgagatatggcccgcgctggagtttcaataccggagatcatgcaagctggtggctggaccaatgtaaatattgtcatgaactatatccgtaacctggatagtgaaacaggggcaatggtgcgcctgctggaagatggcgattgatctagataagtaatgatcataatcagccatatcacatctgtagaggttttacttgctttaaaaaacctcccacacctccccctgaacctgaaacataaaatgaatgcaattgttgttgttaaacctgccctagttgcggccaattccagctgagcgtgcctccgcaccattaccagttggtctggtgtcaaaaataataataaccgggcaggggggatctaagctctagataagtaatgatcataatcagccatatcacatctgtagaggttttacttgctttaaaaaacctcccacacctccccctgaacctgaaacataaaatgaatgcaattgttgttgttaacttgtttattgcagcttataatggttacaaataaagcaatagcatcacaaatttcacaaataaagcatttttttcactgcattctagttgtggtttgtccaaactcatcaatgtatcttatcatgtctggaataacttcgtataatgtatgctatacgaagttatgctagtaactataacggtcctaaggtagcgagctagctgcaaccgaggaaaaaacgtgccatgaggtctctgtatccaagtgtgact

SEQ ID NO: 20 - DNA, 34073 bp, Artificial Sequence
  Recombinant polynucleotide
gagggagggtggtgctttgctaatggtgaattactaactcctcaataaagaatattatttgaaataatttttgaaatttcataattactttgggttctttcttaatgataaataaataatagtatattacaaacatacattaatatttcctgaatgaatacaccacaaatctcccttaaaatatagcaagaataaaaattatactatttctgacaatttttaatttctcaaataataataccactctgatttttaaacatctacaccactctggctttgccaatctttttaaaaattgaaaagataataattttatcataattacactgaagcatagaactttttctttcaaggaaagcaaatttttgaaattctataatataacctcccataatcctgaataaattaaaggttcaacaacttagtaaagtaagactgaccttcccttttatttctttttcagatcaaaaatcttacttttataggagcagttttcaactcctaaatgttgaatataatagtcagttaaattcaccagctacacaggaatacaggactttgagtggaagaattgaatctctggtaagttaatatttgtctttgctctttattccattataaaatgaatatgataataaacctaatgttttgtaatatattttcagttgctaagtgctctacatattttccttccttgaatggtgaaacatgtgtttctctctgcttttatccagttagtttactcatatactggttcttattcacatctttgtcatgagtaaaaagtgttagaaaggccacgagtaaatatgcattttatttgtttatgaattcaaatactaaaagttttttatttgtttaattaagcattgacattgtctttttaaattcttttcattttaccttcttccctcttccttatccaactaaagacgcaaagcaggaggtgttaaaaaacaggtttaccatatcagcagtaacatagtttggacaacattacactttggttcaatgatagacatagaagtttgaacagaaatatgcaaagcaagtttgagctctaacttgaagagagcctctgggtgcctgccaggaaacctcacgagtggacccttaacattcatgtgtcaccacaaactaggggctgccctttagttttgaccagtctcagtgtcactcacttacccttaccttttcaaaaaaaagtcctaagaatataaagtaattcaatggttctacaattttagcatgtaactgagtcacctggcagggttgctttggtgagctcaagataaaattttatcagcatttctacattttctggaatattccttaatccaggcttttaatcccttggtgcttttctgaaccactgcaatgagcttctaactgttctcactgtgtgcaggctcttttccttctaatctaatttacacacttctgaacacaaatctctcacagcctgtttccttcatgttacctccagctcaagactttttgcctacaaaataaaattcaaacttgttagctaagcaccttctcatgtctatgctttggctcatatttcagccatcgtgtgccccacttattcttatagccaacctgaaaagccatcttttataagaaactacctctgctctccatgattggatataattaatcctccttccacatcacctcgccacaaaattgtatctgtgttgatctcatgccacatacctgtatgtattttatattataaatatttgcagacttgtttaatttgccatgttagactaagttccatgaagacagctccatatccattccatttttatatatccacaacatttggtcgggttgatgcttaataaatgtttattgaaggaacaggagtctcccacttctgacataatgaacttatttcccccagtgttaaccctacatctggttcctgtccaagagtctcttcccaaatcattctgattcaactgttcattctgatctcattaaacatttaaatgatatatctaacttcgcttgctttattctatgctcatcctgcagtctcctcataacttggtttcaatgatgcttgcttctagagaaaaaaatgtattaaataagcttatgattcagtcctccagctgtgatggttctcactgaacattagctcagtggttttcgaagtatggtctctagcataacctagaaacttgttagaaatgcaaattcttgggctcaccaagacatactaaatcaaaaattctgacattggggcctagaaatctgtgttttaacaagcctgccagtgcagcctggtcccttttcttctcggagccccactcaaagctttcagtgctcatctcccaccaatgacagggtcctctatggaaaccggcaggacggtttccaactctaactacgttttagagtttgcttcctagggctatccaggcaccaagtatcacaggttagtttcccagggaagcagactctgagacttgcatgcagggagtgtctctggggtgctctcaaccaacaccttcaggaagagaaggaagcagcattgggcagaggcatagtcaaactacagtgctgttggcacagaagactgaagggagtcagagccagggggtagaggtgggcccttagcatccatccttcaccattaggtgtgagttgccccacctccttgatggtgtaacctcagtcccaaggtgggtgggagtgcagcagagcagcccctacaagggccaaaccagagatacaccaggcgccagaagtgctgccagggaatagagaggaaaggatgggcttaaggtaggatccacagaacttggcaatggattagaagacaggatgagaagtgacaggttaacactaacacagaaatgtctaacttcggtagataatggtgccattggctagaagaggaaaccgaaatgaaagcaggttgttcagggagacaaaagttcactgtggacatctcagcagagtgattcagtggggaaaggaatggatgcccagaccacctcagaggaagatctaagctggagccagcaataaagatacaagatgaacaatccctaacgaactgctcctcagccatgctccccagacacgctgcttcagatttatagtccgggtgaggctaggaggtgcgcctccctcagtggaggacagcaaagcaccagtggctccagggagttaaaatcttttgataatttttgttctagcatctgtctgcagagctgtctctcagccattgcctgcctttacacaggagtgcagtccgaaattgggagatgagtgaaatttattatgcctagagatctggatccccagttgtttgggagtatattttctgaaccacttgttggtttaagtaatgcagatttattgatgccacttctcttgaatctgtgactctggacccaccatctaagtgaatgtgcagagggaacggaatggctgcaatagatctccattaaaaccagtgcatcctcccagacacatacagtagtagggaggtgagtcaatgtcaggacagcaccagctcccgcttcggtacatttccaaagttctcagtctgtgtacaaaggtttgctctggggcagcagaaatagccctgggcaggtagtcaaaggcctggtttgatttcctccacttccaggcaagtcactcgaaggctcacaggctttttcctcacctgccacatgggtccagtgagatctactgagctgtaaataatgaaatgagtgtgtgtgcagtcatctataagttgtaaagtactagaaaatggtgaaactttgggatttgggctatttaaggctgaatgctaaaaatgtcaggcattgtggagaaaggaatttaaatataagattgattgactgggatttaaagacaaatgaaggcacacacgcaagtgcacacccacactgacactgcacagctcccgttggaggcatatcctgaccatgcagacctggggctctgcctgtccaagtgcactcctttactacataaaccctccttctcttttggggctgtcaccccaccagagctggcaccgagcccttgctgctgcgcttccctggggtgtcagcttttgacagggtgtttcctccctctgcaggagccttaacatcccttggacttccttccccccacccacccccagcagttttatctcttcctaactcgggaccctttttttcccacacaaagtttattgtcagttgctggtttcatctgtttgagcggctgcaacaaaataccatagactgggtggcatatgcacgacaaaaatttatttctcacaggagaagtcaaagattaatgcaccagcagatctggtgtctgaggggccaccttctggtttgtagatgatgctttctagttaaaacacctatttaacacactattaaacactaagtgtgttaaatagtgcagttgatgtatttgtcatgtcacctttatcatacactaaatccttctttgtctttttttctgtactctaatctctttctgtaagtaatctttgcttgcagcagtaggatatttagagtactgtggcttgacaatatatttagtatttcaagatttccatgaaattcttctgatgtatgagttccctagttaatcttacatatgtatccctttgtaaaaacactttgaacatttaaaatgatacatgaatagtactctaatacaatgccataaaaattataaatcatttgtatagactggtaagtaaagattgtgagattaagaaacgcatcaaaggccattgagctggaaagtggtataatgagaattcaaaccagggtctcttgactcaaaatctaaggatcataccatttctcatgataatatgagtattattgttatctctatcccatagacaaagtgttaacactgaatgagcagtgaaatagtctcagaattttttattttatttagcaattcacttgtcatttctggtcctcagtttattcacgagtaaaataaaatagttggactagataatttctatagtacattcttacacaaaaaatctatgattttgttatttttaatgtgatatactcatggcactcattcacctcattttcccagcctgcctcactggtcattacttctctgtgttctttacaggctccccctcctctacactgccattaaatattgaaacacctcaaagctttacttatgtccacctctcctctgacactatcattctgtctagatgatcccatacatacatgcccattacttcaacctgtatttatacgccaatgattcactatatttccagcctagacattcttttgtactctagttaccagcttgatatccttacatggctgtttcaaaacaactcaaatatattatctctcaaaatcaaactcatgatgtccccacaccatcctagctttccaccaacaatacctatccctattaatagcaataccatttattcagttatccaaatcaaaaacctagaattcatccttaaaattctactatcattccaaatatcctatccatcagcagccactgtattcttaatcccctgtatttccttcaaatccattcacctctctccatatccattgctgcatgactatccaagccatcgcctctaccctagggtaccaaaatagcaacaaacctaatctgttcatttgcattattttttctccaaaactgattatctatatgtagcaagacagattgttctcaaattgcaaatcccactatattatcctcttgcttcaaacacttccatggtttcccattgtttatgataaaaccaaatgcttcaagttcgaagaccggcatgattgggaatttcctgtcaccctagcctacttgctctccatggtacagttgcactggctttctttcattccttaagtacaacctgtttcctcccacctcaggactgtgcatgtgccattcattctgctgaggagcctttttccttccacttcaatcagctaagtctgattcttcctgacaatctcagctcaataagcatttcctctaagaaatgtctctaatatcattaattggctcaggtccctctactgtattgctgcacttttcacagttataattttacttaattatgaatgattatttgattaggtctatttccatccattagacataagcttcatgatggccagattactgttttctatccatcgttgtattccaatacctgacagaaggagggcgggaggtggtggcacacaagagatgctcaaaaacaattgttgaataagtaaatgaatgaggccatttagaaataacgaaagtacctgtttacaaagtacatgtatcaaaactatgaatgcattctacttacatggttttctccaaataaaacaaaagacttcaatcaggattaatacctgggataaactgagtcattaaatctctcctttgccatcaggagtgacattgaaacaaatgtctgcaaacaacaaatacttttttcccaaaatatattgaatggcatttccataaacaaactagaacatgggaggagaaagaaagcaatattaatttaaaattaatcttatcacataacttataccatcagggatttcgggtaaaattcctttcaggcacatccatttaacaagaattgattgttactgaaagcctagaagagaatttggcacatacttggtgttcaaatatttgttgactgagtgaataaatgatgcaagtgtctaagaaacacaaaataaggacatgattacagtcacggtggagttcacagtcatctccaaaatgaggatatgcatcccagggaggaccaacaattcattggagtgctgaaataaaatactcaaaggtcattttacatgtattttttctctaaattacttttcttaagacacagaaaacaaaaaaagaaacttagctttgttactttctaacaaatagttaaatcattaaacaggattgacactagcatccttgtttggtcttatgccttaggggaacatgaaatgtgtgaagacattctgagatctgagggaagggtagacagtaatacagtgggactgaccaggcttcagcacacctttacctcctctcagcagatttcagtgatgagcagtttacaactagattgaaagattatattatctagttctaaaagaaaactaagcctcccaaaagcaacaagggaactgagaggaatcctgcaaaacaaaaacaaattttaaaacttgcactttgtaataaccctaatatgtaatcacagtaatgaacagtaagataatgacagaactgacatatttccttatctattaaagccatattaacaggtaaagcaatgccagtcagtggtacacttcttagaagatatttaatacatactagacacatacacacacacaacattttccttcaaggtgtatgtatcagaaaatcactttttaaggccggatgcagtggctcaggcctgtaatcccagcactttgggaggccgacgtgggcggatcatctgaggtcaggagttcaagaccagcctgcccaacatggcgaaaccccatctctacaaaaatacaaaaattagccagggatgatggtggatgcttgtagtcccagctactcaagaggcagaggcaggagaatcacttgaacctgggaggcagaggttgcagtgagccaagatcacccattgcactccagcctgggcaacagagtgagactctgtctcaaaaaaaaaaaaatcactttttagataaaattcatgctatagagagaagactatgaaaatatgtttagcaatgtgtccatcattaggtgattgagtttccttttgttttgttttactgaaaatcatataaagtatgttatctgtaaaagttctctgacatgcacacataaaaatttgggagaaaagattaactataatgtttaatagattttgtacacatttctttaaaaatatataaaacacaacacctttcaattggtttgcaagaataaccaattgacatcatggaaaatggaaattcacttgctgaattttaacaaaaatttgcatgatgagtgagactgacaacttagtgtcatgatttaatgaattatgccaatggtaaacttcatgcacatggggccaggtaattatgtggaaactttttcaatgcttaaagccaagtattgaaattaaacttagaatcagacctttgaaccattttatgacaatgttcaaaaattataaattctatccacttatattataatattaaaaatatcattacaaaaaaaacctgtgtttattttataactcagcctttttaatttctaatttcataaatatattataatggatattgttagtaatgtagtattattacatgtatataatttataagtaaatatacatgttttggctactcatgcataaaatgtttcacccataggagcacataatcagaaatgtctggagaccattatagtaatagatagatcatattgccacatattttatctcctccttgacaactgagctttccagatcttctggtgaaacgaaagagaaagttgtaacagaagagtgattaaaatgacaaaagcattacttctattacttctattctaataatatgagcaaagctataactatcaagtaataatgcactaaagaaggtgattaatctgatatattcacaggcaactaataagacctttctattgcagccatgaaaaatatgtgacaattatagatatcctgtgtgcagtgtttcaacctttatgtgacctgttctactaacagatttagtgatgttcactttgttagaattttcttacacatgccataacttgcttcagtcttttgattatgaatattatggatattaaggattctagactattctagatttaaaaaataatattgtcacctcaatcagaagggaaatattaaatagttctcattttttcaatgtttactcagtttttgtccaatgtaatgaaagtgtcagcagtacaggttacaaaataaaatgtgtattaaagtaaactcatttgaacaggttaataattgtagagggagggaaaaggctaaaagattgaatgtaaaacttatgaaaagtagatacatcgtctctatgatttgcagtagtcaactgcatacagatgaatcattttaatacacgttaactactttccttttacagatggagaaactgagaggaagaaagtttatatggttcattaaactttgtgatgcaagctaaactaacctgtctctgtattttccatctactgcccttatcactatctcattagaatactcttcaagcatctccttactgattttcttaccaagcatttgttaagttctaatgagagttggtagtaacattttcacccactctgtgaaatatgaaatcttattcataggcctcttcttttattcttgtatttgcatatcaaccaattaatcaacttgctttctttatgttgcttattatcttagtccttactaaattgcctcttaatgttgtccacataacagaaatgttaaggtggatacttaacattttagtccagtctagccggtgccagtgcaatgccaaatcatgaattaaaatataattacaagaaccacttatcaaattttaacaattccttcagctttgtgacagttttttctacttcgattaaagtcaagtaaaattaaagttaaatatttttattaaaatatctcctttaacattccatattaataaacatattaaagctcatgcttctaagtagattactagaagttactttatcgaattacagcaatggttaattctagatcatagaatttagaatgactttttgccttcttcttttttttccttttttttaaacagagtcttgctctgttgtccaggctggagtgtactggcgcgatcttgactcactgcgacctctgccctgcaggttcaagtgattctcctgccccagcctcttaagtagttgggattacaggtgcctgccaccacacctggctaattttttttttgtatttttaggagagacagggtttcaccatgttggccagactggtctcgaactcctgacctcaagtgatccacttgcctcagcctcccaaagtgctgggattacaggtgtgagccactgtgcctggcctgactttttgctttcttcttaatacttactagtatttcttgaatttttaaaaaagaaacataaagtactttgataaaaccaacagtctcattgttcttaaaattgttcaaaggttctctggaaaaaaaaaagaaaattatcatttggttaagaatcatgttggtctgacatcaatcatcctataggagtgaatattgaaaaagtaagatatattgtggtataatcgagattgcataaattttaccatttttgagaagaatctgctccaaatcctggcttaatgtaatatccagcatgctacttaattttcttgtcttcaccttttcatatccacatccacctaggtgccacctcacagtataagccagcataatccattcttctcaatgaaaccacaatacatctgaccctgcatctcaggagaactgtatcagccacagcacttccagttgactatgaatctgaatgttatgcctcaggagaaacatccttgctgggactgagtagtgattcaaggagatagttatgattcagtcaagaaattaataattagtgttatttttattattgagacagagtctcgttctgtagcccaggctggagtacagtggcatgatctcggctcactgcaacctctacctccccggttcaagtgattctcctgcctcagcctcccaaataactgggacagcaggcacttgccaccacgcctagctaattttttgtatttttagtagagacggagtttcaccgtgttagccaggatggtctcgatctcctgacctcaaggtccacctgcctcagcctcccaaagtgctgggattacaggcgtgagccactgcgcccggccataaattattaactgagccaggcacagtggtacacacttatagtcccagatactcaggagactgaggttggagtatccttttttatgttattttatttttaattattatgggtacataataggtgtacatacccatggagtacaagtcatgttctgatacagacacataatgtttaataatcacatcagggtaattgggatatccatcacctcaagcatttatctttctttgtgttaggaacattccacctccactcttggaataggcaccctgttgtgctattaaatacgaggtcttattcatttcatctaactatatttttctacccattaaccatcacctcttttcccctcttccccactacctttcctgtgaggctgcaggattcttaagcacaacagttagaggccagcctggacaacatagtgagactcaatttctaaaaaataaaaaagaaattaccaactaatgctaaaaaaatagtctctgatgcttaggtatgaattagaaatgaccaaaaaaaaaaaaaaaaaaaagactgccctttgcttccttctccccttctcttcaagttttccattgctactcattttagtctggtttaatcaggtttcatccattaaaagcaattgttgggatcacacattttgagttgtgtcagtggacttccctcatgctggcatgattcctgccccaagcccttagtaaaagccaccaagccatataacataatctctcattgagtaaaacatctgatgtgtttagaatgacttctagcaaaaaaccagcctgtccagcatcatctctgtataacagataaaggaataggtactgcatcaaaaggttatagaacctgcccaaatcaatcccatgtgttttgcaatggaattaggttgaactaaagtgaaaattcagttttctactcctcattaacatgtctcatgttgcaaggttgagaggaaggagaagaagaactgtatttacagagagattccccctctctttctttctacagattactaaaacattcaaagaatcaaatttaagaaatcagttcatcagagctcatgttgccaaactgaggtgagtggaactgtagaaaaaatatttaagtatagatacaatgtggcatacttgactttttgtcacagaatgaatagtaaatgacatgttcagataagttgttgtaatattatgaaaatagtattttagtcagcttaaaaaccaatgccaaaaaagccaaacatatgatctatttagctactaatgtaaataaccatattatatctattcttattgggaagaggaagaaggggtggagagagagttggggtgaaggtacagtaacaaggccatcctattgtaaaactccagtggatatcattcacagtgcagcctatgtaaacagtccctcctggagttgtacaatgctgtggtttgggtgtatccatccaagatcaagacactatgaccaacatcaaaagtggctttttggttttatctgcctgatgtgctataataaaagggtattatggccaaatccaaggcatgtctatcatgaattaataataggaggagtagcagcatgcatgctagttatttgccattcctgccttagttaaatatgatgtgataaaaccagcctttccaactgaaatagtcacctttactgactctcccgcaaatgtctcaaatgaccacattgctctagtctttaaataatatgcaatagttctttggtagaagaggaattatactaattctttctcaaatactagcatcacaagaaaattaattcttgttctctggagagtcacctagtaagtatctggagcacagatgtctggtcaggtaagttttgatgaggagttaaagggataagaagagtccatgagaagggtattttccaaaacacctttcggtcaattcagtgcacattcacttagtactttcttgtcagtatctgtatcagccactaatgttcaaaagtgagtaagccctgaaaacctgtaggactacatgagccttctgccttttctctccttttgttcacttcccacttatcactcaatcctctgcaacctggcttcaataccaccataaaatatcaactgctcttgccgattcaacaatgacatccagataacaaaatccaaagaaaccacatcagtcctattcttggacctttcaacagtatttggtcctgttggcctgtcactccttgaaataggactatcccttggtttgcatggccttgtataccctgattttccccttacctccctagctattccttcttagtttcctttactaggtcttacttctttgtatattccttaaatgttgctgaacatcaggctgtgctctaggcctctcatcttctcaggtcacactctctcctttccttggccttcactgccacccatatgctgagtgctctcaaagttgtatctctaggccagtcctcttttgcctccaaacatgaatatatgcagccatctacttggtaccatcacatggataattctcatgatctcttccagtatgactgcttctttatttttttctgggctcttttttagcattgctttacatggaactttatcatgtctctcaacctctattttatcttttatctatgtatgtagagtctgtgtaatttcttcatctcttttagataactaatatctcttcagctttgacttgtattctgtgtaacccatttattgcgttttcaatttcaatgagtatgttttcctatctgcaagttctatttgtttcttttgagaatcttcctggtcttttaaacacatttcttattttaatttttgggggtacctagtagttgtatgtatttttggagtacatgagatgttttgatacaagcaaacaatgcataataatcacattgtgtaaaatggggtatccatcccctcaagcatttatcctttgtgttacaaacaatccaattatattcttttagttatttttaaatgtacaattaaattattattgaccatagtgactctgttgtgctatcagatactaggtgatcttttaaaaataatgttttctacttaatctcatttttatgattccctcttttacgtcatttgtcatttcaaatacagtcacttgtctgttgattctattatgtgaagtttttgaggataatctttttgttactttgattccaccttggtatggtttggctgtgcccccactaaaatctcatcttgaactctggttcccataatacccacatgttgtgggagggaccttgtgggaggtgattagattatagggacgtttcccccctttgctctgttctttttcctgccaccatgtaagaaagatgtgtttgcttccccttctgccatgattgtaaatttcctgaggcctccgcagccatgcaggacctcttttctttgtaaattacccagtctccggcggttctttatagctccgtgagaaaaaactaatacacacctcatgatgtattgtttaccactgaaattgtatgcttaaatttaatctcacttgggaccctgtacaacctagacttaacatatctacctccagagcagttacatctgtcagacattctagaggaatcagcagcacatggactttgttgttgttaatttgttgtcgggggaggggggagggatagcattaggagatacacctaatgctaaatgacgagttaatgggtgcagcacaccaacatggcacatgtatacatatgtaacaaacctgcacgttgtgcacatataccctaaaacttaaagtataataataataaaattaaaaaaaaaaaggttctgggagtattcaggtagtattaatgaagattcagacatcgtgcagccaggcccatgcttatgaattttcaggtgatacttctttttcttttttcttaatttaaagctggatctcggaaacagataaatttatttttttatgacatgacgagcatttttttcattctagttcatgctgttattgggtgtttagttctttgagactcctggcctttttctaaaacctcaagttcaacttcctattttgcactggcccaaggtcccatctccagtctctatgtaaatgctaaacataagcctgtggaatattctagtctcaccacatactattcacattcttctttgtttttggtcttccaggattttccttacttttctatgaacccagtcttgcatttgaaatggaatttattatatattatctatcctttctatttgttttatgcagaaagtgttttctaaaattatttaggcttccatattgctagacatggaagttgtaattatttgttcagtgcctgtttctacatctaaactgcaagacccatatggcaactgtgaatcttagtcccagctaatttctgaagcttagaatagtgcctagcacaagaagttgtttatctaacatttttaaaaataaatattaaattcatatctggaatgaatattaagttagagctggtcattgaggtgagaggaggaagccaagagagaatatgagagcctcaaagccaaatatctttaatgtactttttcagaaaagaagacagccaatgtcaggtggaggaactggtttatgaggtaactttcctggaagaaaatagaaattactgaggttttagataatccaaatatttaatcaagtcaccaaggtttattgtggggaatctttattattaattaaaatgagtgatgaaatcttaatatacgacaaaagttaaaatttgcttttgcaggcagatgaatggtctaggtatcaaaaaattaagttgagtctctaactcacacaaatttacaaccctatcactttatgaatttgtttaggagattatttttaataacactggtgaagtctaagaatagctaaaatttatagtacacttattgtgtgctattgactcttctttgaagttttgcatatagtgattcatctaatcttcataacccattttacatgtgaagaaacttagatatagaaagattaagaaacttacataacttatccaaagttacacagtaaaactctggcattataacttcaaaatcagctatcctacagtgagtacagtgttctgtgcattgaaatcaaataagtgagatagcatcgtgatatagtattacgtatgcaaacactgttacagagatctgtctaaagttaaattccacaaatgaattctttaaaagggtttaatcaagaagaatatataaacaggatggtgaaaaattgtcatattatttgttttttaaaatatctttatgatttacaggcaagatggtagtggtgtgagagcggatgttgtcatgaaatttcaattcactagaaataacaatggagcatcaatgaaaagcagaattgagtctgttttacgacaaatgctgaataactctggaaacctggaaataaacccttcaactgagataacatgtaagtataatttttcataaacaattttatttcaatatatccctcaagtttaccaattcaaattcatattttaattgagaggctgacttttctttctttgaaactaaactgtgaaaacaatccattaaaaagctaaatataccatatagctccctaacgtaaatcattctaagacttaaagaatcatttggcatttatatagtaaattttatttgctaaaaattctcattaattatccctgcaacattccttatgagtgatgttactgtcagatgtcattagtggataggccataggaggggtacatagatgctcaaggtcagagaactatttaattaatgatccacctcagaggcttcttcatttttctttgtaacatttatcacaattgaaattacaaagttatctgtgtaaattttgtattgtttggcttcatcctacactgtaatcatcctaaaagaaagaaccagtcaaccttcttcatcctactaccctcctaccacccagtctccatcatataacacatattcaataaataattcttgcatgactgaaagaaaagaaataatatatgcatagaatttaaggacattcctccaagttggttacattctgctagtttaataagccattatttcttctcgatgagctcaagattaaaaggattttgatgattcccatactagactggtaggtaccagttacagatgtactaactgttaaatattgaaatgctttcctatttgttggtaaacaattactgcatcaggcccacaaagttgtcttccgagatgtttcaaatccactgcccctgctgctaaagagttatgcttagcaaagcaaagcactctaagacactgctccaactccatggcctgattgcatcttttatgactggccaatgctcacgcactgcagtttgttaggtagttgaatattacctctgcttccacacattaaggaatgctcccgaacgcacttcccaagtgtttatttatttatcattatactagacaatatggtgatacgatggtcacagaatagcggtttccacctccagagcccataatctagttgaagggaaagatattccaacacaagagtgttgacaatcaagatagaatatgatcaagggcccagtgtgaggcccaggcaatgatcactgcaggaatctggggaagaaagagaccagcgtgcttgggatatctagcaaaagtttcatgaaggagaatggactttgactttgaaatatgggtaggatttacatattttgagatgagaaaaagaaagttcccagagaaggaaagcatgaaaaggcaaacagtctgtactgaacgcgatgctttgacagaataatgaagaaagggacctgctggaatgattgatcagtgttcatcattcacaccatcatcatcaaaacacttatttaatgagaacttactgttttttaggcatggctttaatgccctatatgaatttttttcttgattaatccttacaacaaacatatcccatagatagttttattgtcccccttagaaaagataaattgcctaggctgacacagtcagtatatgaggcagtcaggattcaaactaagtctgtttgttcaaaaaattaagaatggccagctttttaaaattttctgtctccagaagtatgatttggctccactgaagtttgcaaaacaaatgtgatacccaaaccttgtgaaacttttagtgggaaataactttgcataagtcggtttgagagagcgtggaaacctgtcttgaaaagttttaatttaacttgcaggaaataaaaatgatgggtttctcaattaaaaatttcaatcaaggaaggatatgagctaacataacatttttttaaaaagatcagtctggtaaggtagaggtgcataaactgaaaaggagcaaaagtggtggaattcagttagaaaattattgtaactgtactgatgtcaaatgatgaaaccatgaactaaagtagtaccaaaaggagtgaggaggatggaataattcaaaagatagaggacagatgtgcagaacctggagattataagatgtgaaaggaggagtttgagaaaatttcagattttggaagtggtgtcattttactaaaaggatataataagtagcaaattttggataaagttgggtcccactgagtttgagatggctgttggacatgcagagaaaactgtcttgtatgctgttcttaaattgaaatagacagacctttaccctctgatactgacatattttcctttccaggctcaccctccatttccctaaacacaacacatgcactagctctccttactttattgctccacaaacatcttacacctccaagcatttgtgcccactgtaccttctatctggaatctcttttgtcctcttgtgtgcctgaaaaattcctttcagatcttcaaaatacagtgcagatgctatttcttctagctcaaatattatctcctccatataatttaattactctcttttttcttttctctactttgcacttacatttatttgaatgattgcttgattaatttctacctgtaaattatgtgagggcaggtcctctatattttgctcgcagttaaatctgcagcacttattatagagtggtatcattagagtaatatacatatatttgaggacatgataaattaacttcccctatagtatttatcacattgcatctcaatgacttgcttatgtttctgttttcccatataaattgagtaacttgaaaaaagagatatctattaagtatttaatgagaaattaaagtacaaactttagtatgcataacaacaaattgggaaaaggttgtaaacaaagagatttgtagggcccatgagttagagatcgtttcagcaggtctgaaaggaagcctaggaatctgcattttagaggaccacctcccaaccccaacaagtaattctgcttcttgttgtctgggtactgtactttaagaaattatggtgaaatgatatcagcctttattgtatttatcttattctcattttttaatactagcacttactgaccaggctgcagcaaattggcttattaatggtaagttttaatattattttgtaactgtaatttgccaaatcataaagagtaaaagtgcaagtcttttgtgtacttttggccaaggcagtatctatcaagttgatgtctttgttcttagttcgctcaggtggtgttgaaacaagacagtgctgatcccaagtgtcccatggagtggactttaggtttcccctttccttttagaaaaaggaagaagttgtagtggaggactacccactctgcactcaaaattgccctcatgaaaatttctttggcagctttgagaaccttttactgccctggttctaaggtggcatttctgtagacttacaaattatgtttgatgacaccgtttatgtagcttctcctaaccaccagagtagcttgctttgttgtgaattcaggttaatcacaaagtataataaaaaagaattgtcagaagtcttcccagctttgggtctataacctgaaggaaaagtcactactcttcaacatcatcctatgtactctcaggctaggatagcagaaatgcaatccctagaaaacagcaacttacttctctgaccaaaaaaatgcagttaaaaattagttcaatgtacctggtagctggcctatcttaggtacttcagtgattttacaaagtgatggtagtcctatgggtgtttttcagcttcactacgtatttaattcatgcttattgttaatgaaactgtgataagcaatttactagggtatttgtttgggagatgccacaaaggaacacatgtatctcttaatggaagcctggtcctcctttatccaggaaatttgctaggaaaaaaaagcctttaggtggttgtgctattaaaccagggcactacttaaaagccagcccagcaatagttgtgtgatttaccattaatttcttagtaatagaccacacaaaagaagaaaattatgggaatgcgagttgagaggaattgggtgatcagcctaccccagcccgtttcagctctggccagtagactattcacgagctctttgaaaacatttaaataaaccttatttagatactagaaaccctctgtcaccctcaagaatattctgtggtatagcgactcctttatgagggcatgtttggtaatacagcatcagtcttggaggtggactggattctacaaggtgaactgcagtcactaaggagtcttttggatgagaccagttttcctccaacttcaatgtgtgcatgaacctcacatcaaaatgtagctttagatttgtcccatgatgtggttccaagaatcagcacttctaataagtttccaggggatgcccatgctgcaggcccacaaaccacactgagcatagcaagactattgagaaaaaggaaatttcccaggagtctgtggcctgagctggcacatccaataatgacctatcttaacctcaactcatgaggaattccagggaactctgaagctgctcaaaatttgaagcctatatgccaactaaattcagaaatgttctccaaaatgctatctataagcaacagtagtcacaaatgcattgtagaaatatatcgatcatgctttttggaaaatccagcatgtcctgaggaagaatgtataagacataaaagtcataaattatggaaagactcttcagcttcttccaaatgtaaaggaatcatgatcttcccagcacattaatgccctttctcattagaatgtggggccggtccagacctaataacattgtctgagcagagaatccttggaggcactgaggctgaggagggaagctggccgtggcaagtcagtctgcggctcaataatgcccaccactgtggaggcagcctgatcaataacatgtggatcctgacagcagctcactgcttcagaaggtgaggccaccactacctacccatctgggaacaattagaatagacaggtcatgaagactgcaccctctaccctaggattgaattgagccagaaataattcaatgcaaaaaaatcagtaagaattttcttcctattcatgaaaggaaaaggatttttcccctttagcatgctaatttagtgctatttctctgtttcaggtaataatatattagcacagtaaagaacaaagatttatatgtcagaatgttttttaaatcctagctataaaagcttaagaaatttactaaatctccataagctttattttttttccaaattaagggacaacactgttatctgtgacttagtgttactggtagcattgagtacactaatgtaaacatacgttaaatgttagcgaaacgaattgctgtggaagatttgcacattatatcatgggagctgatggctaacctagagactgccccatgccattaatttattcattcataaagattattgagtatctagtatgagcacagtgttatatattgtagaagctactagtataaacaaagtattgcctctgccttcaaagagcttacactcgaatgttggaatcagaatgcacaaaaataatgatcaattacaatgagtagcataaataaaattaatgtaggcaacttacaagaattcttaattgaggtgactaaactattgccaacactagggtgatatgctaccagtggcgagtaggttgcataaacttaccttattggtaaaaagaaaagttcacattgctcataaaagaaggattttagatttcagcataactaaaatctgtttcaaacctgccttgttactggggcatcgcagaccacaacagttgttgggaacttaactcaaaaagttcacccagaaaaataatggagatttgaactcgtgtgcccctgaccatatcaattttcttctcagactcttactctaaactggacctccttatcacacacacaaagccttccataggcagatcaatccagtcttatttctcaaagcatgtaccttgagcttcagataaacagcattgttctcttcccctggactcttcctacatttccctacctatgagtatctgatcaatctgcttatccttgaaatgttaatatatttaccacatctctatttgaattttatgaaatttttgataatttctaagtagttttttcagatttataggcactacttcatggtacagtgactgttacaaacgtatttgttaaatttagaaggaataaagatttaaaagactagggtagttactgaactaaagttttaggaaatcccaaattatttcaaatttttcttatggtaattttatgacttaatatttttatatgcagtgaacaaatttgaaactttaaaagatactcccagaattatcagttttctgatgtagattggcaaatttattactatatcccaaataacccaagagacaaaattcacaaaaacatttcaattttcattgccacttgaaaggccaaaaagcagaaatggcacgcattgatttcaatcgtactcttgagtgtgggaaccaggaattaaaatacctggacttatcaggcacttagcataaccaagaacggaatagaaacctccctggattctaagccctattcagtcccaatcaccaaaaaccaagtaaacgatatcactataatgaaagccacagttataaatatcgacaacgattaccaaaggaatccatggaactttgaattttgccaccccacatccttctattcattaccatgattgatccactaaagctaacagactctgtgaaccttgtattggacccctccctaaagacctgattgtcactgagaaccatcagtgaggatttgtttggggcatgaccagccttacatcaaagtacatagaagtgatgaggtcttatcaaagaggattattgaattatcacctcttctatgtagctttccctgatactctctttcctctccattgagttccacagaaatttttttatctgcctttaacagttgtcctcatgatttgtgatatttgacttacctcttgtcagtttccttcactagtgtagagttcctcaaagaaagagaccataattacttatatttttattcctggagactcatactattccttatacaaagtagacacttaacaatggcttgttgaactataattaatgaaaataatagctaccttcatgaaagttcactttgtgccaaacactatagttgacataatacatttgtctcattaatacttaacaattgtgtgagaaggtatcaccaatcacattttatatgtaaataaaccccagagctattaattaacttgtcataaataacacttttcatatgtggcatagccaagatttaaatataaatgttactggttccaaaatgatgctctaattcacttgctggaaagaaggaaaggaagaaaataaacgagtggaaggaagagagggagggaagagagaaaaggaaggaaagaaaaaagagtctcttcagaaccttcactgtaaagactccgagcaaaagaagttgaatataaaaacaacataggtttgtttgttttctaatattttttcttcaaaatttttaactcaggttcactcttacacaaactactgtgtcttataaaagtatttccggtcatagaatttttattttctgtattaactccactatctaatctccataaaactcctaaattggtattatcggtaacattttgtttttactcaacccttaggaacaatgttaagttaatcagccctccacatcacagatccttattttcatcagtctgtacaaggcatttctctcattttaattttttttcctcctgtcatccctggatttcactttcactgccctccttccacccatatgcctcatactaatatattcgaaatatacatgtcttaaaggtacatgcacgcacctacaaaacctatagtgtttttttgtatgtatatgtctttaatttaaataagtagcattgtgtaaaagtctaatattgtttcttactgttttcactcaattcttggaattttcatctgatgcactgctgcatagcaccccatggtatgcagccaccatatttccttcatccaattaggttgcatgacctaccttcccattgccacaaagagtacacacaaaatatttgtacttatctttctgtaaaccttcaggaatttcagaagcacacatgcaggctgctaaatataccagaatactttccagccacttaaatctttaccagtattgcaaaagaggccccatttccctccacatcaacatttagtattattcttttgtttaagttttatcaatcttttaaatgtacacaagatgctcatttttataattttaatttctcagattactagtttgagtatcttttcatatatctaagagctgttttgatctcccctaccatgaactgccactaatattctttgcctattttacaatggtttttctgcttatttattactggtttacagacttttaaaatatattctacaaaaattttagacattaaacattaccaatattttcccatggttcctcatccatctggtaaacttgtctatggtatatctaattttgatttaatagaattcattctatttttaccttttagtttgtgtttttgttgtttagccaaaaagtccccattcctaggtcataaaggtaatgtcctttttttttttttaacgctactgttctctctctgtctccccctatgtatataggtgcacatatacttgtacacacatacatatacctatatatgaggggagttcgataagtttatggaaaataaaattaaaagataaaataaaaaattataaactttatttctcaacataagctccttcaagttcaagacacttttgtaagcaataataccagccatatcgtccatccctaaagaactgagggtcctgagaatttaactatgtcaatgcagtcttttttacattacttttttacagtacttattgatgaaaaatgggtgccttttaaagattgttttaagattagggaacaaaaataagtcagaggaagtcaaatcaggactgaaaggtggatgcctagtgatttattgctgaaactttcataaaactaaccttatttgatgagaggaatgagcatgagcatggttgtgatggagaagaactctggtggagctttcctggacactttttctactaaagctttggctaactttcttactctcataagaagaagatgttatttttcactgaccctttagaaggtcaacaagcaaaatgccttcagcatcccaaatgtctgttgtcatgacttttgttcttgactagtctggttttgctttgactggaccacttctacctctttatagccattgctttgatggtgctttgtcttcaagattgtattagtaaagccatatttcatcttctgttacaattcttcaaagaaatacttcagaatcttgatctgacatgtttaaaatttctattggaagctctgaccttgggtgcagctgatctgggcgaaacagttttggcatccatcaagtagaaagtttgctcaactttagtttttcagtcagaattgtataagctgaaccagttgagatgtctatggtgttgtctattgtttctcacagttaattgttggtcctctttgagacatgaacaagatgaaatttttcctagcaaactgatgtggatgatctgttgctgcgggcttcaccctcaacaacatctctttctttcttgaaacaaattatccattagtaaactgatgattgggggagatgctgtccccataaactttttgtaaggcataaataatttcaccattcttccagtttcaccataaatttgacgtttttttgcttcaattttagcagcattcatgttgctttgataagagctcttttcaaattcatgtcttattcctcttagtgcctcaaactagatcttgttcagtatgacaagttagtatgagtttatctgcatgcaaaaatctttgaaatccatgcatagtttgtttataatatacattttcaatgaacttttgaagaccccatacatacatatgtatatatatgcacacacacacacacacacacaccaaaatcttcaaccattatcagacttagtgcagaaaaattattcatccattaacaagataagaatgccccttatcatcactactatttaaatggagctcctggctaaaggaaaagacagggattgaaaaaaattagttaaatctaaaatgtttattatttcaggtttcttagttgcttaaatgggaagggaggtatggacaaaagagaaatcaaagatatttgtgttatgctacttatcattaaagtatcagaataacttcattggaatagaaaaacaccaagatcaccccacgatatgttttctaaaatcttctccatttctttagacaagtgaccatgtattcggccagtgaagaattaaactcacttgccagcttataatgcaggaaaatatagcaaagagatgtggatccaatagtttctagatagtggtacaggatggctaagatgaatttatatatctgaaatgttcacaaattccctactcatatagcatgttttcataatgttttagcaactctaatcctcgtgactggattgccacgtctggtatttccacaacatttcctaaactaagaatgagagtaagaaatattttaattcataacaattataaatctgcaactcatgaaaatgacattgcacttgtgagacttgagaacagtgtcacctttaccaaagatatccatagtgtgtgtctcccagctgctacccagaatattccacctggctctactgcttatgtaacaggatggggcgctcaagaatatgctggtaagtgtctcggaaaaaaaaattaacaatagaaatgtcttatatttgctattaggtaattttttaaattaggaaacatctggaataggtgtttctattcttctacagacagaaccattctatattctgctcagcccaagctctggctacccctgagtctccttagcaaagcaaagcaatgctccagaaactatgggaattctcaaatatagtaataggaaaatgtaaaagaaagttatgaagacacgagttctttaataatccagagattctataagattcaaatagcttccctataaacaataaaaaagattttgtttgtttgtttgtttgcttgttttttagagacaaagactttctcagactggagtgcagtggtgcaatcatggcttactgcagcctcaaactctggtcttaagaaatcctcttgcttcagcctcccaagtagctagaattataaataagtgtgtaccaccatacccagctttttttttttttttctacagacaggttcttgctctgttgcccaggctggtctggaattcctgccctcaagccatcctcctgccttgttggcctcccaaagcaatgggaggatttagattagacattgtatgagggcttaataatccttaaggtattaactgccctttaaagtattctgggatatggcaaaaactcgatgtgtatataaacattggtcatatttgtttattgaatgaataaaatggaaactaaaatgaggacaatgcacaagagctactagaaccagtaagagtatcagcgaaggagtggaagggtagcattgacaatttccctgggcttttacccatgttgtagattgtctctccaaggaataatacaaagccttaatagtcctagaacacattctattgtgttcttatggcccaaagtaaattggtgtagtagataacatttgcaccagtcatgaaaaactattggtgtcattctgagagtacatcaatataaaatagactagttctttagccttgaaactagactggtttctcttttgctgctaggttaaaggttattcaatatgtaatcttccaatccaaaatctgtcagtggataatttaaaagcttttagtcaattttaagatatttgttttcttaaaattttaaggggcactgtgtcacaaagctaaagaaaaaaaagaaaaaaaaactgatctgtgaaaggggttatcctcatctacttggggaattttggctgcgaagaaactccaaagtaaatctttagaagccttcattgttaaatatgaaataatgtttggagtacatttatttcttctcaaatttattatagggtcaataatgtacacatcttgaagtccatttttttcctgcttttataacaaacaggccacacagttccagagctaaggcaaggacaggtcagaataataagtaatgatgtatgtaatgcaccacatagttataatggagccatcttgtctggaatgctgtgtgctggagtacctcaaggtggagtggacgcatgtcaggtaagctcaagacaatctcatccatgtcatcatccaagaagtgtataagcacttcctagtatgtgataatgtgatagacataagtgtaacagttacaatacacagccctgttcctctaaaatttataatctagattttagaaataaatttttttatgaatgaagtttatctatcatgaaagcattaactctgagaggccaaattacagagtagttaaccatccaaagctcaagaatcagaaagacctcgatttgaattccttaacctctattaccaagtctctaactaaaagctggggataatcataatagcacctaactttttgggtactaagaaaagttaaatgaagactaaatatatcaggcacatggtaaacaacaaagaaatctcatctatttcactattattaatgtagaccatggtcactcgtgttaataactttaacctcaaccttttaactgctgtgaaggattaaataaaaaattaatcactatattataaaaattaattgatatataataaatgaattttaagagatacgtaataattcatggactccttgaagatagaaaatttatacaaaatcctagtaatttgagtcacaaaagctcctacaataatgaaacagtatgaatgaaaaagaaaagaaataactattatatttggatctagcccataatttttaaccaaatgcacaaaaacaaacaacaaatatgaaattctcactgtaaagtgattaaaatcaaatttgaattctaaaattttaaattaaattatctaaacataattgatgcagttatatgttttaataggttttgttcacatatctgaaatccaactccacacagtagcaggaacagctggtgtcagaaattaaatattcttttagtctggagttttaaaaaatcaatctgtttacttgagtaatttgttgctgttttcatgggtgaattgtatacagaaggataagaattattcttcgcatcaaaaggtcactgactttcatatttagtgctcatggtctttaaaaagtggataaaaagtagttctcacatttcatggaaagcccccaatccatgagcacatttcccaaaatgaaacatttttatcaactgcaagttgtgtgtaggtggagatttgtttttcaattgtcaagatactgttaattacccagtcctttatctccttttggtggagatgtctctgtgctaggaaacccttcttgctctccttcctgtttctcttttactactggccctgaaacaacaaattctcaagtttcatgacagctttccaaagaatccatcaatcaaataagcaacacaactcgacactgacaattccagacctactaagagcattaattaagacttaaaaataaacatgagttttaaaagggtgttattcattattttcccatttataacgtcccttaccttctgtccttcagtgcatacaaattattatcttccttgaagcccagttcaagccgtacctcaccatgataccttccatgtatattccactctaggcctcactgatttttaactgaaatactataatgcatagttcacacttaaaaaaaaaaaaaaaacacagcactttacataagagcttacaggatcctatttgttttatccattcttttgttcatttttacaatcattaattcaaaggaattatattaattactttctatgcacccgacgttgtgttaacacaacaatactatccctgcattcagcaagtctatggtctacaagagaggacacaaattcaaatgtctgtagtcaagcagtgaagctggctagatatggaaaaattacaagtccctcttgctttaacatttgcttgcccacatttggtcagacatcatgcaaaataatttctcactatagaaaaaaaaacactacaaaaacaataatataaagaactgagaactggttaactgaagcatgcatatgtcatctaaaagaagcaggtgacgaccagcttcatgaagtacttgccatgcatattggcacttcacacactgacccttctccccacctagaccagtaattaaacaggtatggatgagctagctactaagagcagccaactgaatagctgactaacttagaagcacacttggtaataatagctgacttttattagtactgactatactatatgctaagctgtactcaaagtgctttgagttttaaactgatacaaacattatatgaggaaacagaggtacagagagctattcaccagcttaccaaaggtcacatagctggtaagtggaggacttaaacccagactatctagtttcagaacccacagacttaatccatcgtgcagaacataagacatactccatctgtctccccaactaggttattatgtgcacaaatatttattggttggttggttcattattatgactgggtggtaagtatgtcattaggagtgttttgcttatgactatataaatttcttcaccaaaagaagactttctgatgatatactatgcatcagacaccacgcagggtgctaaggttaggaagataagtgagacttctagaaactcattcattcaacaaatatctcctaagggctagaagcttaggtttcagcagtgaacagaataggtatgttctctttcgtgttggaccttatagtatatctgggaaaacagacattgaataaatatcacaaatgcaagtgagtgtttcagagacatgcagctgctacatcaaaacaaaacagaacaaaacaaacaaacaaaaactgaccagtgggattaagtgtaaataggcacacaaatgcacaaatatgcttttataaaatagtgaagcagtgacagagacacacacaagatataaagacacaatgaagaacaattgagcccaaagctggaaagggtgagagtgtgaaggaaaaaggttgatcagagaagttttcccgaaggagagaaagcctggatgattaggaggcaaccactcggtgactgagggaaatctgaaaaatgtatttgtcatcttctcagacttgctgaaggaatgacttgggtactttgaggatttcagtaatttttccatgacttggtataatatttcaaaaggaaataggctgactttatttgtataatgaatgtgactccttcctcgactgccatagaaataaactccttaatattttgggtttgtctttgcacttaagtaatcagtcattctgtttttttacagggtgactctggtggcccactagtacaagaagactcacggcggctttggtttattgtggggatagtaagctggggagatcagtgtggcctgccggataagccaggagtgtatactcgagtgacagcctaccttgactggattaggcaacaaactgggatctagtgcaacaagtgcatccctgttgcaaagtctgtatgcaggtgtgcctgtcttaaattccaaagctttacatttcaactgaaaaagaaactagaaatgtcctaatttaacatcttgttacataaatatggtttaacaaacactgtttaacctttctttattattaaaggttttctattttctccagagaactatatgaatgttgcatagtactgtggctgtgtaacagaagaaacacactaaactaattacaaagttaacaatttcattacagttgtgctaaatgcccgtagtgagaagaacaggaaccttgagcatgtatagtagaggaacctgcacaggtctgatgggtcagaggggtcttctctgggtttcactgaggatgagaagtaagcaaactgtggaaacatgcaaaggaaaaagtgatagaataatattcaagacaaaaagaacagtatgaggcaagagaaataatatgtatttaaaatttttggttactcaatatcttatacttagtatgagtcctaaaattaaaaatgtgaaactgttgtactatacgtataacctaaccttaattattctgtaagaacatgcttccataggaaatagtggataattttcagctatttaaggcaaaagctaaaatagttcactcctcaactgagacccaaagaattatagatatttttcatgatgacccatgaaaaatatcactcatctacataaaggagagactatatctattttatagagaagctaagaaatatacctacacaaacttgtcaggtgctttacaactacatagtactttttaacaacaaaataataattttaagaatgaaaaatttaatcatcgggaagaacgtcccactacagacttcctatcactggcagttatatttttgagcgtaaaagggtcgtcaaacgctaaatctaagtaacgaattgaaagtttaaagagggggaagagttggtttgcaaaggaaaagtttaaatagcttaatatcaatagaatgatcctgaagacagaaaaaactttgtcactcttcctctctcattttctttctctctctctccccttctcatacacatgcctcccccaccaaagaatataatgtaaattaaatccactaaaatgtaatggcatgaaaatctctgtagtctgaatcactaatattcctgagtttttatgagctcctagtacagctaaagtttgcctatgcatgatcatctatgcgtcagagcttcctccttctacaagctaactccctgcatctgggcatcaggactgctccatacatttgctgaaaacttcttgtatttcctgatgtaaaattgtgcaaacacctacaataaagccatctacttttagggaaagggagttgaaaatgcaaccaactcttggcgaactgtacaaacaaatctttgctatactttatttcaaataaattctttttaaaataatttccctgcctaattatttatggaagttatgacttttgaaggacaattcaaaaccatttatttaattggttctgcaatgaaagaactgccccatatactctactaaaggcttggcactttctgctgccttttaatccagcgctataattgaggcaagcgtccagcttgacacctcgagataacttcgtataatgtatgctatacgaagttatgctagtaactataacggtcctaaggtagcgagctagctgcaaccgaggaaaaaacgtgccatgaggtctctgtatccaagtgtgact

SEQ ID NO: 21 - protein, 418 aa, Artificial Sequence
  Recombinant protein
MYRPRPMLSPSRFFTPFAVAFVVIITVGLLAMMAGLLIHFLAFDQKSYFYRSSFQLLNVEYNSQLNSPATQEYRTLSGRIESLITKTFKESNLRNQFIRAHVAKLRQDGSGVRADVVMKFQFTRNNNGASMKSRIESVLRQMLNNSGNLEINPSTEITSLTDQAAANWLINECGAGPDLITLSEQRILGGTEAEEGSWPWQVSLRLNNAHHCGGSLINNMWILTAAHCFRSNSNPRDWIATSGISTTFPKLRMRVRNILIHNNYKSATHENDIALVRLENSVTFTKDIHSVCLPAATQNIPPGSTAYVTGWGAQEYAGHTVPELRQGQVRIISNDVCNAPHSYNGAILSGMLCAGVPQGGVDACQGDSGGPLVQEDSRRLWFIVGIVSWGDQCGLPDKPGVYTRVTAYLDWIRQQTGI

SEQ ID NO: 22 - DNA, 257 bp, Artificial Sequence
  synthetic oligonucleotide
agcacccctctcttccgcagagtctaagaaatcgctgtgtttagccctcgccctgggcactgtcctcacgggagctgctgtggctgctgtcttgctttggaagttcagtaagtgcagggagcctcgatcccaccatgtgctcctgcagtccccagtgctctgagccagaccctgctctctgggctattgagacctctggaggccctccgtgaggttcctctcttacataacgaggctgtctctcttcccttctcttg

SEQ ID NO: 23 - DNA, 190 bp, Artificial Sequence
  synthetic oligonucleotide
ggtcagaggaccaaaggtgaggcaaggccagacttggtgctcctgtggttctcgagataacttcgtataatgtatgctatacgaagttatatgcatggcctccgcgccgggttttggcgcctcccgcgggcgcccccctcctcacggcgagcgctgccacgtcagacgaagggcgcagcgagcgtcctga

SEQ ID NO: 24 - DNA, 171 bp, Artificial Sequence
  synthetic oligonucleotide
attgttttgccaagttctaattccatcagacctcgacctgcagcccctagataacttcgtataatgtatgctatacgaagttatgctagtaactataacggtcctaaggtagcgagctagctccacgtggctttgtcccagacttcctttgtcttcaacaaccttctgcaa

SEQ ID NO: 25 - DNA, 177 bp, Artificial Sequence
  synthetic oligonucleotide
ggtcagaggaccaaaggtgaggcaaggccagacttggtgctcctgtggttctcgagataacttcgtataatgtatgctatacgaagttatgctagtaactataacggtcctaaggtagcgagctagctccacgtggctttgtcccagacttcctttgtcttcaacaaccttctgcaa

SEQ ID NO: 26 - DNA, 20 bp, Artificial Sequence
  synthetic oligonucleotide
gccgtgactgtgaccttctc

SEQ ID NO: 27 - DNA, 22 bp, Artificial Sequence
  synthetic oligonucleotide
tggaggagccacctgatgcctc

SEQ ID NO: 28 - DNA, 20 bp, Artificial Sequence
  synthetic oligonucleotide
gccttgccctcaatggaaac

SEQ ID NO: 29 - DNA, 21 bp, Artificial Sequence
  synthetic oligonucleotide
ggttgcacagcaaggaagaag

SEQ ID NO: 30 - DNA, 24 bp, Artificial Sequence
  synthetic oligonucleotide
ccaggagttcctgtgagcctaccc

SEQ ID NO: 31 - DNA, 20 bp, Artificial Sequence
  synthetic oligonucleotide
tggaatggaaggagctggag

SEQ ID NO: 32 - DNA, 19 bp, Artificial Sequence
  synthetic oligonucleotide
gtcccacctcctgcaactg

SEQ ID NO: 33 - DNA, 22 bp, Artificial Sequence
  synthetic oligonucleotide
tgagccttcccatcagcctggg

SEQ ID NO: 34 - DNA, 21 bp, Artificial Sequence
  synthetic oligonucleotide
ccacaatggcacatgggtctg

SEQ ID NO: 35 - DNA, 18 bp, Artificial Sequence
  synthetic oligonucleotide
ggtgcttgctccccaaga

SEQ ID NO: 36 - DNA, 20 bp, Artificial Sequence
  synthetic oligonucleotide
cctaaaaggtgttgtaatgg

SEQ ID NO: 37 - DNA, 24 bp, Artificial Sequence
  synthetic oligonucleotide
ggcaataaagaaggaagacgtttt

SEQ ID NO: 38 - DNA, 120 bp, Artificial Sequence
  synthetic oligonucleotide
ccagtcagggacacacatgctcacacgcccgcccacccgcacacactacagtcgagataacttcgtataatgtatgctatacgaagttatatgcatggcctccgcgccgggttttggcgc

SEQ ID NO: 39 - DNA, 198 bp, Artificial Sequence
  synthetic oligonucleotide
attctagttgtggtttgtccaaactcatcaatgtatcttatcatgtctggaataacttcgtataatgtatgctatacgaagttatgctagtaactataacggtcctaaggtagcgagctagccaagtctgtgtgctaccaagtagcaaaactgagcctggaactcacacatgcgtgtctgagagcccagcactatcgc

SEQ ID NO: 40 - DNA, 100 bp, Artificial Sequence
  synthetic oligonucleotide
taatctgactttctcttcatcggtctctcttattctaggctgagctgtaacgctgccgtcccccacatccagaagctgcttcccttcagacctacctacg

SEQ ID NO: 41 - DNA, 177 bp, Artificial Sequence
  synthetic oligonucleotide
ccagtcagggacacacatgctcacacgcccgcccacccgcacacactacagtcgagataacttcgtataatgtatgctatacgaagttatgctagtaactataacggtcctaaggtagcgagctagccaagtctgtgtgctaccaagtagcaaaactgagcctggaactcacacatg

SEQ ID NO: 42 - DNA, 19 bp, Artificial Sequence
  synthetic oligonucleotide
gagcagggccatgacacat

SEQ ID NO: 43 - DNA, 24 bp, Artificial Sequence
  synthetic oligonucleotide
accattagatcccagcactggaca

SEQ ID NO: 44 - DNA, 20 bp, Artificial Sequence
  synthetic oligonucleotide
aaacccttcccgagagagaa

SEQ ID NO: 45 - DNA, 23 bp, Artificial Sequence
  synthetic oligonucleotide
gaggaacactgtgtcaaggactt

SEQ ID NO: 46 - DNA, 22 bp, Artificial Sequence
  synthetic oligonucleotide
cctgaaaagcccggagtggcag

SEQ ID NO: 47 - DNA, 19 bp, Artificial Sequence
  synthetic oligonucleotide
gggcagagaccacatctga

SEQ ID NO: 48 - DNA, 22 bp, Artificial Sequence
  synthetic oligonucleotide
ggaagccctctctcgatacttg

SEQ ID NO: 49 - DNA, 22 bp, Artificial Sequence
  synthetic oligonucleotide
ttctaccctgagggcatgcagc

SEQ ID NO: 50 - DNA, 22 bp, Artificial Sequence
  synthetic oligonucleotide
tgggatgtagaaggttgtcaga

SEQ ID NO: 51 - DNA, 22 bp, Artificial Sequence
  synthetic oligonucleotide
ctgagcctggaactcacacatg

SEQ ID NO: 52 - DNA, 23 bp, Artificial Sequence
  synthetic oligonucleotide
tctgagagcccagcactatcgcc

SEQ ID NO: 53 - DNA, 19 bp, Artificial Sequence
  synthetic oligonucleotide
gctgagggtcaggcttgag

SEQ ID NO: 54 - DNA, 21 bp, Artificial Sequence
  synthetic oligonucleotide
tctgcagggtagggagagaag

SEQ ID NO: 55 - DNA, 29 bp, Artificial Sequence
  synthetic oligonucleotide
tgtttcagaaaaggaagactcacgttaca

SEQ ID NO: 56 - DNA, 24 bp, Artificial Sequence
  synthetic oligonucleotide
gagaccgatgaagagaaagtcaga

SEQ ID NO: 57 - DNA, 100 bp, Artificial Sequence
  synthetic oligonucleotide
gaccattttaaggttttgcttggttgttttggagggagggtggtgctttgctaatggtgaattactaactcctcaataaagaatattatttgaaataatt

SEQ ID NO: 58 - DNA, 190 bp, Artificial Sequence
  synthetic oligonucleotide
gctgccttttaatccagcgctataattgaggcaagcgtccagcttgacacctcgagataacttcgtataatgtatgctatacgaagttatatgcatggcctccgcgccgggttttggcgcctcccgcgggcgcccccctcctcacggcgagcgctgccacgtcagacgaagggcgcagcgagcgtcctga

SEQ ID NO: 59 - DNA, 171 bp, Artificial Sequence
  synthetic oligonucleotide
attgttttgccaagttctaattccatcagacctcgacctgcagcccctagataacttcgtataatgtatgctatacgaagttatgctagtaactataacggtcctaaggtagcgagctagctgcaaccgaggaaaaaacgtgccatgaggtctctgtatccaagtgtgact

SEQ ID NO: 60 - DNA, 177 bp, Artificial Sequence
  synthetic oligonucleotide
ccagtcagggacacacatgctcacacgcccgcccacccgcacacactacactcgagataacttcgtataatgtatgctatacgaagttatgctagtaactataacggtcctaaggtagcgagctagctgcaaccgaggaaaaaacgtgccatgaggtctctgtatccaagtgtgact

SEQ ID NO: 61 - DNA, 21 bp, Artificial Sequence
  synthetic oligonucleotide
tcctctccagacaagaaagct

SEQ ID NO: 62 - DNA, 30 bp, Artificial Sequence
  synthetic oligonucleotide
tcatagcagctttcaaatcctaaacgttga

SEQ ID NO: 63 - DNA, 20 bp, Artificial Sequence
  synthetic oligonucleotide
tcgtgtgtagctggtgagtt

SEQ ID NO: 64 - DNA, 22 bp, Artificial Sequence
  synthetic oligonucleotide
catgcgatcacaggaggagatc

SEQ ID NO: 65 - DNA, 22 bp, Artificial Sequence
  synthetic oligonucleotide
aattgggcccgaagccagatgc

SEQ ID NO: 66 - DNA, 20 bp, Artificial Sequence
  synthetic oligonucleotide
cggaaggcttctgtgacttc

SEQ ID NO: 67 - DNA, 25 bp, Artificial Sequence
  synthetic oligonucleotide
gtctcccacttctgacataatgaac

SEQ ID NO: 68 - DNA, 27 bp, Artificial Sequence
  synthetic oligonucleotide
cccagtgttaaccctacatctggttcc

SEQ ID NO: 69 - DNA, 20 bp, Artificial Sequence
  synthetic oligonucleotide
tgggaagagactcttggaca

SEQ ID NO: 70 - DNA, 25 bp, Artificial Sequence
  synthetic oligonucleotide
atgagctcctagtacagctaaagtt

SEQ ID NO: 71 - DNA, 26 bp, Artificial Sequence
  synthetic oligonucleotide
atgcatgatcatctatgcgtcagagc

SEQ ID NO: 72 - DNA, 21 bp, Artificial Sequence
  synthetic oligonucleotide
tgcccagatgcagggagttag